European Patent Specification EP 3 240 889 B1, published August 13, 2025. Title: COMPOSITIONS AND METHODS FOR HIGH EFFICIENCY IN VIVO GENOME EDITING. Applicant: SYNTHETIC GENOMICS, INC. VERRUTO, John MOELLERING, Eric. The sequence listing filed with the application follows.

SEQUENCE LISTING (118 sequences)

SEQ ID NO: 1 - DNA, 4101 bp, Artificial Sequence
  S. pyogenes
  misc_feature: CAS9 gene codon optimized for Nannochloropsis
gacaagaagtactccatcgggctggacatcgggacgaactccgtgggatgggccgtgatcacagacgaatacaaggtgccttccaagaagttcaaggtgctggggaacacggacagacactccatcaagaagaacctcatcggggccttgctcttcgactccggagaaaccgccgaagcaacgcgattgaaaagaaccgccagaagacgatacacacgacggaagaaccgcatctgctacctccaggagatcttcagcaacgagatggccaaggtggacgactcgttctttcatcgcctggaggagagcttcctggtggaggaagacaagaaacatgagcgccacccgatcttcgggaacatcgtggacgaagtggcctaccacgagaaataccccacgatctaccacttgcgcaagaaactcgtggactccacggacaaagcggacttgcggttgatctacttggccttggcccacatgatcaaatttcggggccacttcctgatcgagggcgacttgaatcccgacaattccgacgtggacaagctcttcatccagctggtgcagacctacaaccagctcttcgaggagaaccccatcaatgcctccggagtggacgccaaagccatcttgtccgcccgattgtccaaatccagacgcttggagaacttgatcgcacaacttcctggcgagaagaagaacggcctcttcggcaacttgatcgcgctgtcgctgggattgacgcctaacttcaagtccaacttcgacttggccgaggacgccaagttgcaactgtccaaggacacctacgacgacgacctcgacaacctgctggcccaaattggcgaccaatacgcggacttgtttttggcggccaagaacttgagcgacgccatcttgttgagcgacatcttgcgcgtgaatacggagatcaccaaagcccctttgtccgcctctatgatcaagcggtacgacgagcaccaccaagacttgaccctgttgaaagccctcgtgcggcaacaattgcccgagaagtacaaggagatcttcttcgaccagtccaagaacgggtacgccggctacatcgacggaggagcctcccaagaagagttctacaagttcatcaagcccatcctggagaagatggacggcaccgaggagttgctcgtgaagctgaaccgcgaagacttgttgcgaaaacagcggacgttcgacaatggcagcatcccccaccaaatccatttgggagagttgcacgccatcttgcgacggcaagaggacttctacccgttcctgaaggacaaccgcgagaaaatcgagaagatcctgacgttcagaatcccctactacgtgggacccttggcccgaggcaattcccggtttgcatggatgacgcgcaaaagcgaagagacgatcaccccctggaacttcgaagaagtggtcgacaaaggagcatccgcacagagcttcatcgagcgaatgacgaacttcgacaagaacctgcccaacgagaaggtgttgcccaagcattcgctgctgtacgagtacttcacggtgtacaacgagctgaccaaggtgaagtacgtgaccgagggcatgcgcaaacccgcgttcctgtcgggagagcaaaagaaggccattgtggacctgctgttcaagaccaaccggaaggtgaccgtgaaacagctgaaagaggactacttcaagaagatcgagtgcttcgactccgtggagatctccggcgtggaggaccgattcaatgcctccttgggaacctaccatgacctcctgaagatcatcaaggacaaggacttcctggacaacgaggagaacgaggacatcctggaggacatcgtgctgaccctgaccctgttcgaggaccgagagatgatcgaggaacggttgaaaacgtacgcccacttgttcgacgacaaggtgatgaagcagctgaaacgccgccgctacaccggatggggacgattgagccgcaaactgattaatggaattcgcgacaagcaatccggaaagaccatcctggacttcctgaagtccgacgggttcgccaaccgcaacttcatgcagctcatccacgacgactccttgaccttcaaggaggacatccagaaggcccaagtgtccggacaaggagactccttgcacgagcacatcgccaatttggccggatcccccgcaatcaaaaaaggcatcttgcaaaccgtgaaagtggtcgacgaactggtgaaggtgatgggacggcacaagcccgagaacatcgtgatcgaaatggcccgcgagaaccaaaccacccaaaaaggacagaagaactcccgagagcgcatgaagcggatcgaagagggcatcaaggagttgggctcccagatcctgaaggagcatcccgtggagaatacccaattgcaaaacgagaagctctacctctactacctccagaacgggcgggacatgtacgtcgaccaagagctggacatcaaccgcctctccgactacgatgtggatcatattgtgccccagagcttcctcaaggacgacagcatcgacaacaaggtcctgacgcgcagcgacaagaaccggggcaagtctgacaatgtgccttccgaagaagtcgtgaagaagatgaagaactactggcggcagctgctcaacgccaagctcatcacccaacggaagttcgacaacctgaccaaggccgagagaggaggattgtccgagttggacaaagccggcttcattaaacgccaactcgtggagacccgccagatcacgaagcacgtggcccaaatcttggactcccggatgaacacgaaatacgacgagaatgacaagctgatccgcgaggtgaaggtgatcacgctgaagtccaagctggtgagcgacttccggaaggacttccagttctacaaggtgcgggagatcaacaactaccatcacgcccatgacgcctacctgaacgccgtggtcggaaccgccctgatcaagaaataccccaagctggagtccgaattcgtgtacggagattacaaggtctacgacgtgcggaagatgatcgcgaagtccgagcaggagatcggcaaagccaccgccaagtacttcttttactccaacatcatgaacttcttcaagaccgagatcacgctcgccaacggcgagatccgcaagcgccccctgatcgagaccaacggcgagacgggagagattgtgtgggacaaaggaagagattttgccacagtgcgcaaggtgctgtccatgcctcaggtgaacatcgtgaagaagaccgaggtgcaaacaggagggttttccaaagagtccattttgcctaagaggaattccgacaagctcatcgcccgcaagaaggactgggaccccaagaagtacgggggcttcgactcccccacggtggcctactccgtgttggtggtggccaaagtggagaaagggaagagcaagaagctgaaatccgtgaaggagttgctcggaatcacgatcatggaacgatcgtcgttcgagaaaaaccccatcgacttcctcgaagccaaagggtacaaagaggtgaagaaggacctgatcatcaagctgcccaagtactccctgttcgagctggagaacggccgcaagcggatgctggcctccgccggggaactgcagaaagggaacgaattggccttgccctccaaatacgtgaacttcctctacttggcctcccattacgaaaagctcaaaggatcccctgaggacaatgagcagaagcaactcttcgtggaacaacacaagcactacctggacgagatcatcgagcagatcagcgagttctccaagcgcgtgatcctcgccgacgccaacctggacaaggtgctctccgcctacaacaagcaccgcgacaagcctatccgcgagcaagccgagaatatcattcacctgtttaccctgacgaatttgggagcccctgccgcctttaaatactttgacaccaccatcgaccgcaaaagatacacctccaccaaggaagtcttggacgccaccctcatccaccagtccatcacgggcctctacgagacgcgcatcgacctctcccaattgggcggcgac

SEQ ID NO: 2 - protein, 1367 aa, Streptococcus pyogenes
  misc_feature: Cas9
DKKYSIGLDIGTNSVGWAVITDEYKVPSKKFKVLGNTDRHSIKKNLIGALLFDSGETAEATRLKRTARRRYTRRKNRICYLQEIFSNEMAKVDDSFFHRLEESFLVEEDKKHERHPIFGNIVDEVAYHEKYPTIYHLRKKLVDSTDKADLRLIYLALAHMIKFRGHFLIEGDLNPDNSDVDKLFIQLVQTYNQLFEENPINASGVDAKAILSARLSKSRRLENLIAQLPGEKKNGLFGNLIALSLGLTPNFKSNFDLAEDAKLQLSKDTYDDDLDNLLAQIGDQYADLFLAAKNLSDAILLSDILRVNTEITKAPLSASMIKRYDEHHQDLTLLKALVRQQLPEKYKEIFFDQSKNGYAGYIDGGASQEEFYKFIKPILEKMDGTEELLVKLNREDLLRKQRTFDNGSIPHQIHLGELHAILRRQEDFYPFLKDNREKIEKILTFRIPYYVGPLARGNSRFAWMTRKSEETITPWNFEEVVDKGASAQSFIERMTNFDKNLPNEKVLPKHSLLYEYFTVYNELTKVKYVTEGMRKPAFLSGEQKKAIVDLLFKTNRKVTVKQLKEDYFKKIECFDSVEISGVEDRFNASLGTYHDLLKIIKDKDFLDNEENEDILEDIVLTLTLFEDREMIEERLKTYAHLFDDKVMKQLKRRRYTGWGRLSRKLINGIRDKQSGKTILDFLKSDGFANRNFMQLIHDDSLTFKEDIQKAQVSGQGDSLHEHIANLAGSPAIKKGILQTVKVVDELVKVMGRHKPENIVIEMARENQTTQKGQKNSRERMKRIEEGIKELGSQILKEHPVENTQLQNEKLYLYYLQNGRDMYVDQELDINRLSDYDVDHIVPQSFLKDDSIDNKVLTRSDKNRGKSDNVPSEEVVKKMKNYWRQLLNAKLITQRKFDNLTKAERGGLSELDKAGFIKRQLVETRQITKHVAQILDSRMNTKYDENDKLIREVKVITLKSKLVSDFRKDFQFYKVREINNYHHAHDAYLNAVVGTALIKKYPKLESEFVYGDYKVYDVRKMIAKSEQEIGKATAKYFFYSNIMNFFKTEITLANGEIRKRPLIETNGETGEIVWDKGRDFATVRKVLSMPQVNIVKKTEVQTGGFSKESILPKRNSDKLIARKKDWDPKKYGGFDSPTVAYSVLVVAKVEKGKSKKLKSVKELLGITIMERSSFEKNPIDFLEAKGYKEVKKDLIIKLPKYSLFELENGRKRMLASAGELQKGNELALPSKYVNFLYLASHYEKLKGSPEDNEQKQLFVEQHKHYLDEIIEQISEFSKRVILADANLDKVLSAYNKHRDKPIREQAENIIHLFTLTNLGAPAAFKYFDTTIDRKRYTSTKEVLDATLIHQSITGLYETRIDLSQLGGD

SEQ ID NO: 3 - protein, 8 aa, SV40 virus
  misc_feature: nuclear localization signal peptide
PKKKRKVG

SEQ ID NO: 4 - DNA, 24 bp, Artificial Sequence
  encoding codon optimized SV40 nuclear localization sequence
cccaagaaaaagcggaaggtcggc

SEQ ID NO: 5 - DNA, 24 bp, Artificial Sequence
  Encoding FLAG tag
gactacaaggatgacgatgacaag

SEQ ID NO: 6 - protein, 8 aa, Artificial Sequence
  FLAG tag peptide
DYKDDDDK

SEQ ID NO: 7 - DNA, 4158 bp, Artificial Sequence
  Engineered Cas9 gene encoding NLS-Cas9-C terminal FLAG tag
atggctcccaagaaaaagcggaaggtcggcgacaagaagtactccatcgggctggacatcgggacgaactccgtgggatgggccgtgatcacagacgaatacaaggtgccttccaagaagttcaaggtgctggggaacacggacagacactccatcaagaagaacctcatcggggccttgctcttcgactccggagaaaccgccgaagcaacgcgattgaaaagaaccgccagaagacgatacacacgacggaagaaccgcatctgctacctccaggagatcttcagcaacgagatggccaaggtggacgactcgttctttcatcgcctggaggagagcttcctggtggaggaagacaagaaacatgagcgccacccgatcttcgggaacatcgtggacgaagtggcctaccacgagaaataccccacgatctaccacttgcgcaagaaactcgtggactccacggacaaagcggacttgcggttgatctacttggccttggcccacatgatcaaatttcggggccacttcctgatcgagggcgacttgaatcccgacaattccgacgtggacaagctcttcatccagctggtgcagacctacaaccagctcttcgaggagaaccccatcaatgcctccggagtggacgccaaagccatcttgtccgcccgattgtccaaatccagacgcttggagaacttgatcgcacaacttcctggcgagaagaagaacggcctcttcggcaacttgatcgcgctgtcgctgggattgacgcctaacttcaagtccaacttcgacttggccgaggacgccaagttgcaactgtccaaggacacctacgacgacgacctcgacaacctgctggcccaaattggcgaccaatacgcggacttgtttttggcggccaagaacttgagcgacgccatcttgttgagcgacatcttgcgcgtgaatacggagatcaccaaagcccctttgtccgcctctatgatcaagcggtacgacgagcaccaccaagacttgaccctgttgaaagccctcgtgcggcaacaattgcccgagaagtacaaggagatcttcttcgaccagtccaagaacgggtacgccggctacatcgacggaggagcctcccaagaagagttctacaagttcatcaagcccatcctggagaagatggacggcaccgaggagttgctcgtgaagctgaaccgcgaagacttgttgcgaaaacagcggacgttcgacaatggcagcatcccccaccaaatccatttgggagagttgcacgccatcttgcgacggcaagaggacttctacccgttcctgaaggacaaccgcgagaaaatcgagaagatcctgacgttcagaatcccctactacgtgggacccttggcccgaggcaattcccggtttgcatggatgacgcgcaaaagcgaagagacgatcaccccctggaacttcgaagaagtggtcgacaaaggagcatccgcacagagcttcatcgagcgaatgacgaacttcgacaagaacctgcccaacgagaaggtgttgcccaagcattcgctgctgtacgagtacttcacggtgtacaacgagctgaccaaggtgaagtacgtgaccgagggcatgcgcaaacccgcgttcctgtcgggagagcaaaagaaggccattgtggacctgctgttcaagaccaaccggaaggtgaccgtgaaacagctgaaagaggactacttcaagaagatcgagtgcttcgactccgtggagatctccggcgtggaggaccgattcaatgcctccttgggaacctaccatgacctcctgaagatcatcaaggacaaggacttcctggacaacgaggagaacgaggacatcctggaggacatcgtgctgaccctgaccctgttcgaggaccgagagatgatcgaggaacggttgaaaacgtacgcccacttgttcgacgacaaggtgatgaagcagctgaaacgccgccgctacaccggatggggacgattgagccgcaaactgattaatggaattcgcgacaagcaatccggaaagaccatcctggacttcctgaagtccgacgggttcgccaaccgcaacttcatgcagctcatccacgacgactccttgaccttcaaggaggacatccagaaggcccaagtgtccggacaaggagactccttgcacgagcacatcgccaatttggccggatcccccgcaatcaaaaaaggcatcttgcaaaccgtgaaagtggtcgacgaactggtgaaggtgatgggacggcacaagcccgagaacatcgtgatcgaaatggcccgcgagaaccaaaccacccaaaaaggacagaagaactcccgagagcgcatgaagcggatcgaagagggcatcaaggagttgggctcccagatcctgaaggagcatcccgtggagaatacccaattgcaaaacgagaagctctacctctactacctccagaacgggcgggacatgtacgtcgaccaagagctggacatcaaccgcctctccgactacgatgtggatcatattgtgccccagagcttcctcaaggacgacagcatcgacaacaaggtcctgacgcgcagcgacaagaaccggggcaagtctgacaatgtgccttccgaagaagtcgtgaagaagatgaagaactactggcggcagctgctcaacgccaagctcatcacccaacggaagttcgacaacctgaccaaggccgagagaggaggattgtccgagttggacaaagccggcttcattaaacgccaactcgtggagacccgccagatcacgaagcacgtggcccaaatcttggactcccggatgaacacgaaatacgacgagaatgacaagctgatccgcgaggtgaaggtgatcacgctgaagtccaagctggtgagcgacttccggaaggacttccagttctacaaggtgcgggagatcaacaactaccatcacgcccatgacgcctacctgaacgccgtggtcggaaccgccctgatcaagaaataccccaagctggagtccgaattcgtgtacggagattacaaggtctacgacgtgcggaagatgatcgcgaagtccgagcaggagatcggcaaagccaccgccaagtacttcttttactccaacatcatgaacttcttcaagaccgagatcacgctcgccaacggcgagatccgcaagcgccccctgatcgagaccaacggcgagacgggagagattgtgtgggacaaaggaagagattttgccacagtgcgcaaggtgctgtccatgcctcaggtgaacatcgtgaagaagaccgaggtgcaaacaggagggttttccaaagagtccattttgcctaagaggaattccgacaagctcatcgcccgcaagaaggactgggaccccaagaagtacgggggcttcgactcccccacggtggcctactccgtgttggtggtggccaaagtggagaaagggaagagcaagaagctgaaatccgtgaaggagttgctcggaatcacgatcatggaacgatcgtcgttcgagaaaaaccccatcgacttcctcgaagccaaagggtacaaagaggtgaagaaggacctgatcatcaagctgcccaagtactccctgttcgagctggagaacggccgcaagcggatgctggcctccgccggggaactgcagaaagggaacgaattggccttgccctccaaatacgtgaacttcctctacttggcctcccattacgaaaagctcaaaggatcccctgaggacaatgagcagaagcaactcttcgtggaacaacacaagcactacctggacgagatcatcgagcagatcagcgagttctccaagcgcgtgatcctcgccgacgccaacctggacaaggtgctctccgcctacaacaagcaccgcgacaagcctatccgcgagcaagccgagaatatcattcacctgtttaccctgacgaatttgggagcccctgccgcctttaaatactttgacaccaccatcgaccgcaaaagatacacctccaccaaggaagtcttggacgccaccctcatccaccagtccatcacgggcctctacgagacgcgcatcgacctctcccaattgggcggcgacgactacaaggatgacgatgacaagtga

SEQ ID NO: 8 - protein, 1385 aa, Artificial Sequence
  NLS-Cas9-C terminal FLAG tag
MAPKKKRKVGDKKYSIGLDIGTNSVGWAVITDEYKVPSKKFKVLGNTDRHSIKKNLIGALLFDSGETAEATRLKRTARRRYTRRKNRICYLQEIFSNEMAKVDDSFFHRLEESFLVEEDKKHERHPIFGNIVDEVAYHEKYPTIYHLRKKLVDSTDKADLRLIYLALAHMIKFRGHFLIEGDLNPDNSDVDKLFIQLVQTYNQLFEENPINASGVDAKAILSARLSKSRRLENLIAQLPGEKKNGLFGNLIALSLGLTPNFKSNFDLAEDAKLQLSKDTYDDDLDNLLAQIGDQYADLFLAAKNLSDAILLSDILRVNTEITKAPLSASMIKRYDEHHQDLTLLKALVRQQLPEKYKEIFFDQSKNGYAGYIDGGASQEEFYKFIKPILEKMDGTEELLVKLNREDLLRKQRTFDNGSIPHQIHLGELHAILRRQEDFYPFLKDNREKIEKILTFRIPYYVGPLARGNSRFAWMTRKSEETITPWNFEEVVDKGASAQSFIERMTNFDKNLPNEKVLPKHSLLYEYFTVYNELTKVKYVTEGMRKPAFLSGEQKKAIVDLLFKTNRKVTVKQLKEDYFKKIECFDSVEISGVEDRFNASLGTYHDLLKIIKDKDFLDNEENEDILEDIVLTLTLFEDREMIEERLKTYAHLFDDKVMKQLKRRRYTGWGRLSRKLINGIRDKQSGKTILDFLKSDGFANRNFMQLIHDDSLTFKEDIQKAQVSGQGDSLHEHIANLAGSPAIKKGILQTVKVVDELVKVMGRHKPENIVIEMARENQTTQKGQKNSRERMKRIEEGIKELGSQILKEHPVENTQLQNEKLYLYYLQNGRDMYVDQELDINRLSDYDVDHIVPQSFLKDDSIDNKVLTRSDKNRGKSDNVPSEEVVKKMKNYWRQLLNAKLITQRKFDNLTKAERGGLSELDKAGFIKRQLVETRQITKHVAQILDSRMNTKYDENDKLIREVKVITLKSKLVSDFRKDFQFYKVREINNYHHAHDAYLNAVVGTALIKKYPKLESEFVYGDYKVYDVRKMIAKSEQEIGKATAKYFFYSNIMNFFKTEITLANGEIRKRPLIETNGETGEIVWDKGRDFATVRKVLSMPQVNIVKKTEVQTGGFSKESILPKRNSDKLIARKKDWDPKKYGGFDSPTVAYSVLVVAKVEKGKSKKLKSVKELLGITIMERSSFEKNPIDFLEAKGYKEVKKDLIIKLPKYSLFELENGRKRMLASAGELQKGNELALPSKYVNFLYLASHYEKLKGSPEDNEQKQLFVEQHKHYLDEIIEQISEFSKRVILADANLDKVLSAYNKHRDKPIREQAENIIHLFTLTNLGAPAAFKYFDTTIDRKRYTSTKEVLDATLIHQSITGLYETRIDLSQLGGDDYKDDDDK

SEQ ID NO: 9 - DNA, 1000 bp, Nannochloropsis gaditana
  misc_feature: RPL7 promoter
gaatgctggcgacctcatgaactttgttgatttttttagaattgtgtcatcgaaaaatatacaatgtcgaagtaaagtttatacactctgggtactcttcttctttgccatccagtaggtgtgggataggagtgcgtggtaattctctgagacagttttcctaccatgtttcgggtccacatagtacaagttgttactcgtgacacctcatttcgcttttgtttctccactaatggactacatttttcaaagcagcagcgtccgcgtttctcgattaagaatctcccgtccgctttgagtttgtttattttaaggattagaaggataaaagcggagctgcaaaggtgaaacatgcctgagaggactagaagacatacggagctgaagtgcggggaggttaaacccgatgatcccattccttgcatttgtcaaggctcaccgcattcatagttctaaaaagaaaatatttccgaataatgttaacacaaaaataattaaatactgttctatgtactccgttcatttgttgatggaatcaaaaggccagaaaaaaagagggggggactccaagctgccgcagacgctcgcctcgtctctcgttcgcggaatgccggtcgtggaaccgctgtgaagataccgtgccttggggatcaattcacacattgacgagggcgcctcacgccgtggcgtacttattcgggccaaaatgttatttccaaggggtgacggatggcatgctcgactcgtgtgatggctgatgcatcaaccctttcaatgctccttcctacttcctcttatccactggtagtctgtcatgagatgtggtgaaccgcgtccgtgataatagtgttctcatttaacctaacaaccaacacaatacaaaacttgattagatacccagtgcatcgaattttgggtgccttcaccgacaagcttgcactttctcgagggacgacaacaacaaaccacctacagcattaccgggcaatagcagcacaac

SEQ ID NO: 10 - DNA, 399 bp, Artificial Sequence
  Aspergillus terreus
  misc_feature: BLAST gene codon optimized for N. gaditana
atggccaagcctttatcccaagaggaatccacgctgatcgaacgtgcaactgcgaccatcaacagcatacctattagcgaggactactcggtggccagtgcagccctctcgtccgacggtcggatctttaccggcgtgaatgtatatcatttcaccggagggccatgcgcggagctcgtggtcctcggaacggccgctgcggctgctgccggaaatctgacgtgcatagtggccatcgggaacgaaaaccgcggcattctgtctccgtgcgggcgatgtcggcaggtgctgcttgacttgcacccggggatcaaggcaattgtcaaagattccgatgggcagcccacagcggttggcatcagggagttgcttccctctggctacgtctgggagggttga

SEQ ID NO: 11 - DNA, 999 bp, Nannochloropsis gaditana
  misc_feature: TCTP promoter
cgtgcaggtgtacagattgaaggaaacaatggagatatctttggcagttgaaaaccgtgttcgaatcatgcttttctactctccaactgagacgaaatttatagcgccatgtcgcttctgactaccaggcttaggaaggcctcatcacaagctggatcggttcgaattaagcaggcactgaagccaagcttgcaagacagccaccttttaattccctcaaaacactttctcaattcagcccggtaaatatgccgattcacagcggccaagatagaggggaggttagcaagaatgttgcgatccctccccagtcgttgcctcgcacacaacctaggccttcacctttccatggaaaattgagaagtgaatattggttttcttacggcatatcagatgaaatcatgacccctaaacatgaagagctgcaggcaaaacacctgctctggacgagcacgatgaaatctcgagaacccgccgtacttcagttgatcccgcatgatgacggccgccattgaaataagccacctcactttattctagcaccgatttccaccgttgtgagggccgaacgaggacaatttcgtgcgaaacaagcacgaacacgcacacgattagtagtacagacgagcagatcgatggcatgcggcacggtctcgcgttctcggcgaccaggacaacggagcagagggaggcctgccgagttccgaggggcattttagtccaaaattgtgttgacacgtgaacaagtggcttgaaaagaggaaggaaatgcctgggtttcccttcgagagcgggaactcgcttgtgcgtcatcctagctacccatggtccctttgtgggggaggctgtttcgtcctaccgaatgtgtggcgctccatgcatcttctgcctcccaaaccaccaacatgagcacgcgaaggaaggagaaaaaagtggccgcaacgttctcttctcatatttattgtctcatcacaaacataggtacataatacaacaatc

SEQ ID NO: 12 - DNA, 318 bp, Nannochloropsis gaditana
  misc_feature: EIF3 terminator
ggcactgtaaccccggttccgctcgacgaaggctgggagcgccctttcggtgggataaaatggatgctttaccgctgcgcttcggctgaggaagagagaaatgcgagcggggatcggggtcctagaaacgaagaaaggagaacaagttcctggccaaagaaaaacaagacaaataccctctccaggcctgggcccattacttttttttgctgtttcttatacctgcactcgtgcttctctagtctgtcgagaccttacctgatcttcctccctccatcgctccccgccccccccatccgagcaaccgtcgaccatacg

SEQ ID NO: 13 - RNA, 112 nt, Artificial Sequence
  Chimeric guide RNA targeting acyl-CoA oxidase gene
gacgggggcuguggcgcgcgguuuuagagcuagaaauagcaaguuaaaauaaggcuaguccguuaucaacuugaaaaaguggcaccgagucggugcuuuuuuuuuuccuuuu

SEQ ID NO: 14 - DNA, 20 bp, Nannochloropsis gaditana
  misc_feature: 20 nucleotide target sequence of acyl-CoA oxidase gene
gacgggggctgtggcgcgcg

SEQ ID NO: 15 - DNA, 861 bp, Nannochloropsis gaditana
  misc_feature: U6 promoter
gcaaaatccttttcgatgctgccatttacttccacagtcttcaggtttaattgcttctcgatgtcagcagtcatcaggagtaccatcaaactttgaattatcaagacccgcgcgaccaagaatgccgggaacgaatgaattaatatgcataatacttatatatgtatggatttgaagatgcaattcaaaagctgggtctgagtacgtctccgaaaaggactcccaaaataggacaagccatacgtacgcgtcttgcacgtaaaaggagaccgtcgaaaacgccacttttacgcattccaggaaggaatagtctcttgcatggcgacatcaaaagtaaccacgtcaaatttcaataacgtgttacatgttgttggtcaatgggtgcatgagtgtccgtatgtcacaagagggtggggggctcgagctggaacatctgcttactgcacgctaggaaggtcgccataagtactttgtgcaaattgtggaaccatcactccttcactacactactcattatcaatgaaatgttgacagctgttcctagtcgtggttgtgtcagattttccctgcatttgcccaactaaaggcactaaagccgactggcatgccagtaggattatggtagttgcctcgcattatatctctctcgtccgtcttgatagccagaaaatacgtaaccactacccatacggcaagcatgtccatgtataaaggttactctgcaaagaaacaatttgaaaatcccagaaaagagagtgtttgaaaaaaccctgcccgatatccacatgttccaaggccattgcaaacaacaccaagctttatagctagcatggtatccgtatttctcgtttacgggaaacc

SEQ ID NO: 16 - DNA, 15 bp, Nannochloropsis gaditana
  misc_feature: U6 terminator
tttttttttcctttt

SEQ ID NO: 17 - DNA, 37 bp, Artificial Sequence
  ACO2-upstream Forward Primer
tcaaagatcatttagcagagacgggggctgtggcgcg

SEQ ID NO: 18 - DNA, 36 bp, Artificial Sequence
  ACO2-downstream Reverse Primer
agtcgagagatggtgcgttcacggatctagccagag

SEQ ID NO: 19 - DNA, 853 bp, Nannochloropsis gaditana
tcaaagatcatttagcagagacgggggctgtggcgcgcgcggtacgtgtggagtcttgctttcttcagggggggtcccggggggggggcgagtcagacaaagggtagagcgtactggaaggacagacagatgctggcatgaccctgcatccagaacacacatttaataattgagggtctggtgatcgaggggctcggcaaccgcgcggctgctagcacgtgacacggttttttacctctactgttccacaatcaacccctacttccccttctccctccctctttccctccctcccctacgttaattttccctcccgctgtactatatcgcttcactttcagccgattagctcctctgccatcaatgccacgccttttgcggcgaggacgacgcataccatggagcgcatggcaagggaacgagccaaggcctccttccccgtccgagacatgacgtacttcttggacggcgggaggagcatgaccgaggtcaaggtgggtgaaataaaaacataaaaagagaataaacaacgaaaggcgaggtctttgggggatgcctgaatacgtaggcaaccgtactgatcgttttggacccttcttctcttggggccgatggcccacaggagggcatgatggcggacttggcggcgaatccggtctttacggacccagaatggaacgacttgaacagagatcaggtagggatatgggtgattggccggaaggtggggaaggagggggaggtgccccttgtgagcttgccctgtggtcggagcgcttccctcgatcaacccctccctctcccttccccttcccccctctggctagatccgtgaacgcaccatctctcgact

SEQ ID NO: 20 - RNA, 103 nt, Artificial Sequence
  Chimeric guide RNA for knocking out CHORD gene
ggaggcuggucaggaugaaaguuuuagagcuagaaauagcaaguuaaaauaaggcuaguccguuaucaacuugaaaaaguggcaccgagucggugcuuuuuuu

SEQ ID NO: 21 - protein, 335 aa, Nannochloropsis gaditana
  misc_feature: CHORD protein
MKLYVHYEEAGQDEKALTLKLTLPKSWAEQPLLQVLELFIESYNKKKTGLPPLDKDFVHMEKAGGVILPVGNIVSDMLSDRDDLYIRSGPGPARGKIAHLSSPPNAHASSESSTGLLRCKNYGCNQSFSEENNSEEACRFHKAPPVFHDTKKGWSCCAKRVYDWDEFHTIEGCTTGRHSLIDPKEIFAPSPTLAAAAQAERGDCSNTSSAATVIKSIDEFNQSNPNAAAACKTAASMTLAGTRCTVKPDGSATCLNKGCQKDYLLKENHPSACRYHAAGPVFHDAGKYWSCCPGTVKYDFDDFLKIPGCMLSSHYDGSQESLEAFTRHAKTSEGT

SEQ ID NO: 22 - DNA, 1029 bp, Artificial Sequence
  Hygromycin resistance gene, codon optimized for Nannochloropsis
atggggaagaaaccggaactgaccgctacgtccgtggagaaattccttattgagaagttcgactctgtctccgacttgatgcaactgagcgagggagaggagagtagggcgttctcgtttgacgtagggggtcggggatacgtgttgagggttaatagttgtgcggacgggttctacaaggatcggtatgtctaccgtcatttcgcctccgccgctctccccataccagaggtactggacattggggagtttagcgaatctctcacgtactgcatctcgcgccgagcccagggagtgacgttgcaagatctgcccgaaactgaattgcctgccgttttgcaacccgtggccgaggccatggacgcgatcgctgccgcagatctgtctcagacgtccggctttggaccttttgggccccagggcatcgggcagtacacgacctggcgagacttcatctgcgccattgccgatcctcacgtctatcattggcagacagtcatggatgacaccgtgtctgcatccgtggcccaagcactggacgaactcatgttgtgggccgaggattgccctgaggtcaggcacctggtgcacgcggatttcggcagcaataacgtacttacagacaatggtcggattactgctgtcatcgactggtccgaagcgatgtttggtgatagccaatacgaagtggcgaacatattcttctggcgtccctggttggcgtgcatggagcagcagacacgctactttgaacggaggcacccggagctggccggctccccacgactccgcgcctatatgttgcgtatcggactcgatcagctttaccagtctctcgtcgacggcaacttcgacgacgccgcgtgggcgcagggccgctgcgacgcgatagtccgcagcggggctgggacggtgggtcggacccaaatcgcacgccggtcggctgcggtgtggacagacggctgtgttgaggtgcttgcggactcgggcaaccgtaggccgagcacccgaccgcgtgcaaaggagtga

SEQ ID NO: 23 - DNA, 1000 bp, Nannochloropsis gaditana
  misc_feature: EIF3 promoter
tcataatcaaagatgagccagccacgaagctaccggagaattctgtaagaaaaatgtttaaagttgaaaatgctaacagtgaagtgatatccttttttaatggagtgttgaggtgaagtctagcatcgtaggggaaaacaggattctgtgtcttccattctactccttgataaagcgaagaaatccgacaaaaccaaagagattgttcaagtttaagatttgtaagcgtacaactatgaacttcttctctttgtaggcctgagtggtcgtatgcatacgattcatgaagtgaatcagtatcgctggattttgcttaggagtaaagcacaactaagaaaatatgctgcctggcaggcatcctgagacatgaggcaagcgacgtagcaattgaatcctaatttaagccagggcatctgtatgactctgttagttaattgatgaaccaatgagctttaaaaaaaaatcgttgcgcgtaatgtagttttaattctccgccttgaggtgcggggccatttcggacaaggttctttggacggagatggcagcatgtgtcccttctccaaattggtccgtgtggtagttgagatgctgccttaaaattctgctcggtcatcctgccttcgcattcactcctttcgagctgtcgggttcctcacgaggcctccgggagcggattgcgcagaaaggcgacccggagacacagagaccatacaccgactaaattgcactggacgatacggcatggcgacgacgatggccaagcattgctacgtgattattcgccttgtcattcagggagaaatgatgacatgtgtgggacggtctttacatgggaagagggcatgaaaataacatggcctggcgggatggagcgtcacacctgtgtatgcgttcgatccacaagcaactcaccatttgcgtcggggcctgtctccaatctgctttaggctacttttctctaatttagcctattctatacagacagagacacacagggatc

SEQ ID NO: 24 - DNA, 702 bp, Artificial Sequence
  TurboGFP gene codon optimized for N. gaditana
atgttggagagcgacgagagcggcctgcccgccatggagatcgagtgccgcatcaccggcaccctgaacggcgtggagttcgagctggtgggcggcggagagggcacccccgagcagggccgcatgaccaacaagatgaagagcaccaaaggcgccctgaccttcagcccctacctgctgagccacgtgatgggctacggcttctaccacttcggcacctaccccagcggctacgagaaccccttcctgcacgccatcaacaacggcggctacaccaacacccgcatcgagaagtacgaggacggcggcgtgctgcacgtgagcttcagctaccgctacgaggccggccgcgtgatcggcgacttcaaggtgatgggcaccggcttccccgaggacagcgtgatcttcaccgacaagatcatccgcagcaacgccaccgtggagcacctgcaccccatgggcgataacgatctggatggcagcttcacccgcaccttcagcctgcgcgacggcggctactacagctccgtggtggacagccacatgcacttcaagagcgccatccaccccagcatcctgcagaacgggggccccatgttcgccttccgccgcgtggaggaggatcacagcaacaccgagctgggcatcgtggagtaccagcacgccttcaagaccccggatgcagatgccggtgaagaataa

SEQ ID NO: 25 - DNA, 1000 bp, Nannochloropsis gaditana
  misc_feature: RPL24 promoter
aataagcatacatcatatgaatacaattcagcttaaatttatcatacaaagatgtaagtgcagcgtgggtctgtaacgatcgggcgtaatttaagataatgcgagggaccgggggaggttttggaacggaatgaggaatgggtcatggcccataataataatatgggtttggtcgcctcgcacagcaaccgtacgtgcgaaaaaggaacagatccatttaataagttgaacgttattctttcctatgcaatgcgtgtatcggaggcgagagcaagtcataggtggctgcgcacaataattgagtctcagctgagcgccgtccgcgggtggtgtgagtggtcatcctcctcccggcctatcgctcacatcgcctctcaatggtggtggtggggcctgatatgacctcaatgccgacccatattaaaacccagtaaagcattcaccaacgaacgaggggctcttttgtgtgtgttttgagtatgattttacacctctttgtgcatctctctggtcttccttggttcccgtagtttgggcatcatcactcacgcttccctcgaccttcgttcttcctttacaaccccgacacaggtcagagttggagtaatcaaaaaaggggtgcacgaatgagatacattagattttgacagatatccttttactggagagggttcaagggatcaaatgaacagcgggcgttggcaatctagggagggatcggaggttggcagcgagcgaaagcgtgtccatccttttggctgtcacacctcacgaaccaactgttagcaggccagcacagatgacatacgagaatctttattatatcgtagaccttatgtggatgacctttggtgctgtgtgtctggcaatgaacctgaaggcttgatagggaggtggctcccgtaaaccctttgtcctttccacgctgagtctcccccgcactgtcctttatacaaattgttacagtcatctgcaggcggtttttctttggcaggcaaag

SEQ ID NO: 26 - DNA, 317 bp, Nannochloropsis gaditana
  misc_feature: Bidirectional terminator 2
agtgatgcggcctttaggaaacaccacaaaagtaattgacaatctcaggaacgatctgcgtgtttacagcttcccaaataacaattataccacgtaccaaaaggggtttaatgtatctcacaaattcttctaataggtacagcttctcaaattgggtgtatgatgtgacacttcgtctcacacacgtcacgataattcagcgtatggcttcccttcatcacattcacgcaaacttctacacaaccctgggcatatttcttgtgttggcaacactcccgaaatcgattctgcacacaatggttcattcaatgattcaa

SEQ ID NO: 27 - DNA, 10103 bp, Artificial Sequence
  Chord3-KOvector
ctgtcagaccaagtttactcatatatactttagattgatttaaaacttcatttttaatttaaaaggatctaggtgaagatcctttttgataatctcatgaccaaaatcccttaacgtgagttttcgttccactgagcgtcagaccccgtagaaaagatcaaaggatcttcttgagatcctttttttctgcgcgtaatctgctgcttgcaaacaaaaaaaccaccgctaccagcggtggtttgtttgccggatcaagagctaccaactctttttccgaaggtaactggcttcagcagagcgcagataccaaatactgtccttctagtgtagccgtagttaggccaccacttcaagaactctgtagcaccgcctacatacctcgctctgctaatcctgttaccagtggctgctgccagtggcgataagtcgtgtcttaccgggttggactcaagacgatagttaccggataaggcgcagcggtcgggctgaacggggggttcgtgcacacagcccagcttggagcgaacgacctacaccgaactgagatacctacagcgtgagctatgagaaagcgccacgcttcccgaagggagaaaggcggacaggtatccggtaagcggcagggtcggaacaggagagcgcacgagggagcttccagggggaaacgcctggtatctttatagtcctgtcgggtttcgccacctctgacttgagcgtcgatttttgtgatgctcgtcaggggggcggagcctatggaaaaacgccagcaacgcggcctttttacggttcctggccttttgctggccttttgctcacatgttctttcctgcgttatcccctgattctgtggataaccgtattaccgcctttgagtgagctgataccgctcgccgcagccgaacgaccgagcgcagcgagtcagtgagcgaggaagcggaagagtttaaacagggggcatcagaatctatgccgtatatgagcttatgaatgtcatccattatctcatgtctgtcaacgcggtcctcgggtgtaacaaaacacaggaggagcgtctcacttttgaccagcagctttctgccttagagcgcaccgtccgtgtcaaagaaaatgagctcaaagaattggagcttctatctagtacgtgacattatataaggaggcaaagtgctctattaatatgttgacgagaaggtttaatacatgcagcaggtaacagatgcaggacaagtgtgtgaaatttaaccggctacttcctatgaatcaaacagaagatgcttacaatgcacaggagatcgctgaacaagaactagcaaaagagcgctctgaatataatgaggagcgtgcgcgaagggaaagaaggctacgggaacgacagcgtaatgcaaaatattgtttacaaagacaaatgcaagagcaggagaagtcgcaaggcgaaagtgcgggtggtagcatatgccaacaggaaactgaccagcaggacgagcaagacgacgaagctggtagcgaagattacgtgactacacagcaagtggaagcggacagattaagaactttgacaatgcttgtcaaaagtataactgggatcggtgatgcacaggcattgcgctcaaaacttgagcaccaaggggaggtcttgcggaagtcacaagaaattagcaaagataatcaggtgactacaagaatgatagactggtactaccccagactcgttgacatccggcgtgtcgagcgttcacatcagagatatgaaggtagatgacggtaaaagtttcctaaaatcgagcacgcgacttttttttcttcttcaatatctgagcaggatcgcttagagaagctacagaaagagcgggacatcctctggaatcaattacagagttccagatattcaccgcgccccctcaaggtctgtaacgaataataagagaggtcatcacttggccctgatcgcgatgctgtagaggttattgatgaaaggggaggaaagaatggcaggggccgtatagaaataatcctcaggattttgaaggcgtgcgtcatcctagaccaaatttgcaggaaagatgcttagaaatctcaaaattgacgcggatatttttgactaatcgacaaacatgctttcacgaccacagtccgaaggcctacttcgccagctgttgcacgacaaggaaaaagtcaaggagatcgaaaataggtgcgagtacttagcacaacttgtggcacatttgcagtgtggtttagtggagcgtttatggcctttagtaatgcgaagcaatcggaatcaccttgctgcttcgccaaagacggaaaatctcgatcgagtggcgcttcaacgtatgcttaaaaagttagaagtccgctgcttgcagctgcttgacaccaaatccatcccacaaaagcattgaaattctcaaatatggggaaccaaacgctcatccaacccatcccaagccccaggcttgcttctgtcgaatccgcagcactcagcacgcatgtgtagtatcttttggataaatcattgcaaagaaggtgtataaggctttttcccggaagcaaaagctcccgtgggcactgtagaaacaaaagtgaggtgatagttatttttcgatgcacggaacggtatatatattcgcaaagcttgtggaggctatcgctgtcctttgtttgaagcagtcttcagcgaagctgccacggagcttcgttcaggaccgtttcttggcattcaaaactctacgactatgatactatcgagcattccgcatgattacagcgcaaagcctaccaaaaagatgcggtaattcacttgcgggaccgcaatcattgtcagccatcagcgcactgtactcgtaaaaaggcgaacattgtccggtaactcgctcatgtctcacttgagctgatgtcctctctaaaataatagggtcggtcccaaactcttttaaactccgatgaaactctatgtgcactacgagcggccgcaataagcatacatcatatgaatacaattcagcttaaatttatcatacaaagatgtaagtgcagcgtgggtctgtaacgatcgggcgtaatttaagataatgcgagggaccgggggaggttttggaacggaatgaggaatgggtcatggcccataataataatatgggtttggtcgcctcgcacagcaaccgtacgtgcgaaaaaggaacagatccatttaataagttgaacgttattctttcctatgcaatgcgtgtatcggaggcgagagcaagtcataggtggctgcgcacaataattgagtctcagctgagcgccgtccgcgggtggtgtgagtggtcatcctcctcccggcctatcgctcacatcgcctctcaatggtggtggtggggcctgatatgacctcaatgccgacccatattaaaacccagtaaagcattcaccaacgaacgaggggctcttttgtgtgtgttttgagtatgattttacacctctttgtgcatctctctggtcttccttggttcccgtagtttgggcatcatcactcacgcttccctcgaccttcgttcttcctttacaaccccgacacaggtcagagttggagtaatcaaaaaaggggtgcacgaatgagatacattagattttgacagatatccttttactggagagggttcaagggatcaaatgaacagcgggcgttggcaatctagggagggatcggaggttggcagcgagcgaaagcgtgtccatccttttggctgtcacacctcacgaaccaactgttagcaggccagcacagatgacatacgagaatctttattatatcgtagaccttatgtggatgacctttggtgctgtgtgtctggcaatgaacctgaaggcttgatagggaggtggctcccgtaaaccctttgtcctttccacgctgagtctcccccgcactgtcctttatacaaattgttacagtcatctgcaggcggtttttctttggcaggcaaacatgttggagagcgacgagagcggcctgcccgccatggagatcgagtgccgcatcaccggcaccctgaacggcgtggagttcgagctggtgggcggcggagagggcacccccgagcagggccgcatgaccaacaagatgaagagcaccaaaggcgccctgaccttcagcccctacctgctgagccacgtgatgggctacggcttctaccacttcggcacctaccccagcggctacgagaaccccttcctgcacgccatcaacaacggcggctacaccaacacccgcatcgagaagtacgaggacggcggcgtgctgcacgtgagcttcagctaccgctacgaggccggccgcgtgatcggcgacttcaaggtgatgggcaccggcttccccgaggacagcgtgatcttcaccgacaagatcatccgcagcaacgccaccgtggagcacctgcaccccatgggcgataacgatctggatggcagcttcacccgcaccttcagcctgcgcgacggcggctactacagctccgtggtggacagccacatgcacttcaagagcgccatccaccccagcatcctgcagaacgggggccccatgttcgccttccgccgcgtggaggaggatcacagcaacaccgagctgggcatcgtggagtaccagcacgccttcaagaccccggatgcagatgccggtgaagaataaatttaaatagtgatgcggcctttaggaaacaccacaaaagtaattgacaatctcaggaacgatctgcgtgtttacagcttcccaaataacaattataccacgtaccaaaaggggtttaatgtatctcacaaattcttctaataggtacagcttctcaaattgggtgtatgatgtgacacttcgtctcacacacgtcacgataattcagcgtatggcttcccttcatcacattcacgcaaacttctacacaaccctgggcatatttcttgtgttggcaacactcccgaaatcgattctgcacacaatggttcattcaatgattcaatcactcctttgcacgcggtcgggtgctcggcctacggttgcccgagtccgcaagcacctcaacacagccgtctgtccacaccgcagccgaccggcgtgcgatttgggtccgacccaccgtcccagccccgctgcggactatcgcgtcgcagcggccctgcgcccacgcggcgtcgtcgaagttgccgtcgacgagagactggtaaagctgatcgagtccgatacgcaacatataggcgcggagtcgtggggagccggccagctccgggtgcctccgttcaaagtagcgtgtctgctgctccatgcacgccaaccagggacgccagaagaatatgttcgccacttcgtattggctatcaccaaacatcgcttcggaccagtcgatgacagcagtaatccgaccattgtctgtaagtacgttattgctgccgaaatccgcgtgcaccaggtgcctgacctcagggcaatcctcggcccacaacatgagttcgtccagtgcttgggccacggatgcagacacggtgtcatccatgactgtctgccaatgatagacgtgaggatcggcaatggcgcagatgaagtctcgccaggtcgtgtactgcccgatgccctggggcccaaaaggtccaaagccggacgtctgagacagatctgcggcagcgatcgcgtccatggcctcggccacgggttgcaaaacggcaggcaattcagtttcgggcagatcttgcaacgtcactccctgggctcggcgcgagatgcagtacgtgagagattcgctaaactccccaatgtccagtacctctggtatggggagagcggcggaggcgaaatgacggtagacataccgatccttgtagaacccgtccgcacaactattaaccctcaacacgtatccccgaccccctacgtcaaacgagaacgccctactctcctctccctcgctcagttgcatcaagtcggagacagagtcgaacttctcaataaggaatttctccacggacgtagcggtcagttccggtttcttccccatgatccctgtgtgtctctgtctgtatagaataggctaaattagagaaaagtagcctaaagcagattggagacaggccccgacgcaaatggtgagttgcttgtggatcgaacgcatacacaggtgtgacgctccatcccgccaggccatgttattttcatgccctcttcccatgtaaagaccgtcccacacatgtcatcatttctccctgaatgacaaggcgaataatcacgtagcaatgcttggccatcgtcgtcgccatgccgtatcgtccagtgcaatttagtcggtgtatggtctctgtgtctccgggtcgcctttctgcgcaatccgctcccggaggcctcgtgaggaacccgacagctcgaaaggagtgaatgcgaaggcaggatgaccgagcagaattttaaggcagcatctcaactaccacacggaccaatttggagaagggacacatgctgccatctccgtccaaagaaccttgtccgaaatggccccgcacctcaaggcggagaattaaaactacattacgcgcaacgatttttttttaaagctcattggttcatcaattaactaacagagtcatacagatgccctggcttaaattaggattcaattgctacgtcgcttgcctcatgtctcaggatgcctgccaggcagcatattttcttagttgtgctttactcctaagcaaaatccagcgatactgattcacttcatgaatcgtatgcatacgaccactcaggcctacaaagagaagaagttcatagttgtacgcttacaaatcttaaacttgaacaatctctttggttttgtcggatttcttcgctttatcaaggagtagaatggaagacacagaatcctgttttcccctacgatgctagacttcacctcaacactccattaaaaaaggatatcacttcactgttagcattttcaactttaaacatttttcttacagaattctccggtagcttcgtggctggctcatctttgattatgaggcgcgccaggcattgacgcttaagttgactctgcccaaaagctgggcggagcagccgttgcttcaagtactggagctgttcatcgaatcctacaacaagaaaaagaccggtctacctcccttggacaaagactttgtccacatggaaaaagctgggtaagtccttactcgtgacagcgttccctttctccagactagacgcctaatagtgttctaatgtaccactgggacacgcctcgctgcctgtgcaccatgctccatactcaacgctgctacaggggcgtaatccttccagtcggcaacattgtgagcgacatgttgagcgatagagatgatttgtatatcagatccgggccagggcctgctcgtgggaagattgcccatctcagttcgcccccaaacgcgcacgcttcgagtgagtcgagcacaggattgttgcgctgcaaaaactatggatgcaatcagtcattttcggaagaaaacaattcagaagaggcgtgccgctttcacaaggcaccccccgtctttcatgatacgaagaaagggtggtcgtgctgcgcgaagcgagtatatgactgggacgagttccatacggtaagcgtggaagtgttcgttctcggccccaggactttgttttgaggcaattggtgtactttaattggcggataaagggaggactcacaactttcgatattcaccgtctccagatcgaggggtgcaccacaggacggcacagtctcatcgatccgaaggaaattttcgcgccgtcccccaccctggctgcagccgcgcaggccgagaggggagattgcagcaatacgtcaagcgctgctacagtcatcaagagcattgatgaattcaatcagtcgaatccaaatgccgccgctgcatgcaaaacagcagcctcgatgacgctggcgggcacgcgctgcaccgtcaaaccggacgggtctgccacctgtttgaacaaaggctgccaaaaggactacttgctcaaggagaatcacccctctgcatgtcggtaaggacaccgcgctcgatggaatcgtgagctttacgttcccacgccaacacttcgccatttctcctcccttcctttctttagctaccacgcagccggccccgtcttccacgacgcgggtaaatactggtcatgttgccctggaacggtcaagtacgacttcgacgactttctcaagatccctggatgcatgctcagtagtcattacgacggaagccaggagagcctggaggcgttcactagacacgccaaaacgtctgagggcacatgagaatgtgggatggggagaaagaaccacgtatccccacgaggaatggcgcattgggagcgagggggatcgacataggaagaagcaataaaaattctgctcaatacggtattttttattttttggcgtcttccgttcgtagccggcggacgaacagcgatgcaaactcgagacggacagtgccccacggtcttcgttcgaaaacatcattgccaacaacctcgcacacttacttccaggatcctataaatatcttacaaccaccatccgcctcttccttctcacgcgcatggataatcaacgccacgattcacaccgttgcctggacatttcccccccatgacgggtaatcctacccgtttccttccagcgttccccttctcttccattcgaacttgaatgcactttacttatttctcttgtgagcatcgtgcatccgcttgctggcaacggcaatgggaatgataatcacaagcaggatcgccaggattgccagtcccataaccattttcatctagatcgtatggagcaaaggaagagagagggggtaagggcgagaagatcgcaatgaaaagggatgacggcccacgccgcctcctgcgacttccaatcgtccgaggtttacacacatggcacagccagaaacacccccggcataggagcaggataggggtaagacaaccaagcacgtactcggagctgtttccagcacatctgtttaaacgacgaaagggcctcgtgatacgcctatttttataggttaatgtcatgataataatggtttcttagacgtcaggtggcacttttcggggaaatgtgcgcggaacccctatttgtttatttttctaaatacattcaaatatgtatccgctcatgagacaataaccctgataaatgcttcaataatattgaaaaaggaagagtatgagtattcaacatttccgtgtcgcccttattcccttttttgcggcattttgccttcctgtttttgctcacccagaaacgctggtgaaagtaaaagatgctgaagatcagttgggtgcacgagtgggttacatcgaactggatctcaacagcggtaagatccttgagagttttcgccccgaagaacgttttccaatgatgagcacttttaaagttctgctatgtggcgcggtattatcccgtattgacgccgggcaagagcaactcggtcgccgcatacactattctcagaatgacttggttgagtactcaccagtcacagaaaagcatcttacggatggcatgacagtaagagaattatgcagtgctgccataaccatgagtgataacactgcggccaacttacttctgacaacgatcggaggaccgaaggagctaaccgcttttttgcacaacatgggggatcatgtaactcgccttgatcgttgggaaccggagctgaatgaagccataccaaacgacgagcgtgacaccacgatgcctgtagcaatggcaacaacgttgcgcaaactattaactggcgaactacttactctagcttcccggcaacaattaatagactggatggaggcggataaagttgcaggaccacttctgcgctcggcccttccggctggctggtttattgctgataaatctggagccggtgagcgtgggtctcgcggtatcattgcagcactggggccagatggtaagccctcccgtatcgtagttatctacacgacggggagtcaggcaactatggatgaacgaaatagacagatcgctgagataggtgcctcactgattaagcattggtaa

SEQ ID NO: 28 - DNA, 2016 bp, Nannochloropsis gaditana
  misc_feature: CHORD target upstream homology arm
agggggcatcagaatctatgccgtatatgagcttatgaatgtcatccattatctcatgtctgtcaacgcggtcctcgggtgtaacaaaacacaggaggagcgtctcacttttgaccagcagctttctgccttagagcgcaccgtccgtgtcaaagaaaatgagctcaaagaattggagcttctatctagtacgtgacattatataaggaggcaaagtgctctattaatatgttgacgagaaggtttaatacatgcagcaggtaacagatgcaggacaagtgtgtgaaatttaaccggctacttcctatgaatcaaacagaagatgcttacaatgcacaggagatcgctgaacaagaactagcaaaagagcgctctgaatataatgaggagcgtgcgcgaagggaaagaaggctacgggaacgacagcgtaatgcaaaatattgtttacaaagacaaatgcaagagcaggagaagtcgcaaggcgaaagtgcgggtggtagcatatgccaacaggaaactgaccagcaggacgagcaagacgacgaagctggtagcgaagattacgtgactacacagcaagtggaagcggacagattaagaactttgacaatgcttgtcaaaagtataactgggatcggtgatgcacaggcattgcgctcaaaacttgagcaccaaggggaggtcttgcggaagtcacaagaaattagcaaagataatcaggtgactacaagaatgatagactggtactaccccagactcgttgacatccggcgtgtcgagcgttcacatcagagatatgaaggtagatgacggtaaaagtttcctaaaatcgagcacgcgacttttttttcttcttcaatatctgagcaggatcgcttagagaagctacagaaagagcgggacatcctctggaatcaattacagagttccagatattcaccgcgccccctcaaggtctgtaacgaataataagagaggtcatcacttggccctgatcgcgatgctgtagaggttattgatgaaaggggaggaaagaatggcaggggccgtatagaaataatcctcaggattttgaaggcgtgcgtcatcctagaccaaatttgcaggaaagatgcttagaaatctcaaaattgacgcggatatttttgactaatcgacaaacatgctttcacgaccacagtccgaaggcctacttcgccagctgttgcacgacaaggaaaaagtcaaggagatcgaaaataggtgcgagtacttagcacaacttgtggcacatttgcagtgtggtttagtggagcgtttatggcctttagtaatgcgaagcaatcggaatcaccttgctgcttcgccaaagacggaaaatctcgatcgagtggcgcttcaacgtatgcttaaaaagttagaagtccgctgcttgcagctgcttgacaccaaatccatcccacaaaagcattgaaattctcaaatatggggaaccaaacgctcatccaacccatcccaagccccaggcttgcttctgtcgaatccgcagcactcagcacgcatgtgtagtatcttttggataaatcattgcaaagaaggtgtataaggctttttcccggaagcaaaagctcccgtgggcactgtagaaacaaaagtgaggtgatagttatttttcgatgcacggaacggtatatatattcgcaaagcttgtggaggctatcgctgtcctttgtttgaagcagtcttcagcgaagctgccacggagcttcgttcaggaccgtttcttggcattcaaaactctacgactatgatactatcgagcattccgcatgattacagcgcaaagcctaccaaaaagatgcggtaattcacttgcgggaccgcaatcattgtcagccatcagcgcactgtactcgtaaaaaggcgaacattgtccggtaactcgctcatgtctcacttgagctgatgtcctctctaaaataatagggtcggtcccaaactcttttaaactccgatgaaactctatgtgcactacga

SEQ ID NO: 29 - DNA, 1997 bp, Nannochloropsis gaditana
  misc_feature: CHORD target upstream homology arm
aggcattgacgcttaagttgactctgcccaaaagctgggcggagcagccgttgcttcaagtactggagctgttcatcgaatcctacaacaagaaaaagaccggtctacctcccttggacaaagactttgtccacatggaaaaagctgggtaagtccttactcgtgacagcgttccctttctccagactagacgcctaatagtgttctaatgtaccactgggacacgcctcgctgcctgtgcaccatgctccatactcaacgctgctacaggggcgtaatccttccagtcggcaacattgtgagcgacatgttgagcgatagagatgatttgtatatcagatccgggccagggcctgctcgtgggaagattgcccatctcagttcgcccccaaacgcgcacgcttcgagtgagtcgagcacaggattgttgcgctgcaaaaactatggatgcaatcagtcattttcggaagaaaacaattcagaagaggcgtgccgctttcacaaggcaccccccgtctttcatgatacgaagaaagggtggtcgtgctgcgcgaagcgagtatatgactgggacgagttccatacggtaagcgtggaagtgttcgttctcggccccaggactttgttttgaggcaattggtgtactttaattggcggataaagggaggactcacaactttcgatattcaccgtctccagatcgaggggtgcaccacaggacggcacagtctcatcgatccgaaggaaattttcgcgccgtcccccaccctggctgcagccgcgcaggccgagaggggagattgcagcaatacgtcaagcgctgctacagtcatcaagagcattgatgaattcaatcagtcgaatccaaatgccgccgctgcatgcaaaacagcagcctcgatgacgctggcgggcacgcgctgcaccgtcaaaccggacgggtctgccacctgtttgaacaaaggctgccaaaaggactacttgctcaaggagaatcacccctctgcatgtcggtaaggacaccgcgctcgatggaatcgtgagctttacgttcccacgccaacacttcgccatttctcctcccttcctttctttagctaccacgcagccggccccgtcttccacgacgcgggtaaatactggtcatgttgccctggaacggtcaagtacgacttcgacgactttctcaagatccctggatgcatgctcagtagtcattacgacggaagccaggagagcctggaggcgttcactagacacgccaaaacgtctgagggcacatgagaatgtgggatggggagaaagaaccacgtatccccacgaggaatggcgcattgggagcgagggggatcgacataggaagaagcaataaaaattctgctcaatacggtattttttattttttggcgtcttccgttcgtagccggcggacgaacagcgatgcaaactcgagacggacagtgccccacggtcttcgttcgaaaacatcattgccaacaacctcgcacacttacttccaggatcctataaatatcttacaaccaccatccgcctcttccttctcacgcgcatggataatcaacgccacgattcacaccgttgcctggacatttcccccccatgacgggtaatcctacccgtttccttccagcgttccccttctcttccattcgaacttgaatgcactttacttatttctcttgtgagcatcgtgcatccgcttgctggcaacggcaatgggaatgataatcacaagcaggatcgccaggattgccagtcccataaccattttcatctagatcgtatggagcaaaggaagagagagggggtaagggcgagaagatcgcaatgaaaagggatgacggcccacgccgcctcctgcgacttccaatcgtccgaggtttacacacatggcacagccagaaacacccccggcataggagcaggataggggtaagacaaccaagcacgtactcggagctgtttccagcacatct

SEQ ID NO: 30 - DNA, 23 bp, Nannochloropsis gaditana
  misc_feature: CHORD-CRISPR target, including PAM sequence
ggaggctggtcaggatgaaaagg

SEQ ID NO: 31 - RNA, 20 nt, Artificial Sequence
  20 nucleotide targeting sequence homologous to CHORD gene
ggaggcuggucaggaugaaa

SEQ ID NO: 32 - RNA, 103 nt, Artificial Sequence; identical to SEQ ID NO: 20
  Entire chimeric guide RNA for targeting CHORD gene

SEQ ID NO: 33 - DNA, 120 bp, Artificial Sequence
  oligo-chord3 sense oligonucleotide
taatacgactcactataggaggctggtcaggatgaaagttttagagctagaaatagcaagttaaaataaggctagtccgttatcaacttgaaaaagtggcaccgagtcggtgcttttttt

SEQ ID NO: 34 - DNA, 120 bp, Artificial Sequence
  Oligo-chord3 reverse complement oligonucleotide
aaaaaaagcaccgactcggtgccactttttcaagttgataacggactagccttattttaacttgctatttctagctctaaaactttcatcctgaccagcctcctatagtgagtcgtatta

SEQ ID NO: 35 - DNA, 19 bp, Artificial Sequence
  T7 Promoter
taatacgactcactatagg

SEQ ID NO: 36 - DNA, 25 bp, Artificial Sequence
  oligo- KFchord3 Forward primer
gtcggtcccaaactcttttaaactc

SEQ ID NO: 37 - DNA, 25 bp, Artificial Sequence
  misc_feature: Synthetic
  misc_feature: oligo- KFchord3 Reverse primer
gtcggtcccaaactcttttaaactc

SEQ ID NO: 38 - DNA, 11263 bp, Artificial Sequence
  pSGE-6206 vector
gcggccgccgtatggtcgacggttgctcggatggggggggcggggagcgatggagggaggaagatcaggtaaggtctcgacagactagagaagcacgagtgcaggtataagaaacagcaaaaaaaagtaatgggcccaggcctggagagggtatttgtcttgtttttctttggccaggaacttgttctcctttcttcgtttctaggaccccgatccccgctcgcatttctctcttcctcagccgaagcgcagcggtaaagcatccattttatcccaccgaaagggcgctcccagccttcgtcgagcggaaccggggttacagtgcctcaaccctcccagacgtagccagagggaagcaactccctgatgccaaccgctgtgggctgcccatcggaatctttgacaattgccttgatccccgggtgcaagtcaagcagcacctgccgacatcgcccgcacggagacagaatgccgcggttttcgttcccgatggccactatgcacgtcagatttccggcagcagccgcagcggccgttccgaggaccacgagctccgcgcatggccctccggtgaaatgatatacattcacgccggtaaagatccgaccgtcggacgagagggctgcactggccaccgagtagtcctcgctaataggtatgctgttgatggtcgcagttgcacgttcgatcagcgtggattcctcttgggataaaggcttggccatcgagctcggtacccggggatccatgattgttgtattatgtacctatgtttgtgatgagacaataaatatgagaagagaacgttgcggccacttttttctccttccttcgcgtgctcatgttggtggtttgggaggcagaagatgcatggagcgccacacattcggtaggacgaaacagcctcccccacaaagggaccatgggtagctaggatgacgcacaagcgagttcccgctctcgaagggaaacccaggcatttccttcctcttttcaagccacttgttcacgtgtcaacacaattttggactaaaatgcccctcggaactcggcaggcctccctctgctccgttgtcctggtcgccgagaacgcgagaccgtgccgcatgccatcgatctgctcgtctgtactactaatcgtgtgcgtgttcgtgcttgtttcgcacgaaattgtcctcgttcggccctcacaacggtggaaatcggtgctagaataaagtgaggtggcttatttcaatggcggccgtcatcatgcgggatcaactgaagtacggcgggttctcgagatttcatcgtgctcgtccagagcaggtgttttgcctgcagctcttcatgtttaggggtcatgatttcatctgatatgccgtaagaaaaccaatattcacttctcaattttccatggaaaggtgaaggcctaggttgtgtgcgaggcaacgactggggagggatcgcaacattcttgctaacctcccctctatcttggccgctgtgaatcggcatatttaccgggctgaattgagaaagtgttttgagggaattaaaaggtggctgtcttgcaagcttggcttcagtgcctgcttaattcgaaccgatccagcttgtgatgaggccttcctaagcctggtagtcagaagcgacatggcgctataaatttcgtctcagttggagagtagaaaagcatgattcgaacacggttttcaactgccaaagatatctccattgtttccttcaatctgtacacctgcacggtgcaccagttggtacggcatattatggtttaataagcatacatcatatgaatacaattcagcttaaatttatcatacaaagatgtaagtgcagcgtgggtctgtaacgatcgggcgtaatttaagataatgcgagggaccgggggaggttttggaacggaatgaggaatgggtcatggcccataataataatatgggtttggtcgcctcgcacagcaaccgtacgtgcgaaaaaggaacagatccatttaataagttgaacgttattctttcctatgcaatgcgtgtatcggaggcgagagcaagtcataggtggctgcgcacaataattgagtctcagctgagcgccgtccgcgggtggtgtgagtggtcatcctcctcccggcctatcgctcacatcgcctctcaatggtggtggtggggcctgatatgacctcaatgccgacccatattaaaacccagtaaagcattcaccaacgaacgaggggctcttttgtgtgtgttttgagtatgattttacacctctttgtgcatctctctggtcttccttggttcccgtagtttgggcatcatcactcacgcttccctcgaccttcgttcttcctttacaaccccgacacaggtcagagttggagtaatcaaaaaaggggtgcacgaatgagatacattagattttgacagatatccttttactggagagggttcaagggatcaaatgaacagcgggcgttggcaatctagggagggatcggaggttggcagcgagcgaaagcgtgtccatccttttggctgtcacacctcacgaaccaactgttagcaggccagcacagatgacatacgagaatctttattatatcgtagaccttatgtggatgacctttggtgctgtgtgtctggcaatgaacctgaaggcttgatagggaggtggctcccgtaaaccctttgtcctttccacgctgagtctcccccgcactgtcctttatacaaattgttacagtcatctgcaggcggtttttctttggcaggcaaagatgcccaagaaaaagcggaaggtcggcgactacaaggatgacgatgacaagttggagcctggagagaagccctacaaatgccctgagtgcggaaagagcttcagccaatctggagccttgacccggcatcaacgaacgcatacacgagacaagaagtactccatcgggctggacatcgggacgaactccgtgggatgggccgtgatcacagacgaatacaaggtgccttccaagaagttcaaggtgctggggaacacggacagacactccatcaagaagaacctcatcggggccttgctcttcgactccggagaaaccgccgaagcaacgcgattgaaaagaaccgccagaagacgatacacacgacggaagaaccgcatctgctacctccaggagatcttcagcaacgagatggccaaggtggacgactcgttctttcatcgcctggaggagagcttcctggtggaggaagacaagaaacatgagcgccacccgatcttcgggaacatcgtggacgaagtggcctaccacgagaaataccccacgatctaccacttgcgcaagaaactcgtggactccacggacaaagcggacttgcggttgatctacttggccttggcccacatgatcaaatttcggggccacttcctgatcgagggcgacttgaatcccgacaattccgacgtggacaagctcttcatccagctggtgcagacctacaaccagctcttcgaggagaaccccatcaatgcctccggagtggacgccaaagccatcttgtccgcccgattgtccaaatccagacgcttggagaacttgatcgcacaacttcctggcgagaagaagaacggcctcttcggcaacttgatcgcgctgtcgctgggattgacgcctaacttcaagtccaacttcgacttggccgaggacgccaagttgcaactgtccaaggacacctacgacgacgacctcgacaacctgctggcccaaattggcgaccaatacgcggacttgtttttggcggccaagaacttgagcgacgccatcttgttgagcgacatcttgcgcgtgaatacggagatcaccaaagcccctttgtccgcctctatgatcaagcggtacgacgagcaccaccaagacttgaccctgttgaaagccctcgtgcggcaacaattgcccgagaagtacaaggagatcttcttcgaccagtccaagaacgggtacgccggctacatcgacggaggagcctcccaagaagagttctacaagttcatcaagcccatcctggagaagatggacggcaccgaggagttgctcgtgaagctgaaccgcgaagacttgttgcgaaaacagcggacgttcgacaatggcagcatcccccaccaaatccatttgggagagttgcacgccatcttgcgacggcaagaggacttctacccgttcctgaaggacaaccgcgagaaaatcgagaagatcctgacgttcagaatcccctactacgtgggacccttggcccgaggcaattcccggtttgcatggatgacgcgcaaaagcgaagagacgatcaccccctggaacttcgaagaagtggtcgacaaaggagcatccgcacagagcttcatcgagcgaatgacgaacttcgacaagaacctgcccaacgagaaggtgttgcccaagcattcgctgctgtacgagtacttcacggtgtacaacgagctgaccaaggtgaagtacgtgaccgagggcatgcgcaaacccgcgttcctgtcgggagagcaaaagaaggccattgtggacctgctgttcaagaccaaccggaaggtgaccgtgaaacagctgaaagaggactacttcaagaagatcgagtgcttcgactccgtggagatctccggcgtggaggaccgattcaatgcctccttgggaacctaccatgacctcctgaagatcatcaaggacaaggacttcctggacaacgaggagaacgaggacatcctggaggacatcgtgctgaccctgaccctgttcgaggaccgagagatgatcgaggaacggttgaaaacgtacgcccacttgttcgacgacaaggtgatgaagcagctgaaacgccgccgctacaccggatggggacgattgagccgcaaactgattaatggaattcgcgacaagcaatccggaaagaccatcctggacttcctgaagtccgacgggttcgccaaccgcaacttcatgcagctcatccacgacgactccttgaccttcaaggaggacatccagaaggcccaagtgtccggacaaggagactccttgcacgagcacatcgccaatttggccggatcccccgcaatcaaaaaaggcatcttgcaaaccgtgaaagtggtcgacgaactggtgaaggtgatgggacggcacaagcccgagaacatcgtgatcgaaatggcccgcgagaaccaaaccacccaaaaaggacagaagaactcccgagagcgcatgaagcggatcgaagagggcatcaaggagttgggctcccagatcctgaaggagcatcccgtggagaatacccaattgcaaaacgagaagctctacctctactacctccagaacgggcgggacatgtacgtcgaccaagagctggacatcaaccgcctctccgactacgatgtggatcatattgtgccccagagcttcctcaaggacgacagcatcgacaacaaggtcctgacgcgcagcgacaagaaccggggcaagtctgacaatgtgccttccgaagaagtcgtgaagaagatgaagaactactggcggcagctgctcaacgccaagctcatcacccaacggaagttcgacaacctgaccaaggccgagagaggaggattgtccgagttggacaaagccggcttcattaaacgccaactcgtggagacccgccagatcacgaagcacgtggcccaaatcttggactcccggatgaacacgaaatacgacgagaatgacaagctgatccgcgaggtgaaggtgatcacgctgaagtccaagctggtgagcgacttccggaaggacttccagttctacaaggtgcgggagatcaacaactaccatcacgcccatgacgcctacctgaacgccgtggtcggaaccgccctgatcaagaaataccccaagctggagtccgaattcgtgtacggagattacaaggtctacgacgtgcggaagatgatcgcgaagtccgagcaggagatcggcaaagccaccgccaagtacttcttttactccaacatcatgaacttcttcaagaccgagatcacgctcgccaacggcgagatccgcaagcgccccctgatcgagaccaacggcgagacgggagagattgtgtgggacaaaggaagagattttgccacagtgcgcaaggtgctgtccatgcctcaggtgaacatcgtgaagaagaccgaggtgcaaacaggagggttttccaaagagtccattttgcctaagaggaattccgacaagctcatcgcccgcaagaaggactgggaccccaagaagtacgggggcttcgactcccccacggtggcctactccgtgttggtggtggccaaagtggagaaagggaagagcaagaagctgaaatccgtgaaggagttgctcggaatcacgatcatggaacgatcgtcgttcgagaaaaaccccatcgacttcctcgaagccaaagggtacaaagaggtgaagaaggacctgatcatcaagctgcccaagtactccctgttcgagctggagaacggccgcaagcggatgctggcctccgccggggaactgcagaaagggaacgaattggccttgccctccaaatacgtgaacttcctctacttggcctcccattacgaaaagctcaaaggatcccctgaggacaatgagcagaagcaactcttcgtggaacaacacaagcactacctggacgagatcatcgagcagatcagcgagttctccaagcgcgtgatcctcgccgacgccaacctggacaaggtgctctccgcctacaacaagcaccgcgacaagcctatccgcgagcaagccgagaatatcattcacctgtttaccctgacgaatttgggagcccctgccgcctttaaatactttgacaccaccatcgaccgcaaaagatacacctccaccaaggaagtcttggacgccaccctcatccaccagtccatcacgggcctctacgagacgcgcatcgacctctcccaattgggcggcgactaaagtgatgcggcctttaggaaacaccacaaaagtaattgacaatctcaggaacgatctgcgtgtttacagcttcccaaataacaattataccacgtaccaaaaggggtttaatgtatctcacaaattcttctaataggtacagcttctcaaattgggtgtatgatgtgacacttcgtctcacacacgtcacgataattcagcgtatggcttcccttcatcacattcacgcaaacttctacacaaccctgggcatatttcttgtgttggcaacactcccgaaatcgattctgcacacaatggttcattcaatgattcaagtacgttttagacggactaggcagtttaattaaaaacatctatcctccagatcaccagggccagtgaggccggcataaaggacggcaaggaaagaaaagaaagaaagaaaaggacacttatagcatagtttgaagttataagtagtcgcaatctgtgtgcagccgacagatgctttttttttccgtttggcaggaggtgtagggatgtcgaagaccagtccagctagtatctatcctacaagtcaatcatgctgcgacaaaaatttctcgcacgaggcctctcgataaacaaaactttaaaagcacacttcattgtcatgcagagtaataactcttccgcgtcgatcaatttatcaatctctatcatttccgcccctttccttgcatagagcaagaaaagcgacccggatgaggataacatgtcctgcgccagtagtgtggcattgcctgtctctcatttacacgtactgaaagcataatgcacgcgcataccaatatttttcgtgtacggagatgaagagacgcgacacgtaagatcacgagaaggcgagcacggttgccaatggcagacgcgctagtctccattatcgcgttgttcggtagcttgctgcatgtcttcagtggcactatatccactctgcctcgtcttctacacgagggccacatcggtgcaagttcgaaaaatcatatctcaatcttcagatcctttccagaaacggtgctcaggcgggaaagtgaaggttttctactctagtggctaccccaattctctccgactgtcgcagacggtccttcgttgcgcacgcaccgcgcactacctctgaaattcgacaaccgaagttcaattttacatctaacttctttcccattctctcaccaaaagcctagcttacatgttggagagcgacgagagcggcctgcccgccatggagatcgagtgccgcatcaccggcaccctgaacggcgtggagttcgagctggtgggcggcggagagggcacccccgagcagggccgcatgaccaacaagatgaagagcaccaaaggcgccctgaccttcagcccctacctgctgagccacgtgatgggctacggcttctaccacttcggcacctaccccagcggctacgagaaccccttcctgcacgccatcaacaacggcggctacaccaacacccgcatcgagaagtacgaggacggcggcgtgctgcacgtgagcttcagctaccgctacgaggccggccgcgtgatcggcgacttcaaggtgatgggcaccggcttccccgaggacagcgtgatcttcaccgacaagatcatccgcagcaacgccaccgtggagcacctgcaccccatgggcgataacgatctggatggcagcttcacccgcaccttcagcctgcgcgacggcggctactacagctccgtggtggacagccacatgcacttcaagagcgccatccaccccagcatcctgcagaacgggggccccatgttcgccttccgccgcgtggaggaggatcacagcaacaccgagctgggcatcgtggagtaccagcacgccttcaagaccccggatgcagatgccggtgaagaataagggtgggaaggagtcggggagggtcctggcagagcggcgtcctcatgatgtgttggagacctggagagtcgagagcttcctcgtcacctgattgtcatgtgtgtataggttaagggggcccactcaaagccataaagacgaacacaaacactaatctcaacaaagtctactagcatgccgtctgtccatctttatttcctggcgcgcctatgcttgtaaaccgttttgtgaaaaaatttttaaaataaaaaaggggacctctagggtccccaattaattagtaatataatctattaaaggtcattcaaaaggtcatccagacgaaagggcctcgtgatacgcctatttttataggttaatgtcatgataataatggtttcttagacgtcaggtggcacttttcggggaaatgtgcgcggaacccctatttgtttatttttctaaatacattcaaatatgtatccgctcatgagacaataaccctgataaatgcttcaataatattgaaaaaggaagagtatgagtattcaacatttccgtgtcgcccttattcccttttttgcggcattttgccttcctgtttttgctcacccagaaacgctggtgaaagtaaaagatgctgaagatcagttgggtgcacgagtgggttacatcgaactggatctcaacagcggtaagatccttgagagttttcgccccgaagaacgttttccaatgatgagcacttttaaagttctgctatgtggcgcggtattatcccgtattgacgccgggcaagagcaactcggtcgccgcatacactattctcagaatgacttggttgagtactcaccagtcacagaaaagcatcttacggatggcatgacagtaagagaattatgcagtgctgccataaccatgagtgataacactgcggccaacttacttctgacaacgatcggaggaccgaaggagctaaccgcttttttgcacaacatgggggatcatgtaactcgccttgatcgttgggaaccggagctgaatgaagccataccaaacgacgagcgtgacaccacgatgcctgtagcaatggcaacaacgttgcgcaaactattaactggcgaactacttactctagcttcccggcaacaattaatagactggatggaggcggataaagttgcaggaccacttctgcgctcggcccttccggctggctggtttattgctgataaatctggagccggtgagcgtgggtctcgcggtatcattgcagcactggggccagatggtaagccctcccgtatcgtagttatctacacgacggggagtcaggcaactatggatgaacgaaatagacagatcgctgagataggtgcctcactgattaagcattggtaactgtcagaccaagtttactcatatatactttagattgatttaaaacttcatttttaatttaaaaggatctaggtgaagatcctttttgataatctcatgaccaaaatcccttaacgtgagttttcgttccactgagcgtcagaccccgtagaaaagatcaaaggatcttcttgagatcctttttttctgcgcgtaatctgctgcttgcaaacaaaaaaaccaccgctaccagcggtggtttgtttgccggatcaagagctaccaactctttttccgaaggtaactggcttcagcagagcgcagataccaaatactgtccttctagtgtagccgtagttaggccaccacttcaagaactctgtagcaccgcctacatacctcgctctgctaatcctgttaccagtggctgctgccagtggcgataagtcgtgtcttaccgggttggactcaagacgatagttaccggataaggcgcagcggtcgggctgaacggggggttcgtgcacacagcccagcttggagcgaacgacctacaccgaactgagatacctacagcgtgagctatgagaaagcgccacgcttcccgaagggagaaaggcggacaggtatccggtaagcggcagggtcggaacaggagagcgcacgagggagcttccagggggaaacgcctggtatctttatagtcctgtcgggtttcgccacctctgacttgagcgtcgatttttgtgatgctcgtcaggggggcggagcctatggaaaaacgccagcaacgcggcctttttacggttcctggccttttgctggccttttgctcacatgttctttcctgcgttatcccctgattctgtggataaccgtattaccgcctttgagtgagctgataccgctcgccgcagccgaacgaccgagcgcagcgagtcagtgagcgaggaagcggaaga

SEQ ID NO: 39 - DNA, 147 bp, Artificial Sequence
  Encodes N-terminal peptide linker
atgcccaagaaaaagcggaaggtcggcgactacaaggatgacgatgacaagttggagcctggagagaagccctacaaatgccctgagtgcggaaagagcttcagccaatctggagccttgacccggcatcaacgaacgcatacacga

SEQ ID NO: 40 - DNA, 822 bp, Nannochloropsis gaditana
  misc_feature: 4A-III promoter
ggcataaaggacggcaaggaaagaaaagaaagaaagaaaaggacacttatagcatagtttgaagttataagtagtcgcaatctgtgtgcagccgacagatgctttttttttccgtttggcaggaggtgtagggatgtcgaagaccagtccagctagtatctatcctacaagtcaatcatgctgcgacaaaaatttctcgcacgaggcctctcgataaacaaaactttaaaagcacacttcattgtcatgcagagtaataactcttccgcgtcgatcaatttatcaatctctatcatttccgcccctttccttgcatagagcaagaaaagcgacccggatgaggataacatgtcctgcgccagtagtgtggcattgcctgtctctcatttacacgtactgaaagcataatgcacgcgcataccaatatttttcgtgtacggagatgaagagacgcgacacgtaagatcacgagaaggcgagcacggttgccaatggcagacgcgctagtctccattatcgcgttgttcggtagcttgctgcatgtcttcagtggcactatatccactctgcctcgtcttctacacgagggccacatcggtgcaagttcgaaaaatcatatctcaatcttcagatcctttccagaaacggtgctcaggcgggaaagtgaaggttttctactctagtggctaccccaattctctccgactgtcgcagacggtccttcgttgcgcacgcaccgcgcactacctctgaaattcgacaaccgaagttcaattttacatctaacttctttcccattctctcaccaaaagcctagcttac

SEQ ID NO: 41 - DNA, 200 bp, Nannochloropsis gaditana
  misc_feature: bidirectional terminator 5
gggtgggaaggagtcggggagggtcctggcagagcggcgtcctcatgatgtgttggagacctggagagtcgagagcttcctcgtcacctgattgtcatgtgtgtataggttaagggggcccactcaaagccataaagacgaacacaaacactaatctcaacaaagtctactagcatgccgtctgtccatctttatttcct

SEQ ID NO: 42 - DNA, 213 bp, Nannochloropsis gaditana
  misc_feature: 6487 terminator
tgagatgcggaactcgcatcttatattgcaatttgatatacacagacatgacttggaaagtaaaagcaagctgggtatcggcgttacaagaaataccaggcctctggtgatgtattacactcaaaaaattaaaaggtggtagagacaatcatgcatatgcattgtcttttgcctaatgaggaaatttcgaggtgttcttcagaaaaaatctta

SEQ ID NO: 43 - DNA, 27 bp, Artificial Sequence
  misc_feature: Synthetic
  misc_feature: 5'ID sequence
tccacagcccgaacccatgagagagaa

SEQ ID NO: 44 - DNA, 27 bp, Artificial Sequence
  misc_feature: Synthetic
  misc_feature: 3'ID sequence
gcccgaatcgagttgatggcccgcaaa

SEQ ID NO: 45 - DNA, 2346 bp, Artificial Sequence
  HygR Cassette
tcataatcaaagatgagccagccacgaagctaccggagaattctgtaagaaaaatgtttaaagttgaaaatgctaacagtgaagtgatatccttttttaatggagtgttgaggtgaagtctagcatcgtaggggaaaacaggattctgtgtcttccattctactccttgataaagcgaagaaatccgacaaaaccaaagagattgttcaagtttaagatttgtaagcgtacaactatgaacttcttctctttgtaggcctgagtggtcgtatgcatacgattcatgaagtgaatcagtatcgctggattttgcttaggagtaaagcacaactaagaaaatatgctgcctggcaggcatcctgagacatgaggcaagcgacgtagcaattgaatcctaatttaagccagggcatctgtatgactctgttagttaattgatgaaccaatgagctttaaaaaaaaatcgttgcgcgtaatgtagttttaattctccgccttgaggtgcggggccatttcggacaaggttctttggacggagatggcagcatgtgtcccttctccaaattggtccgtgtggtagttgagatgctgccttaaaattctgctcggtcatcctgccttcgcattcactcctttcgagctgtcgggttcctcacgaggcctccgggagcggattgcgcagaaaggcgacccggagacacagagaccatacaccgactaaattgcactggacgatacggcatggcgacgacgatggccaagcattgctacgtgattattcgccttgtcattcagggagaaatgatgacatgtgtgggacggtctttacatgggaagagggcatgaaaataacatggcctggcgggatggagcgtcacacctgtgtatgcgttcgatccacaagcaactcaccatttgcgtcggggcctgtctccaatctgctttaggctacttttctctaatttagcctattctatacagacagagacacacagggatcatggggaagaaaccggaactgaccgctacgtccgtggagaaattccttattgagaagttcgactctgtctccgacttgatgcaactgagcgagggagaggagagtagggcgttctcgtttgacgtagggggtcggggatacgtgttgagggttaatagttgtgcggacgggttctacaaggatcggtatgtctaccgtcatttcgcctccgccgctctccccataccagaggtactggacattggggagtttagcgaatctctcacgtactgcatctcgcgccgagcccagggagtgacgttgcaagatctgcccgaaactgaattgcctgccgttttgcaacccgtggccgaggccatggacgcgatcgctgccgcagatctgtctcagacgtccggctttggaccttttgggccccagggcatcgggcagtacacgacctggcgagacttcatctgcgccattgccgatcctcacgtctatcattggcagacagtcatggatgacaccgtgtctgcatccgtggcccaagcactggacgaactcatgttgtgggccgaggattgccctgaggtcaggcacctggtgcacgcggatttcggcagcaataacgtacttacagacaatggtcggattactgctgtcatcgactggtccgaagcgatgtttggtgatagccaatacgaagtggcgaacatattcttctggcgtccctggttggcgtgcatggagcagcagacacgctactttgaacggaggcacccggagctggccggctccccacgactccgcgcctatatgttgcgtatcggactcgatcagctttaccagtctctcgtcgacggcaacttcgacgacgccgcgtgggcgcagggccgctgcgacgcgatagtccgcagcggggctgggacggtgggtcggacccaaatcgcacgccggtcggctgcggtgtggacagacggctgtgttgaggtgcttgcggactcgggcaaccgtaggccgagcacccgaccgcgtgcaaaggagtgattgaatcattgaatgaaccattgtgtgcagaatcgatttcgggagtgttgccaacacaagaaatatgcccagggttgtgtagaagtttgcgtgaatgtgatgaagggaagccatacgctgaattatcgtgacgtgtgtgagacgaagtgtcacatcatacacccaatttgagaagctgtacctattagaagaatttgtgagatacattaaaccccttttggtacgtggtataattgttatttgggaagctgtaaacacgcagatcgttcctgagattgtcaattacttttgtggtgtttcctaaaggccgcatcact

SEQ ID NO: 46 - DNA, 2400 bp, Artificial Sequence
  HygR Cassette with flanking ID sequences
tccacagcccgaacccatgagagagaatcataatcaaagatgagccagccacgaagctaccggagaattctgtaagaaaaatgtttaaagttgaaaatgctaacagtgaagtgatatccttttttaatggagtgttgaggtgaagtctagcatcgtaggggaaaacaggattctgtgtcttccattctactccttgataaagcgaagaaatccgacaaaaccaaagagattgttcaagtttaagatttgtaagcgtacaactatgaacttcttctctttgtaggcctgagtggtcgtatgcatacgattcatgaagtgaatcagtatcgctggattttgcttaggagtaaagcacaactaagaaaatatgctgcctggcaggcatcctgagacatgaggcaagcgacgtagcaattgaatcctaatttaagccagggcatctgtatgactctgttagttaattgatgaaccaatgagctttaaaaaaaaatcgttgcgcgtaatgtagttttaattctccgccttgaggtgcggggccatttcggacaaggttctttggacggagatggcagcatgtgtcccttctccaaattggtccgtgtggtagttgagatgctgccttaaaattctgctcggtcatcctgccttcgcattcactcctttcgagctgtcgggttcctcacgaggcctccgggagcggattgcgcagaaaggcgacccggagacacagagaccatacaccgactaaattgcactggacgatacggcatggcgacgacgatggccaagcattgctacgtgattattcgccttgtcattcagggagaaatgatgacatgtgtgggacggtctttacatgggaagagggcatgaaaataacatggcctggcgggatggagcgtcacacctgtgtatgcgttcgatccacaagcaactcaccatttgcgtcggggcctgtctccaatctgctttaggctacttttctctaatttagcctattctatacagacagagacacacagggatcatggggaagaaaccggaactgaccgctacgtccgtggagaaattccttattgagaagttcgactctgtctccgacttgatgcaactgagcgagggagaggagagtagggcgttctcgtttgacgtagggggtcggggatacgtgttgagggttaatagttgtgcggacgggttctacaaggatcggtatgtctaccgtcatttcgcctccgccgctctccccataccagaggtactggacattggggagtttagcgaatctctcacgtactgcatctcgcgccgagcccagggagtgacgttgcaagatctgcccgaaactgaattgcctgccgttttgcaacccgtggccgaggccatggacgcgatcgctgccgcagatctgtctcagacgtccggctttggaccttttgggccccagggcatcgggcagtacacgacctggcgagacttcatctgcgccattgccgatcctcacgtctatcattggcagacagtcatggatgacaccgtgtctgcatccgtggcccaagcactggacgaactcatgttgtgggccgaggattgccctgaggtcaggcacctggtgcacgcggatttcggcagcaataacgtacttacagacaatggtcggattactgctgtcatcgactggtccgaagcgatgtttggtgatagccaatacgaagtggcgaacatattcttctggcgtccctggttggcgtgcatggagcagcagacacgctactttgaacggaggcacccggagctggccggctccccacgactccgcgcctatatgttgcgtatcggactcgatcagctttaccagtctctcgtcgacggcaacttcgacgacgccgcgtgggcgcagggccgctgcgacgcgatagtccgcagcggggctgggacggtgggtcggacccaaatcgcacgccggtcggctgcggtgtggacagacggctgtgttgaggtgcttgcggactcgggcaaccgtaggccgagcacccgaccgcgtgcaaaggagtgattgaatcattgaatgaaccattgtgtgcagaatcgatttcgggagtgttgccaacacaagaaatatgcccagggttgtgtagaagtttgcgtgaatgtgatgaagggaagccatacgctgaattatcgtgacgtgtgtgagacgaagtgtcacatcatacacccaatttgagaagctgtacctattagaagaatttgtgagatacattaaaccccttttggtacgtggtataattgttatttgggaagctgtaaacacgcagatcgttcctgagattgtcaattacttttgtggtgtttcctaaaggccgcatcactgcccgaatcgagttgatggcccgcaaa

SEQ ID NO: 47 - DNA, 8393 bp, Artificial Sequence
  pSGE-6281
ctgtcagaccaagtttactcatatatactttagattgatttaaaacttcatttttaatttaaaaggatctaggtgaagatcctttttgataatctcatgaccaaaatcccttaacgtgagttttcgttccactgagcgtcagaccccgtagaaaagatcaaaggatcttcttgagatcctttttttctgcgcgtaatctgctgcttgcaaacaaaaaaaccaccgctaccagcggtggtttgtttgccggatcaagagctaccaactctttttccgaaggtaactggcttcagcagagcgcagataccaaatactgtccttctagtgtagccgtagttaggccaccacttcaagaactctgtagcaccgcctacatacctcgctctgctaatcctgttaccagtggctgctgccagtggcgataagtcgtgtcttaccgggttggactcaagacgatagttaccggataaggcgcagcggtcgggctgaacggggggttcgtgcacacagcccagcttggagcgaacgacctacaccgaactgagatacctacagcgtgagctatgagaaagcgccacgcttcccgaagggagaaaggcggacaggtatccggtaagcggcagggtcggaacaggagagcgcacgagggagcttccagggggaaacgcctggtatctttatagtcctgtcgggtttcgccacctctgacttgagcgtcgatttttgtgatgctcgtcaggggggcggagcctatggaaaaacgccagcaacgcggcctttttacggttcctggccttttgctggccttttgctcacatgttctttcctgcgttatcccctgattctgtggataaccgtattaccgcctttgagtgagctgataccgctcgccgcagccgaacgaccgagcgcagcgagtcagtgagcgaggaagcggaagagtttaaacagggggcatcagaatctatgccgtatatgagcttatgaatgtcatccattatctcatgtctgtcaacgcggtcctcgggtgtaacaaaacacaggaggagcgtctcacttttgaccagcagctttctgccttagagcgcaccgtccgtgtcaaagaaaatgagctcaaagaattggagcttctatctagtacgtgacattatataaggaggcaaagtgctctattaatatgttgacgagaaggtttaatacatgcagcaggtaacagatgcaggacaagtgtgtgaaatttaaccggctacttcctatgaatcaaacagaagatgcttacaatgcacaggagatcgctgaacaagaactagcaaaagagcgctctgaatataatgaggagcgtgcgcgaagggaaagaaggctacgggaacgacagcgtaatgcaaaatattgtttacaaagacaaatgcaagagcaggagaagtcgcaaggcgaaagtgcgggtggtagcatatgccaacaggaaactgaccagcaggacgagcaagacgacgaagctggtagcgaagattacgtgactacacagcaagtggaagcggacagattaagaactttgacaatgcttgtcaaaagtataactgggatcggtgatgcacaggcattgcgctcaaaacttgagcaccaaggggaggtcttgcggaagtcacaagaaattagcaaagataatcaggtgactacaagaatgatagactggtactaccccagactcgttgacatccggcgtgtcgagcgttcacatcagagatatgaaggtagatgacggtaaaagtttcctaaaatcgagcacgcgacttttttttcttcttcaatatctgagcaggatcgcttagagaagctacagaaagagcgggacatcctctggaatcaattacagagttccagatattcaccgcgccccctcaaggtctgtaacgaataataagagaggtcatcacttggccctgatcgcgatgctgtagaggttattgatgaaaggggaggaaagaatggcaggggccgtatagaaataatcctcaggattttgaaggcgtgcgtcatcctagaccaaatttgcaggaaagatgcttagaaatctcaaaattgacgcggatatttttgactaatcgacaaacatgctttcacgaccacagtccgaaggcctacttcgccagctgttgcacgacaaggaaaaagtcaaggagatcgaaaataggtgcgagtacttagcacaacttgtggcacatttgcagtgtggtttagtggagcgtttatggcctttagtaatgcgaagcaatcggaatcaccttgctgcttcgccaaagacggaaaatctcgatcgagtggcgcttcaacgtatgcttaaaaagttagaagtccgctgcttgcagctgcttgacaccaaatccatcccacaaaagcattgaaattctcaaatatggggaaccaaacgctcatccaacccatcccaagccccaggcttgcttctgtcgaatccgcagcactcagcacgcatgtgtagtatcttttggataaatcattgcaaagaaggtgtataaggctttttcccggaagcaaaagctcccgtgggcactgtagaaacaaaagtgaggtgatagttatttttcgatgcacggaacggtatatatattcgcaaagcttgtggaggctatcgctgtcctttgtttgaagcagtcttcagcgaagctgccacggagcttcgttcaggaccgtttcttggcattcaaaactctacgactatgatactatcgagcattccgcatgattacagcgcaaagcctaccaaaaagatgcggtaattcacttgcgggaccgcaatcattgtcagccatcagcgcactgtactcgtaaaaaggcgaacattgtccggtaactcgctcatgtctcacttgagctgatgtcctctctaaaataatagggtcggtcccaaactcttttaaactccgatgaaactctatgtgcactacgagcggccgcagtgatgcggcctttaggaaacaccacaaaagtaattgacaatctcaggaacgatctgcgtgtttacagcttcccaaataacaattataccacgtaccaaaaggggtttaatgtatctcacaaattcttctaataggtacagcttctcaaattgggtgtatgatgtgacacttcgtctcacacacgtcacgataattcagcgtatggcttcccttcatcacattcacgcaaacttctacacaaccctgggcatatttcttgtgttggcaacactcccgaaatcgattctgcacacaatggttcattcaatgattcaatcactcctttgcacgcggtcgggtgctcggcctacggttgcccgagtccgcaagcacctcaacacagccgtctgtccacaccgcagccgaccggcgtgcgatttgggtccgacccaccgtcccagccccgctgcggactatcgcgtcgcagcggccctgcgcccacgcggcgtcgtcgaagttgccgtcgacgagagactggtaaagctgatcgagtccgatacgcaacatataggcgcggagtcgtggggagccggccagctccgggtgcctccgttcaaagtagcgtgtctgctgctccatgcacgccaaccagggacgccagaagaatatgttcgccacttcgtattggctatcaccaaacatcgcttcggaccagtcgatgacagcagtaatccgaccattgtctgtaagtacgttattgctgccgaaatccgcgtgcaccaggtgcctgacctcagggcaatcctcggcccacaacatgagttcgtccagtgcttgggccacggatgcagacacggtgtcatccatgactgtctgccaatgatagacgtgaggatcggcaatggcgcagatgaagtctcgccaggtcgtgtactgcccgatgccctggggcccaaaaggtccaaagccggacgtctgagacagatctgcggcagcgatcgcgtccatggcctcggccacgggttgcaaaacggcaggcaattcagtttcgggcagatcttgcaacgtcactccctgggctcggcgcgagatgcagtacgtgagagattcgctaaactccccaatgtccagtacctctggtatggggagagcggcggaggcgaaatgacggtagacataccgatccttgtagaacccgtccgcacaactattaaccctcaacacgtatccccgaccccctacgtcaaacgagaacgccctactctcctctccctcgctcagttgcatcaagtcggagacagagtcgaacttctcaataaggaatttctccacggacgtagcggtcagttccggtttcttccccatgatccctgtgtgtctctgtctgtatagaataggctaaattagagaaaagtagcctaaagcagattggagacaggccccgacgcaaatggtgagttgcttgtggatcgaacgcatacacaggtgtgacgctccatcccgccaggccatgttattttcatgccctcttcccatgtaaagaccgtcccacacatgtcatcatttctccctgaatgacaaggcgaataatcacgtagcaatgcttggccatcgtcgtcgccatgccgtatcgtccagtgcaatttagtcggtgtatggtctctgtgtctccgggtcgcctttctgcgcaatccgctcccggaggcctcgtgaggaacccgacagctcgaaaggagtgaatgcgaaggcaggatgaccgagcagaattttaaggcagcatctcaactaccacacggaccaatttggagaagggacacatgctgccatctccgtccaaagaaccttgtccgaaatggccccgcacctcaaggcggagaattaaaactacattacgcgcaacgatttttttttaaagctcattggttcatcaattaactaacagagtcatacagatgccctggcttaaattaggattcaattgctacgtcgcttgcctcatgtctcaggatgcctgccaggcagcatattttcttagttgtgctttactcctaagcaaaatccagcgatactgattcacttcatgaatcgtatgcatacgaccactcaggcctacaaagagaagaagttcatagttgtacgcttacaaatcttaaacttgaacaatctctttggttttgtcggatttcttcgctttatcaaggagtagaatggaagacacagaatcctgttttcccctacgatgctagacttcacctcaacactccattaaaaaaggatatcacttcactgttagcattttcaactttaaacatttttcttacagaattctccggtagcttcgtggctggctcatctttgattatgaggcgcgccaggcattgacgcttaagttgactctgcccaaaagctgggcggagcagccgttgcttcaagtactggagctgttcatcgaatcctacaacaagaaaaagaccggtctacctcccttggacaaagactttgtccacatggaaaaagctgggtaagtccttactcgtgacagcgttccctttctccagactagacgcctaatagtgttctaatgtaccactgggacacgcctcgctgcctgtgcaccatgctccatactcaacgctgctacaggggcgtaatccttccagtcggcaacattgtgagcgacatgttgagcgatagagatgatttgtatatcagatccgggccagggcctgctcgtgggaagattgcccatctcagttcgcccccaaacgcgcacgcttcgagtgagtcgagcacaggattgttgcgctgcaaaaactatggatgcaatcagtcattttcggaagaaaacaattcagaagaggcgtgccgctttcacaaggcaccccccgtctttcatgatacgaagaaagggtggtcgtgctgcgcgaagcgagtatatgactgggacgagttccatacggtaagcgtggaagtgttcgttctcggccccaggactttgttttgaggcaattggtgtactttaattggcggataaagggaggactcacaactttcgatattcaccgtctccagatcgaggggtgcaccacaggacggcacagtctcatcgatccgaaggaaattttcgcgccgtcccccaccctggctgcagccgcgcaggccgagaggggagattgcagcaatacgtcaagcgctgctacagtcatcaagagcattgatgaattcaatcagtcgaatccaaatgccgccgctgcatgcaaaacagcagcctcgatgacgctggcgggcacgcgctgcaccgtcaaaccggacgggtctgccacctgtttgaacaaaggctgccaaaaggactacttgctcaaggagaatcacccctctgcatgtcggtaaggacaccgcgctcgatggaatcgtgagctttacgttcccacgccaacacttcgccatttctcctcccttcctttctttagctaccacgcagccggccccgtcttccacgacgcgggtaaatactggtcatgttgccctggaacggtcaagtacgacttcgacgactttctcaagatccctggatgcatgctcagtagtcattacgacggaagccaggagagcctggaggcgttcactagacacgccaaaacgtctgagggcacatgagaatgtgggatggggagaaagaaccacgtatccccacgaggaatggcgcattgggagcgagggggatcgacataggaagaagcaataaaaattctgctcaatacggtattttttattttttggcgtcttccgttcgtagccggcggacgaacagcgatgcaaactcgagacggacagtgccccacggtcttcgttcgaaaacatcattgccaacaacctcgcacacttacttccaggatcctataaatatcttacaaccaccatccgcctcttccttctcacgcgcatggataatcaacgccacgattcacaccgttgcctggacatttcccccccatgacgggtaatcctacccgtttccttccagcgttccccttctcttccattcgaacttgaatgcactttacttatttctcttgtgagcatcgtgcatccgcttgctggcaacggcaatgggaatgataatcacaagcaggatcgccaggattgccagtcccataaccattttcatctagatcgtatggagcaaaggaagagagagggggtaagggcgagaagatcgcaatgaaaagggatgacggcccacgccgcctcctgcgacttccaatcgtccgaggtttacacacatggcacagccagaaacacccccggcataggagcaggataggggtaagacaaccaagcacgtactcggagctgtttccagcacatctgtttaaacgacgaaagggcctcgtgatacgcctatttttataggttaatgtcatgataataatggtttcttagacgtcaggtggcacttttcggggaaatgtgcgcggaacccctatttgtttatttttctaaatacattcaaatatgtatccgctcatgagacaataaccctgataaatgcttcaataatattgaaaaaggaagagtatgagtattcaacatttccgtgtcgcccttattcccttttttgcggcattttgccttcctgtttttgctcacccagaaacgctggtgaaagtaaaagatgctgaagatcagttgggtgcacgagtgggttacatcgaactggatctcaacagcggtaagatccttgagagttttcgccccgaagaacgttttccaatgatgagcacttttaaagttctgctatgtggcgcggtattatcccgtattgacgccgggcaagagcaactcggtcgccgcatacactattctcagaatgacttggttgagtactcaccagtcacagaaaagcatcttacggatggcatgacagtaagagaattatgcagtgctgccataaccatgagtgataacactgcggccaacttacttctgacaacgatcggaggaccgaaggagctaaccgcttttttgcacaacatgggggatcatgtaactcgccttgatcgttgggaaccggagctgaatgaagccataccaaacgacgagcgtgacaccacgatgcctgtagcaatggcaacaacgttgcgcaaactattaactggcgaactacttactctagcttcccggcaacaattaatagactggatggaggcggataaagttgcaggaccacttctgcgctcggcccttccggctggctggtttattgctgataaatctggagccggtgagcgtgggtctcgcggtatcattgcagcactggggccagatggtaagccctcccgtatcgtagttatctacacgacggggagtcaggcaactatggatgaacgaaatagacagatcgctgagataggtgcctcactgattaagcattggtaa

SEQ ID NO: 48 - DNA, 5712 bp, Nannochloropsis gaditana
  misc_feature: acyl-CoA oxidase gene, genomic sequence
atgacgaccgccaatgcccgtttgtcgaggctcaaagatcatttagcagagacgggggctgtggcgcgcgcggtacgtgtggagtcttgctttcttcagggggggtcccggggggggggcgagtcagacaaagggtagagcgtactggaaggacagacagatgctggcatgaccctgcatccagaacacacatttaataattgagggtctggtgatcgaggggctcggcaaccgcgcggctgctagcacgtgacacggttttttacctctactgttccacaatcaacccctacttccccttctccctccctctttccctccctcccctacgttaattttccctcccgctgtactatatcgcttcactttcagccgattagctcctctgccatcaatgccacgccttttgcggcgaggacgacgcataccatggagcgcatggcaagggaacgagccaaggcctccttccccgtccgagacatgacgtacttcttggacggcgggaggagcatgaccgaggtcaaggtgggtgaaataaaaacataaaaagagaataaacaacgaaaggcgaggtctttgggggatgcctgaatacgtaggcaaccgtactgatcgttttggacccttcttctcttggggccgatggcccacaggagggcatgatggcggacttggcggcgaatccggtctttacggacccagaatggaacgacttgaacagagatcaggtagggatatgggtgattggccggaaggtggggaaggagggggaggtgccccttgtgagcttgccctgtggtcggagcgcttccctcgatcaacccctccctctcccttccccttcccccctctggctagatccgtgaacgcaccatctctcgactgagagctgcgtacaagctcctgatccgagacggtgccgatgtcagccgccggaatgcccggcttgagattcacgccctccatgacttgggtagcccttcctccctccctccctccctccctcccttgctccctacctcctccccgtgtcctcaccttcgttttttccaagcatttattacttttcagtttcatgtggacgatcatcaaaatgatgccttcctcgcccgacgcgattggtcctccctccctccctctttctctccctccctccctccctccctccctttgcagggtggtacgtgcggcagggtgtgcatttcggcctctttatgggcgccttggccgggcaggggagcgacgaacaacgcgctgagtggctgcccaggaccatgatgtgtgaggtaggagggagggagggagggagggagggaggggaaggacaaacaggctggtggaaaccacttgcaggaaggtttgggaatgtacttcggtctgtccaatccgccatacagcattttcattcctcccctccctccctcccccccctccttcctgctctagatctacgggtgcttcgggatgacggagttggggcacggctcattcttgcggggcctggagaccacagcgatgtacgacaaggtaggtacggagcgagggagggagcgagggagggagcaagggagggagggagcgagggagggagggagacagggaccgacggagggacgctaccgaccggttgtggttgttctctcctttccgtacaggacacgcaagaatttgtaatcaattcccccactgacacaagcaccaaatggtaggtgccctccctccctccctccctccctcgcctccctgtcccctgcgaccatccatccttcctccctccctccctccctccctccctccaggtggatcggtgcggccgggcagacggccacacattcggtggttttcgcccgcctcctccttccctcaggggacgacatgggtgtgcacaacttcatcatacccctccgggatatggaaacgcacttgcccctccctggcatccacattggtacctacctccctccctacctgcctccctccctccctcccgccctgctcattcctctggctccctctctaattgtcgaaaaaaatatgcgaagacttgtgacaacgtcgagccgcacgcttacttcctctcctcctccccctcctcccctccttcccgccctccttcctcccctccttcctcccctcccttcctcgccctccttcctccccctccgttccccctcttcctccccctccgttcccccctccccaggcgatttgggggccaagatgggcttgaatggcatcgacaacgggtggatgcaatttgaccacgtccgcgtgccccgggacaacatgctttgtcgctacgcacaggtgcccctccctccctccctccctccctccctccctcttttcctccctccctccctacctccttcctcctttctcgctttgtgacacacacacaccctttcgggtctcccccccgcgctcagctccctgccttctctccctccctccctccctccctcgatccctccctccctccctccctccctccctccccccctcccaggtcaccccggaggggaaatacatccgtcctcccaggaaggagatggcttacggcgctctcatcggcactcgggcggctctggtcaagacagccgtggactttcaaaaaaaggtgggtcctccctccctccctccctccctccctccctccctccctcccttctttttcctgttgcatgctttctactcttgtcctctgttatttgtgcctttttcccctccctctctccctccctccctcctttcactgacaacgacggcgtgtgtaccgaccacccttccctccctccctccctccctccctccctccctccctcccccaggccctcatgatcgggatccgctacaccgccctccggacacagggcgtggtggaggaaggccaaagggaagagaccgccatcatcgactaccccatccaccgggacaaactcctgaaactcttggcaagccccgccctccctccctccctccctccctccctccctctttcccgtcctgccgctccacgccacggcctgctactgacccccaccacctcctcctccctccctccctccctccctccctcaggcggccgcctacgcctggcacttccaagccgcctacgttctccacctgaacgattccttggaggaggggctcgaggcgggggacctctccatcctcaaggatgtgcatgggaccatggctggtaccccccgccctccctccctccctccctccctccctccctgtttcccgccctgtggggcctcgcagccttttgcatccgcttccccgtgacgctgccctccctccctccctcgctccctccctcccgccctccctccaggcctcaaggctttcggaacctggttcacgtacaacacgatcgaggcctgccggcaagtgtgcgggggccacgggtacagcaagtacaacggcctctccaacaccctccaggtccctccttccctccctccctccctccctccctccctcccttcctccctttcctcctttcttgtcgtatgatcggagcgacgcactgcgtgacgcgttcctacttccttgtggtgctgccgatttcatccctacctccctccttccctccctcccttcctccctcccttcctccctccctcaggactttgctgtcatgtgcacctgggagggcgacaacaccgtgatggctctacagacggcgcggtatctagttcggtcctacgagaaggcgaagcgggggggcggtagggagggagggagggagggagggagggagggagggagggaaagaggaggaaagaaacggccaaagaaaggagaacatccattgccttcacctcggtcaaatcctaaacactgcagcgcacatgaaattaaatcaacccctccctccctccctccctcctctctccctccatccctccctccctccttccctcgttcagagaccctggcaggctccgtctcatacctgcaggatgcgcatcccccggcttggcgggcgaggtctgcggaggacttgatgaacatggaagtgcagatggaggtagggaccgaggaagggatagggaggggggaggaagggccgggccgggagggggggagggagtgaaggaggggaggacggaaggaaagagggagggagggagggagggagggagagagggagagagtaggaaatgagggggataagagatgagaatagcacggtttgttcaatgtgcagcagagatgatcctctccgcacctcctccactccctttcaccccttccatccctccctccctcgctccctcccttcctccctccttccaggcctggcgggccctcctagccgccaaggtctccagagcctcagagcgggtcttggcaaggcaggcggcgttgcgggggaacgaggcgcaggtagggagggagggagggagggagggcgggagggagggagggagggagggaaggcgaggaggacggtgaggggaaaagatctcctgaaaattgatggggacagagtcgttcaaggagtgtcaaaccagaatttcatgtatgcacacccgtccttccttccctccatccctccctccctccctccctggcaggccttcaacgagcatcaggtggagcttttcgagtgcgccaagacccatgtctacttcaatgtggcggcgcggtttgccgaggcggtcgtggaggtcgggtggaagaaagggagggagggagggagggagggagggagggagggagggagggggaaagattgaaagcctaccttgtcgtctctttgcatacgcgcctatttgtccagcggttccaacgttttcttttcctccctccctccctcatttcctccctccctccctccctcatttcctccctccctctctccctccctccctccctccctccctccctccctccctccctccctccctccctccctccaggccggcaccacccaccccgccctggcccctgtcctcgcccgcctctgccacctcttctctctctcgagccttctagaagacgaagcctccctgctcgccagcggtttcgcctccgcggggcagatgcagctcattcgcgaggtggggaaggagggagagagggagagacggagggagggacggaaggagggagggagggccatgtccatgtcgctgctaaagggcctgacggacaagaaatgggaagatccaatcgccgtgactcatccctccctccctccgtcccgccctccctcccgccctccctccaggccgtgggcgccctcctcctcgccctccgcccggacgcggtggcccttgtcgacgccttcaactattccgacgaagttttgaactcacatttaggcaccgccaacggcgatatttatacgggctacctccaacaggtgcagcgcctcgtccctgagaacaaggtccgcccgctcgccctccctccctccctccctcccgccctcccgccctccctccctcttcttctcttccggggccttgtgcccgtgttgacgacgagcacttgacccgcttctcgctttcctcgatccctccctcctacttcccctctttttccctccccccttctcctccctccttcccttccaattacgtcctcttcccctccttcatccagctggccgtcgccccctacatcatgagggaggtgaagcctttaatgcaaggagcagacctgatctccacggacgaggaggaggactga

SEQ ID NO: 49 - DNA, 23 bp, Nannochloropsis gaditana
  misc_feature: aco2-CRISPR target sequence including PAM sequence
ggcgaggacgacgcataccatgg

SEQ ID NO: 50 - RNA, 103 nt, Artificial Sequence
  Entire chimeric guide RNA for targeting N. gaditana aco2 gene
ggcgaggacgacgcauaccaguuuuagagcuagaaauagcaaguuaaaauaaggcuaguccguuaucaacuugaaaaaguggcaccgagucggugcuuuuuuu

SEQ ID NO: 51 - DNA, 120 bp, Artificial Sequence
  aco2 sense oligonucleotide
taatacgactcactataggcgaggacgacgcataccagttttagagctagaaatagcaagttaaaataaggctagtccgttatcaacttgaaaaagtggcaccgagtcggtgcttttttt

SEQ ID NO: 52 - DNA, 120 bp, Artificial Sequence
  aco2 reverse complement oligonucleotide
aaaaaaagcaccgactcggtgccactttttcaagttgataacggactagccttattttaacttgctatttctagctctaaaactggtatgcgtcgtcctcgcctatagtgagtcgtatta

SEQ ID NO: 53 - DNA, 6956 bp, Artificial Sequence
  pSGE6282
ctgtcagaccaagtttactcatatatactttagattgatttaaaacttcatttttaatttaaaaggatctaggtgaagatcctttttgataatctcatgaccaaaatcccttaacgtgagttttcgttccactgagcgtcagaccccgtagaaaagatcaaaggatcttcttgagatcctttttttctgcgcgtaatctgctgcttgcaaacaaaaaaaccaccgctaccagcggtggtttgtttgccggatcaagagctaccaactctttttccgaaggtaactggcttcagcagagcgcagataccaaatactgtccttctagtgtagccgtagttaggccaccacttcaagaactctgtagcaccgcctacatacctcgctctgctaatcctgttaccagtggctgctgccagtggcgataagtcgtgtcttaccgggttggactcaagacgatagttaccggataaggcgcagcggtcgggctgaacggggggttcgtgcacacagcccagcttggagcgaacgacctacaccgaactgagatacctacagcgtgagctatgagaaagcgccacgcttcccgaagggagaaaggcggacaggtatccggtaagcggcagggtcggaacaggagagcgcacgagggagcttccagggggaaacgcctggtatctttatagtcctgtcgggtttcgccacctctgacttgagcgtcgatttttgtgatgctcgtcaggggggcggagcctatggaaaaacgccagcaacgcggcctttttacggttcctggccttttgctggccttttgctcacatgttctttcctgcgttatcccctgattctgtggataaccgtattaccgcctttgagtgagctgataccgctcgccgcagccgaacgaccgagcgcagcgagtcagtgagcgaggaagcggaagagtttaaacatatatgagtgcgattcgatgcaagggggggaggggggaaggttcgaaagccgtcgaccttctggataaagtacggagtttgtcagccctccctcgcggtgtggccacgataagtaacaaagcatgtaataaggatgcagcctggagattgatgtgcgatcagaatcatcatgacacgtcaaaacacaggcggcgacatggcgagacccgtgaccaacgtgatagagaaacctgtcctgaggcacgtattgtaaacaacccagagatgtcagaaaaacaaaggcatgtcaacgctgtttaaggcagcatctccaggcaatctttcctccgtgaggtggatctatcctccctcctttctctttaaaagcggccgtccgtccgtggtcgccttttccccactctccctgcacgttctgcccacacgtcccttccatcaccacaaaaagagcacattattctgtcatgtacatacacagctgggacgggacgttgcggagggcgggccggggcttgtggcccgggcaacaggacacctttccctgcccttaaaccccgactgtctcctttttgctcgtggagccatgaccttcctcctaactaccccacatcccgatacctgtctatggtggaaagaagagtcctcattgcgcggtgtctgcacgagcaattacgaaagttaacttctccagccccagccctagcgggcctctgtcgccctatatccctcatgagagccatggcagcctcttgctgcgcccctttccatcctttttctacctcaagtcattttaagatacattttcaagggaacgtgggggattgttgtgcgatcgaggcttctattctccgacacactttgaatgagagcggtgcctctcctagtgagctcatttgcaacaggagaaggccctcctccctttacaaatataaagtgcccctggtcgtctccttgccactgtataccattgctgtgtctttgattgaaaaaaatcgtaaccatggctttggagggccccatcgccacgtttgcgcgagaacagcaatacttatcccttttagttccttcctttctcgcatttgtggtagccccgtgcgcgcggggaaatgagttaaagtcatgtgcaccagaaactacacattccattttttaccacagcataaaagccttattttctactgctacccagagcggggccaccatttctacggtgacacccgccaaaataaaggacatatgcccgtgtgacgtatcgcggggctatggaggggtacctgcgagttgctgttgaagtgcccccccccccccgtatgtaaaaccacgtccttcggtccgtacccatctcaccgcacattgattacactttacggcagaaatgacgaccgccaatgcccgtttgtcgaggctcaaagatcatttagcagagacgggggctgtggcgcgcgcggtacgtgtggagtcttgctttcttcagggggggtcccggggggggggcgagtcagacaaagggtagagcgtactggaaggacagacagatgctggcatgaccctgcatccagaacacacatttaataattgagggtctggtgatcgaggggctcggcaaccgcgcggctgctagcacgtgacacggttttttacctctactgttccacaatcaacccctacttccccttctccctccctctttccctccctcccctacgttaattttccctcccgctgtactatatcgcttcactttcagccgattagctcctctgccatcagcggccgctccacagcccgaacccatgagagagaatcataatcaaagatgagccagccacgaagctaccggagaattctgtaagaaaaatgtttaaagttgaaaatgctaacagtgaagtgatatccttttttaatggagtgttgaggtgaagtctagcatcgtaggggaaaacaggattctgtgtcttccattctactccttgataaagcgaagaaatccgacaaaaccaaagagattgttcaagtttaagatttgtaagcgtacaactatgaacttcttctctttgtaggcctgagtggtcgtatgcatacgattcatgaagtgaatcagtatcgctggattttgcttaggagtaaagcacaactaagaaaatatgctgcctggcaggcatcctgagacatgaggcaagcgacgtagcaattgaatcctaatttaagccagggcatctgtatgactctgttagttaattgatgaaccaatgagctttaaaaaaaaatcgttgcgcgtaatgtagttttaattctccgccttgaggtgcggggccatttcggacaaggttctttggacggagatggcagcatgtgtcccttctccaaattggtccgtgtggtagttgagatgctgccttaaaattctgctcggtcatcctgccttcgcattcactcctttcgagctgtcgggttcctcacgaggcctccgggagcggattgcgcagaaaggcgacccggagacacagagaccatacaccgactaaattgcactggacgatacggcatggcgacgacgatggccaagcattgctacgtgattattcgccttgtcattcagggagaaatgatgacatgtgtgggacggtctttacatgggaagagggcatgaaaataacatggcctggcgggatggagcgtcacacctgtgtatgcgttcgatccacaagcaactcaccatttgcgtcggggcctgtctccaatctgctttaggctacttttctctaatttagcctattctatacagacagagacacacagggatcatggggaagaaaccggaactgaccgctacgtccgtggagaaattccttattgagaagttcgactctgtctccgacttgatgcaactgagcgagggagaggagagtagggcgttctcgtttgacgtagggggtcggggatacgtgttgagggttaatagttgtgcggacgggttctacaaggatcggtatgtctaccgtcatttcgcctccgccgctctccccataccagaggtactggacattggggagtttagcgaatctctcacgtactgcatctcgcgccgagcccagggagtgacgttgcaagatctgcccgaaactgaattgcctgccgttttgcaacccgtggccgaggccatggacgcgatcgctgccgcagatctgtctcagacgtccggctttggaccttttgggccccagggcatcgggcagtacacgacctggcgagacttcatctgcgccattgccgatcctcacgtctatcattggcagacagtcatggatgacaccgtgtctgcatccgtggcccaagcactggacgaactcatgttgtgggccgaggattgccctgaggtcaggcacctggtgcacgcggatttcggcagcaataacgtacttacagacaatggtcggattactgctgtcatcgactggtccgaagcgatgtttggtgatagccaatacgaagtggcgaacatattcttctggcgtccctggttggcgtgcatggagcagcagacacgctactttgaacggaggcacccggagctggccggctccccacgactccgcgcctatatgttgcgtatcggactcgatcagctttaccagtctctcgtcgacggcaacttcgacgacgccgcgtgggcgcagggccgctgcgacgcgatagtccgcagcggggctgggacggtgggtcggacccaaatcgcacgccggtcggctgcggtgtggacagacggctgtgttgaggtgcttgcggactcgggcaaccgtaggccgagcacccgaccgcgtgcaaaggagtgattgaatcattgaatgaaccattgtgtgcagaatcgatttcgggagtgttgccaacacaagaaatatgcccagggttgtgtagaagtttgcgtgaatgtgatgaagggaagccatacgctgaattatcgtgacgtgtgtgagacgaagtgtcacatcatacacccaatttgagaagctgtacctattagaagaatttgtgagatacattaaaccccttttggtacgtggtataattgttatttgggaagctgtaaacacgcagatcgttcctgagattgtcaattacttttgtggtgtttcctaaaggccgcatcactgcccgaatcgagttgatggcccgcaaaggcgcgccgagcatgaccgaggtcaaggtgggtgaaataaaaacataaaaagagaataaacaacgaaaggcgaggtctttgggggatgcctgaatacgtaggcaaccgtactgatcgttttggacccttcttctcttggggccgatggcccacaggagggcatgatggcggacttggcggcgaatccggtctttacggacccagaatggaacgacttgaacagagatcaggtagggatatgggtgattggccggaaggtggggaaggagggggaggtgccccttgtgagcttgccctgtggtcggagcgcttccctcgatcaacccctccctctcccttccccttcccccctctggctagatccgtgaacgcaccatctctcgactgagagctgcgtacaagctcctgatccgagacggtgccgatgtcagccgccggaatgcccggcttgagattcacgccctccatgacttgggtagcccttcctccctccctccctccctccctcccttgctccctacctcctccccgtgtcctcaccttcgttttttccaagcatttattacttttcagtttcatgtggacgatcatcaaaatgatgccttcctcgcccgacgcgattggtcctccctccctccctctttctctccctccctccctccctccctccctttgcagggtggtacgtgcggcagggtgtgcatttcggcctctttatgggcgccttggccgggcaggggagcgacgaacaacgcgctgagtggtttaaacgacgaaagggcctcgtgatacgcctatttttataggttaatgtcatgataataatggtttcttagacgtcaggtggcacttttcggggaaatgtgcgcggaacccctatttgtttatttttctaaatacattcaaatatgtatccgctcatgagacaataaccctgataaatgcttcaataatattgaaaaaggaagagtatgagtattcaacatttccgtgtcgcccttattcccttttttgcggcattttgccttcctgtttttgctcacccagaaacgctggtgaaagtaaaagatgctgaagatcagttgggtgcacgagtgggttacatcgaactggatctcaacagcggtaagatccttgagagttttcgccccgaagaacgttttccaatgatgagcacttttaaagttctgctatgtggcgcggtattatcccgtattgacgccgggcaagagcaactcggtcgccgcatacactattctcagaatgacttggttgagtactcaccagtcacagaaaagcatcttacggatggcatgacagtaagagaattatgcagtgctgccataaccatgagtgataacactgcggccaacttacttctgacaacgatcggaggaccgaaggagctaaccgcttttttgcacaacatgggggatcatgtaactcgccttgatcgttgggaaccggagctgaatgaagccataccaaacgacgagcgtgacaccacgatgcctgtagcaatggcaacaacgttgcgcaaactattaactggcgaactacttactctagcttcccggcaacaattaatagactggatggaggcggataaagttgcaggaccacttctgcgctcggcccttccggctggctggtttattgctgataaatctggagccggtgagcgtgggtctcgcggtatcattgcagcactggggccagatggtaagccctcccgtatcgtagttatctacacgacggggagtcaggcaactatggatgaacgaaatagacagatcgctgagataggtgcctcactgattaagcattggtaa

SEQ ID NO: 54 - DNA, 1767 bp, Nannochloropsis gaditana
  misc_feature: aco2 target upstream homology arm
atatatgagtgcgattcgatgcaagggggggaggggggaaggttcgaaagccgtcgaccttctggataaagtacggagtttgtcagccctccctcgcggtgtggccacgataagtaacaaagcatgtaataaggatgcagcctggagattgatgtgcgatcagaatcatcatgacacgtcaaaacacaggcggcgacatggcgagacccgtgaccaacgtgatagagaaacctgtcctgaggcacgtattgtaaacaacccagagatgtcagaaaaacaaaggcatgtcaacgctgtttaaggcagcatctccaggcaatctttcctccgtgaggtggatctatcctccctcctttctctttaaaagcggccgtccgtccgtggtcgccttttccccactctccctgcacgttctgcccacacgtcccttccatcaccacaaaaagagcacattattctgtcatgtacatacacagctgggacgggacgttgcggagggcgggccggggcttgtggcccgggcaacaggacacctttccctgcccttaaaccccgactgtctcctttttgctcgtggagccatgaccttcctcctaactaccccacatcccgatacctgtctatggtggaaagaagagtcctcattgcgcggtgtctgcacgagcaattacgaaagttaacttctccagccccagccctagcgggcctctgtcgccctatatccctcatgagagccatggcagcctcttgctgcgcccctttccatcctttttctacctcaagtcattttaagatacattttcaagggaacgtgggggattgttgtgcgatcgaggcttctattctccgacacactttgaatgagagcggtgcctctcctagtgagctcatttgcaacaggagaaggccctcctccctttacaaatataaagtgcccctggtcgtctccttgccactgtataccattgctgtgtctttgattgaaaaaaatcgtaaccatggctttggagggccccatcgccacgtttgcgcgagaacagcaatacttatcccttttagttccttcctttctcgcatttgtggtagccccgtgcgcgcggggaaatgagttaaagtcatgtgcaccagaaactacacattccattttttaccacagcataaaagccttattttctactgctacccagagcggggccaccatttctacggtgacacccgccaaaataaaggacatatgcccgtgtgacgtatcgcggggctatggaggggtacctgcgagttgctgttgaagtgcccccccccccccgtatgtaaaaccacgtccttcggtccgtacccatctcaccgcacattgattacactttacggcagaaatgacgaccgccaatgcccgtttgtcgaggctcaaagatcatttagcagagacgggggctgtggcgcgcgcggtacgtgtggagtcttgctttcttcagggggggtcccggggggggggcgagtcagacaaagggtagagcgtactggaaggacagacagatgctggcatgaccctgcatccagaacacacatttaataattgagggtctggtgatcgaggggctcggcaaccgcgcggctgctagcacgtgacacggttttttacctctactgttccacaatcaacccctacttccccttctccctccctctttccctccctcccctacgttaattttccctcccgctgtactatatcgcttcactttcagccgattagctcctctgccatca

SEQ ID NO: 55 - DNA, 755 bp, Nannochloropsis gaditana
  misc_feature: aco2 target downstream homology arm
gagcatgaccgaggtcaaggtgggtgaaataaaaacataaaaagagaataaacaacgaaaggcgaggtctttgggggatgcctgaatacgtaggcaaccgtactgatcgttttggacccttcttctcttggggccgatggcccacaggagggcatgatggcggacttggcggcgaatccggtctttacggacccagaatggaacgacttgaacagagatcaggtagggatatgggtgattggccggaaggtggggaaggagggggaggtgccccttgtgagcttgccctgtggtcggagcgcttccctcgatcaacccctccctctcccttccccttcccccctctggctagatccgtgaacgcaccatctctcgactgagagctgcgtacaagctcctgatccgagacggtgccgatgtcagccgccggaatgcccggcttgagattcacgccctccatgacttgggtagcccttcctccctccctccctccctccctcccttgctccctacctcctccccgtgtcctcaccttcgttttttccaagcatttattacttttcagtttcatgtggacgatcatcaaaatgatgccttcctcgcccgacgcgattggtcctccctccctccctctttctctccctccctccctccctccctccctttgcagggtggtacgtgcggcagggtgtgcatttcggcctctttatgggcgccttggccgggcaggggagcgacgaacaacgcgctgagtg

SEQ ID NO: 56 - DNA, 5607 bp, Artificial Sequence
  Cas9 with FLAG tag, nuclear localization sequences, peptide linker, and introns, codon optimized for expression in Parachlorella
atgcccaagaagaagcggaaagtcggggactacaaggacgacgatgacaaactggagcctggggagaagccctataagtgtcctgagtgcgggaagagcttcagccaatctggagcactgacaaggcaccagaggacacatacacgcgacaagaagtacagcatcgggctggatatcgggaccaattctgtgggatgggccgtgattaccgacgagtataaggtgcccagcaagaagttcaaggtgctggggaacacagaccgccacagcattaagaagaacctgatcggggcgctgctgtttgattctggagagacagcagaggcaaccgtgagtgagaacagttttcagatcgaatagcacccccccgcctctgcagcagtcgcataccggctgcagtaatagcttggttcaacggcgacctgaacaagtactgtagtttctatgcatacgaactttatcgaatagaatcacgcttgggtatcgatcataccttagcgctcaatttcattggctgctacagaccatattttcctcttcacttgttgcagcgcctgaaaagaacagcaagaaggcgctacacccgccgcaagaataggatttgctacctgcaagagatcttcagcaacgagatggccaaggtggacgacagcttcttccatagactggaggagtcgttcctggtggaggaggataagaagcacgagaggcaccccatcttcggtgagaagagtttggctaccaaatctatcttttcatatcacatataccgcctgatattctgaggtggtggcttttgtctttttctttcagtatttttcttcgttgggaacctaccgcgagggcattcattgtggcggatctgtaagtgcgaccaggctgtatccaatattttttcctatcgcagggaacattgtggatgaggtggcctaccacgagaagtaccccacaatctaccacctgcgcaagaagctggtgagaatctctgcttgtcgaatgtgtccagttgtgtcttgaatcctggcaagatgttcttttcaccatccgtcctgcaaaagtgtcagaagtagcatctctcgatcgcgttgtcacttcaacgcctccgcaactccccccgttgtgaatcctgtggtcatggctcagcttttcagatctctacctgcatgttgtttgcctgtctcagtcctgcctgcacaaatcatcgcccttgtttactccttgcaatcacggattgtgtgcaggtggacagcacagataaggccgatctgaggctgatctacctggcattggcccacatgatcaagtttagggggcacttcctcatcgagggggatttgaaccccgacaacagcgatgtggacaagctgttcatccagctggtgagtggagggctggggtttgggggtggggggtggggagggaggcacggatggtgttttctcatgtccaaccgtggttcatgcaaccgaacagcagtttcacaagatggttccaacagggtgctccatttctccctgacaaaacctcgtgcggtccatctggtatagctgggttagtagggggttgtgggctgtccacagtcagtgcgaagcaggctctattgagcgtgtgctagtgtgtgctgtgctgattggcattttgttgggccgagtgttaggattagggtaaatcaccctaattaaccttacataataggactgtatgcaaatttgttttccaaaaactctacccagcgtggtcagactgcatgcactgtggagcatgcatggggctgaccctgttgatcctgctcattctgcttcctccaggtgcagacctacaaccagctgtttgaggagaaccccatcaacgcatctggggttgacgcaaaggccattctgtctgcaaggtaggtgcaggaagaagtgaatgatgcacacatggtggaatcgtgatacaagcagcagcaagtgttggaccaagacatgtgcgtgctttgctgctgccaagctggcactgcaccaggtcgtgcattgatctgcacatttgatatactgtgagagtcagacgacgtcctttcagagcctgtgtgtgattctccaggggttaacacgagtttcctttctgccagtgagtcaccctctcgctgctcgctcctggtgcaggctgagcaagtcaaggagactggagaacctgatcgcccaattgcctggagagaagaagaacgggctgttcgggaacctgatcgcattgtctctggggttgacccccaacttcaagagcaacttcgacctggcagaggacgcaaaactgcagctgagcaaggacacctacgacgatgatctggacaacctgctggcccagattggagatcagtacgcagacctgttcctggcagccaagaatctgagcgacgcaattctgctgagcgacattctgcgcgtgaacaccgagatcaccaaggcacctctgagcgcaagcatgatcaagaggtacgacgagcaccaccaagacctgacactgctgaaagcactggtgagacagcagctgcctgagaagtacaaggagatcttcttcgaccagagcaagaacgggtacgctgggtacattgatggaggagcaagccaagaggagttctacaagttcatcaagcccatcctggagaagatggacgggacagaagagttgctggtgaagctgaatcgcgaggatctgctgaggaagcagaggacattcgacaatgggagcatcccacaccagatccatctgggagagctgcacgcaattctgaggagacaagaggacttctacccgttcctgaaggacaatcgcgagaagatcgagaagatcctcacgttccgcatcccgtactatgtgggacctctggcaagggggaactctagatttgcctggatgacccgcaagagcgaggagacaattacaccctggaacttcgaggaggtggtggataaaggggcatctgcacagagcttcatcgagaggatgaccaacttcgacaagaacctgcccaacgagaaggtactgcctaagcattcactgctgtacgagtacttcaccgtgtacaacgagctgaccaaggtgaagtacgtgacagaggggatgaggaagccagcatttctgagcggagagcaaaagaaggccatcgtggatctgctgttcaagaccaaccgcaaggtgaccgtgaagcagctgaaggaggactacttcaagaagatcgagtgcttcgacagcgtggagatttctggagtggaggaccgcttcaacgcatctttggggacataccacgacctgctgaagatcatcaaggacaaggacttcctggacaacgaggagaacgaggacatcctggaggacattgtgctgacactgaccctgttcgaggatagggagatgatcgaggagcgcctgaagacatacgcacacctgtttgacgacaaggtgatgaagcagctgaagaggaggcgctatactggatggggaaggctgtcaaggaagctgattaacgggatccgcgacaagcagagcgggaagacaattctggacttcctgaagagcgacgggttcgcaaaccgcaacttcatgcagctgatccacgacgatagcctgaccttcaaggaggacatccagaaggcccaagtgtctggacaaggggatagcctgcatgagcacatcgcaaatctggctgggtcacccgcaatcaagaagggaattctgcagaccgtgaaggtggtggatgagctggtgaaggtgatgggaaggcacaaacccgagaacatcgtgatcgagatggcaagggagaaccagacaacccagaagggacagaagaactctagggagcgcatgaagcgcatcgaggagggaattaaggagctgggaagccagatcctgaaggagcatcctgtggagaacacccaactgcagaacgagaagctgtacctgtactacctgcagaacgggagggacatgtacgtggatcaagagctggacatcaaccgcctgagcgactatgacgtggaccacattgtgcctcagtcgttcctgaaggacgacagcatcgacaacaaggtgctgacaaggagcgacaagaatcgcggaaagagcgacaacgtgccttcagaagaggtggtgaagaagatgaagaactactggcgccagctgctgaacgcaaagctgattacacagcgcaagttcgacaacctgaccaaggcagagaggggaggactgtcagaactggataaggccgggttcatcaagaggcaactggtggagacacgccagatcacaaagcatgtggcccagattctggacagccgcatgaacaccaagtacgacgagaacgacaagctgatccgcgaggtgaaggtgattaccctgaagagcaagctggtgagcgactttcgcaaggacttccagttctacaaggtgcgcgagatcaacaactaccaccacgcacacgacgcctacctgaatgcagttgtgggaacagccctgatcaagaagtaccccaagctggagagcgagttcgtgtatggggactacaaggtgtacgacgtgcgcaagatgatcgccaagtctgagcaagagatcgggaaggcaaccgccaagtacttcttctacagcaacatcatgaacttcttcaagaccgagatcaccctggccaatggggagattaggaagagacccctgatcgagaccaacggagagactggagagatcgtgtgggataaggggagggactttgcaacagtgcgcaaagtgctgagcatgcctcaagtgaacatcgtgaagaagaccgaggtgcagactgggggattctcaaaggagagcattctgcccaagcgcaacagcgataagctgattgcacgcaagaaggactgggaccccaagaagtatggggggtttgatagccccaccgtggcatattctgtgttggttgtggccaaggtggagaaggggaagagcaagaagctgaagagcgtgaaggagctgctggggatcaccattatggagaggagcagcttcgagaagaaccccatcgacttcctggaggcaaaggggtataaggaggtgaagaaggacctgatcatcaagctgcccaagtacagcctgttcgagctggagaatgggaggaagaggatgctggcatctgctggagaactgcagaaggggaatgagttggcactgcctagcaagtacgtgaacttcctgtacctggccagccactacgagaagctgaagggatcacccgaggacaatgagcagaagcagctgtttgtggagcagcacaagcactacctggacgagatcatcgagcagatcagcgagttcagcaagcgcgtgattctggcagacgcaaacctggataaggtgctgagcgcctacaacaagcaccgcgataagcccattcgcgagcaagcagagaacatcatccacctgttcaccctgaccaacctgggagcacctgcagcattcaagtacttcgacaccaccatcgaccgcaagaggtacacaagcaccaaggaagtgctggacgcaaccctgattcaccagagcattactgggctgtacgagacacgcatcgacctgtcacaactgggaggggactga

SEQ ID NO: 57 - DNA, 588 bp, Parachlorella sp.
  misc_feature: RPS17 promoter
caacacctagttggtaaataccgttgctgatattgctctgtaccagtaaaagagggctgcgatgagcgtttttagtgcacttcttcaacacggaatatttttcacaaattggtatgagaaccaattttgcaaaatgttcgccctgtaaagtatcgctctgggacgatcagcttgacgtaattgtaggcgaaaagggcgttcaaagtgcagctttatgtatgaacgtcataaaatataaagcatagcacaatcactgatagaaaatatttgtgcgcattaaaactctcacttctgttgcggatacaacgacggaaatgagaagcttgtgtaagaagcaattcaagttttcattttgtcatctaaggtgtgatcctccgatattcattaccgaatgctgatctgagttggaaagatggcaatatttagctgtgcacactttgacctccaggccttggcgggaatttagtattctagctttcctattggaacgataggccagccaagtctccagcttgtatacgctacaccagcagacatgctctcaatttagctgacagtgtcttcatatttgtattatctgttgtgtct

SEQ ID NO: 58 - DNA, 455 bp, Parachlorella sp.
  misc_feature: RPS17 terminator
ggtgcgaatagtgcttcagtaaaaaagtagcaacttggtgcaatatcgtcagggtcgtgtggtctgctcgccagcaagttttttggcacaggagagcgctttttccgagtaccgccaaagttcaagcatgtgctgtgattcgctgttgcctcttatgataattgctcaaagtttccaagcattctatgtccaccctgcaccactaagttgtatggtgcttattctgcaggggatgattcatggtgcctaaaaattttgtgctgctgtcgcgtctgttttctgtcgcagtttagtgaatgtaactccaaataccaaacttttcatcacaatcatattgatgcctttgtaagtgaattacagcgttttttgccataaaaagaagtaccgtgacattggggtcgtcataacaagaagctttatgaacaagcagcttgatctacgagacttatacataa

SEQ ID NO: 59 - DNA, 2691 bp, Artificial Sequence
  BlastR gene codon optimized for Parachlorella and containing introns
atggcaaaacctctctcccaggaagagtctaccctgattgaaagggcaacagcaaccatcaacagcattcccattagcgaggactactctgttgtgagttctgagaagctgattgttgtttaacttctttgaaagctttatcgaagattctgcaagcgatgaacattgcttgtcaagaccgagagctgcatgcccacttgacatccagctttgaacggctcttcatgtttgatttgtttctgattgtaggcatctgcagcattgagctctgatggaaggatctttacaggagtgagtgcagcgtcagctgtggcagttgttggctttcgtctcagtcagtagtttgctgggattgattatggagggcacagttgcaattttgagttgcacgttgcgacaagcgtgttgacaaagcgtggtcaagccggccagtcttgccggtggcgggtggcttggtctaacttccgctctacggcaatcgttttgttcatggttacggggctggcgtgccagaaagtcctggtcagccaccctcgcttcaaagccgtagcccaacaactttgcgaatatgttcgatttgcaggtgaacgtgtaccactttacaggaggaccttgtgcagaattggtggtgttaggtacagctctgcgtgcaacaggttgcaagatgcagcgcaggtcttccctggtcaaacgatgtatgcagagttgagaggcacttgagctgggtgaatggcgtgggctcgtaggtagtgtgcagggcaggaagggcagccaattttggagttgtggtccggtgtcgttgcttcgagccttattaggactcttgctcatcaaagcgttagttgtgaataagttgatctgaaaggatgttatgtacagcaagcagcagcagttaagagtctggggagtagctgcacagggcgaggtgtcaagatgggaagggtcctgcctccttatgtgtttttccctgtaggggaggaagcctcttatgggcaatggttgggcatattttccagccagcccttctttctataggggccagggtgggcccagctcgtcttggcttccaccaccaggagagtgagggcattgaagggccataaatagtcctcccatctacgtgcaccagagggtgtcgtctaggctgtgcatgccacgaggggaaggagccaagaatgagtgtatgggttgttttcatgtttaggctgggataaaactgttttcaattgcgcctgccgggtgaaaaccacagcagcatcagcaagcttggagaaggccagcccgcccagcacaggctcacgttcccactcaggcggtcagtcgggcgggggtgtgagtcaggcaggcgagggtgtctgtgcctgacatcagcacctctgcttagccactgcagcccctggagcagggtagggcgtcatttgcagcaatcacctgctgcctcacacgtcgcagcttggaatttcaacgaccatcagcgctggggttgttgagggatcatagcagattttggtgcagcctggttgtcatgctctttgtggaatggcctctatgttcgagcaattcgttggatgttgaggtgcttggggacagagagtcgaatgatgggccagggtcaaacatgcgagcgtttggctgagtcagcggtttttgctggtcactttttcttttgtttcttatttaggtttgatggatgtgttttgtgctgctgccctgaagctgcagcagcgtgtctgccctgcgctactgcgggcaccaaggctatgtgctggtgcactcggctgcgctgcacctgtgcacctcgcactccgtccagcctccatgcagcacacgtactcacggtgtcctcctgacctgtcgtacgctattccaaacttgctcttttgctgccgctgctctcgtacacaattgctgttgattatcgatatctaatcgagcgcctgctgactgaactccgcaggtacagcagctgcagcagcagcaggaaatttgacatgcattgtggcaataggtgggtgggctctgaaggaggaggagggagcgggtgattaaacagggcctgcatgaagaggagcaggggctgcgtggacagcagggggaaggtgcagaagggagggtcaagcggggttcaggtggctgtgggtttctgcacgagcagtgaaagaagctgtatccttccacctgcttccactggcgaaaggttgaaaacaggatgtcgcagctggaaagatgttgcgctgtcaagtgcaagccatggttgagggtatgcctgtgtgcatgtgcttcttaaagttactcctgttctatggttctgggtgcttgttgtttgtggtgcagggaacgagaatagggggattttgtcaccttgcggaagatgtagacaggtgttgttggatctgcatcccgggattaaggtgagggggcatgtaagcaatggcaggcaattcaagaacgaatcattgctgcaaatgctgggatggtatgcagctgaggtatctattgccttgtattttgtctcgcattgcatcggtggtgcgttctgtggcctgaggcacagttcttgctgtttgataagggttcgactgagttgtcgtgtgtgctgtgctgcaggcaatcgtgaaggattcagatgggcagcctacagcagtgggaattagagaactgctgccttctgggtatgtgtgggaaggataa

SEQ ID NO: 60 - DNA, 531 bp, Parachlorella sp.
  misc_feature: RPS4 promoter
ccaccatgggggaggtttgaagtgtgcgcctgatataatcatacacctaaaagcaccacttgctgattgtgaagggactatgtcgtttatgacgggacgttacgctggccgatggtttgaatttggacgctgtggtagaatgttatatggacgtaaaggttggcatattgaaaatcgtcttcacaggcaaacttctagacgtgtgacccaccggtaaaacgacaagcgtggcgcgtcgattgcgctttgaacgtcgtttgttggactccagatgaacctcaaaatcaaagcggtgattgacgaaaatcaaatgacagcccgcaaaatttcatcagccttcggatcggattctcagaatctgattgtccctgctggctacatttatgaaatttcgtacattttggcagaaatgtcccaataccatagcactgccgcctgagctcacccgagcaatgcatactgggtacctcgcccatctcgccctctttccaagcccagtgctgttgtaaatagccaaagggctcagtaaca

SEQ ID NO: 61 - DNA, 546 bp, Parachlorella sp.
  misc_feature: RPS4 terminator
gcatagcatcagcctgtggcagggttgtggtagggctgagtggcagggttaaaggggttgcctaccccacccctactctcatgacaccagcaacagcagcagctcatgcagtactcaaatcactgatgtcaatggtgtgacacatttggttaaggctgctttttaaagtgctgctttgggggcagtgactgtgcagagcttggagcgtatccccatgtaatcagaaccgacgagagttcggggcaacctttcatcttcacattttttgtgatcagctacagagtctgaaatcaaatagaggctgccatctaaacgcaggagtcacaacgaaggcgaaaactccaattgctgtactcaatgcactaagtgattgttcaatggataaatacactatgctcaattcatgccagcagagctgctccttccagccagctacaatggctttttccacgccttttgaagtatgaatgttcagcttgctgtgcttgatgcatcaccataaacacaattctacaacatttcatgccaacaacagtacgggctttc

SEQ ID NO: 62 - DNA, 572 bp, Parachlorella sp.
  misc_feature: ACP1 promoter
agtttgcatagttaagtatgctggctattgcagtaccttatatgcaaacaagtgctcaatctgtttcatcattgtctgtgggcaaattgcctgccaatattctccagttattgcctgttgtttcaaatgattgaaattggaagttgtattgctctacatttttgacttgtgattttttcatttgttgatatctgacaactgtgaactgcactgaacttgctgtgcttataaatgcatttttttgttttgggccacgttgattccttgtgatactttcctgctatcaaaccaaaaatatactctcatgactgacgtgcaacaaatgcatggaagctttcaacgttacgacagctgcttgccccccatcagctattctacatgtgtaacctaccttgcatggccaccacaacgctactgcatgcaagatctggcgcaactggatgtcccaatagtagaagtatccggattatctccgagagttttacatatgtaatcgacgccatttctgtcatcaactataaatccattgctcctgcatttctggcactgacattctaccacaagcaatacca

SEQ ID NO: 63 - DNA, 869 bp, Parachlorella sp.
  misc_feature: ACP1 terminator
gcagcagcttgttatgccttccccatgggcatcagcatgctgcaagctgtctagatatccagctttcagtggaggttgagcgagggtcagcagcggttccctggcgatggcggtcagcttttctggaagccttcactaggactgcgcccagcgcatgtgacgccaatcgaacttgtgtgcaaggccaaattttgtgaccctgtgctgcacttcatgtattcaagaattgagaagaaatttcattgctgcccttctttcactttaatttccatccctggatccacctcccaccattgtggttgatgggtaggggttttgggtaggtgcagttcgttgtgcacgttgacatgtgtaacggtgagcaaaggaattgctgggcaagtagctattgcagcttaagggcatggtgaaacacttgtgctgtatttacagaggaagccagacaggtaaggagtgtgtggcagcttggaacaggagggctggtcgcaacaagtatgcatatcccatgattgttgacataagagcagcaggtgcatattgccagcctttgtgaaagtggattgaaaatcgattagttggtgtgatagctgaggctaggcactgccaacctgcagtgaaatgaggctccaagaccgggtaataatacaggcaatcgaatccagttgaaattacggcgattaaatccaagcgagcgttgtaagaacatctgcacctgtctgaagtagtgagcggataatgagcattgcttgccttctatcactatacctgacagttacgtgtcacacactctcaagcacaacacacagcggcaaagttacttgctaaacctcacagtcaagctgaaaataaaggctaaattacgtgagacc

SEQ ID NO: 64 - DNA, 23 bp, Parachlorella sp.
  misc_feature: SRP54 CRISPR target sequence (including PAM)
ggcgtgggacatggtgcgcaagg

SEQ ID NO: 65 - DNA, 1707 bp, Parachlorella sp.
  misc_feature: encodes cpSRP54
atgcttcggcagcagctgttgcacagcggcaggcagccgggtgcgacatgcagcttactaacctgctcgacatggcgaccgtctgccttgttcggccgtcctaagccccaaaaactgcacagccagcgcttgcagcatcagggccgcccctcccgcctcgtcgtgcgcagcgcaatgttcgacaacctgagccgcagcctggagagggcgtgggacatggtgcgcaaggacgggcggctaacggcggacaacatcaaggagcccatgcgggagattcgcagggcgctgcttgaggcggatgtgaggctgggggcgccgctgatcagattcttggtatctaccccccccccctcccaggtctccctccccgtggtgcgcaagtttgtgaaggcggtggaggagaaggcgctgggttctgcagtgaccaagggtgtcacccccgaccagcagctggtgaaggtggtgtacgaccagctgcgggagctgatgggggggcagcaggaagggctggtgcccacttcgccagaggagccgcaggtgatcttgatggcggggctgcagggcacggggaagacgacagctgcggggaagctggccttgttcctgcagaagaaggggcagaaggtgctgctggtggccaccgacatctaccgccccgccgccatcgaccagctggtgaagctgggcgacaggataggggtgccggtgttccagctgggaacccaggtgcagccgccggagattgcaaggcaggggctggagaaggcgcgagcagaggggtttgacgccgtcatcgtcgacacggcggggcggctgcagatcgaccagagcatgatggaggagctggtgcagatcaagtccacggtgaagccctccgacacgctgctagtggtcgatgcgatgacggggcaggaggcagccgggctggtgaaggcgttcaatgatgccgtggacatcacaggcgccgtgctgaccaagcttgacggggacagccgcggcggcgccgcgctgagcgtgcgccaggtcagcgggcggcccatcaagtttgtgggcatgggggagggcatggaggcgctggagcccttctaccccgagcgcatggccagcaggattctgggcatgggtgacgtggtcaccctggtggagaaggctgaggagagcatcaaggaagaggaggcgcaggagatatcgcggaagatgctgtcggccaaatttgactttgacgacttcctgaagcagtacaagatggtggcggggatggggaacatggcccaaatcatgaagatgctgccaggcatgaacaagtttacggagaagcagctggcgggcgttgagaagcagtacaaggtgtacgagagcatgatccagagcatgacggtgaaggagcgcaagcagccggagctgttggtgaagtcgccctccaggaggcggcgcatagcgcgcgggtcggggcgctcggagcgggaggtcacagagctgctgggggtgttcaccaacctgcggacgcagatgcagagcttctccaaaatgatggccatgggggggatgggcatgggctccatgatgagcgacgaggagatgatgcaggccacgctggcaggcgccggcccccgccccgtgccagctggcaaggtgcggcggaagaagctggccgcggcgggcgggtcgcggggcatggctgagctggcatccctgaaggcagaatga

SEQ ID NO: 66 - DNA, 2667 bp, Artificial Sequence
  Bleomycin resistance gene, codon optimized for Parachlorella and containing introns
atggccaaactgacatccgctgttcctgtgttgacagcaagagatgttgcaggtgcagtggagttttgtgagttctgagaagctgattgttgtttaacttctttgaaagctttatcgaagattctgcaagcgatgaacattgcttgtcaagaccgagagctgcatgcccacttgacatccagctttgaacggctcttcatgtttgatttgtttctgattgtagggacagatagactggggtttagcagggactttgtggaggacgattttgcaggagtggtgagggatgatgtgacactgtttatctcagcagtgcaggatcaagtgagtgcagcgtcagctgtggcagttgttggctttcgtctcagtcagtagtttgctgggattgattatggagggcacagttgcaattttgagttgcacgttgcgacaagcgtgttgacaaagcgtggtcaagccggccagtcttgccggtggcgggtggcttggtctaacttccgctctacagcaatcgttttgttcatggttacggggctggcgtgccagaaagtcctggtcagccaccctcgcttcaaagccgtagcccaacaactttgcgaatatgttcgatttgcaggtggtgcccgataatacactggcatgggtttgggtgagaggtacagctctgcgtgcaacaggttgcaagatgcagcgcaggtcttccctggtcaaacgatgtatgcagagttgagaggcacttgagctgggtgaatggcgtgggctcgtaggtagtgtgcagggcaggaagggcagccaattttggagttgtggtccggtgtcgttgcttcgagccttattaggactcttgctcatcaaagcgttagttgtgaataagttgatctgaaaggatgttatgtacagcaagcagcagcagttaagagtctggggagtagctgcacagggcgaggtgtcaagatgggaagggtcctgcctccttatgtgtttttccctgtaggggaggaagcctcttatgggcaatggttgggcatattttccagccagcccttctttctataggggccagggtgggcccagctcgtcttggcttccaccaccaggagagtgagggcattgaagggccataaatagtcctcccatctacgtgcaccagagggtgtcgtctaggctgtgcatgccacgaggggaaggagccaagaatgagtgtatgggttgttttcatgtttaggctgggataaaactgttttcaattgcgcctgccgggtgaaaaccacagcagcatcagcaagcttggagaaggccagcccgcccagcacaggctcacgttcccactcaggcggtcagtcgggcgggggtgtgagtcaggcaggcgagggtgtctgtgcctgacatcagcacctctgcttagccactgcagcccctggagcagggtagggcgtcatttgcagcaatcacctgctgcctcacacgtcgcagcttggaatttcaacgaccatcagcgctggggttgttgagggatcatagcagattttggtgcagcctggttgtcatgctctttgtggaatggcctctatgttcgagcaattcgttggatgttgaggtgcttggggacagagagtcgaatgatgggccagggtcaaacatgcgagcgtttggctgagtcagcggtttttgctggtcactttttcttttgtttcttatttaggtttgatggatgtgttttgtgctgctgccctgaagctgcagcagcgtgtctgccctgcgctactgcgggcaccaaggctatgtgctggtgcactcggctgcgctgcacctgtgcacctcgcactccgtccagcctccatgcagcacacgtactcacggtgtcctcctgacctgtcgtacgctattccaaacttgctcttttgctgccgctgctctcgtacacaattgctgttgattatcgatatctaatcgagcgcctgctgactgaactccgcaggtttggatgaactgtatgcagagtggtctgaagtggtgagcaccaactttaggtgggtgggctctgaaggaggaggagggagcgggtgattaaacagggcctgcatgaagaggagcaggggctgcatggacagcagggggaaggtgcagaagggagggtcaagcggggttcaggtggctgtgggtttctgcacgagcagtgaaagaagctgtatccttccacctgctttcactggcgaaaggttgaaaacaggatgtcgcagctggaaagatgttgcgctgtcaagtgcaagccatggttgagggtatgcctgtgtgcatgtgcttcttaaagttactcctgttctatggttctgggtgcttgttgtttgtggtgcagggatgcaagcggacctgcaatgacagagattggagaacaaccttggggaagggagtttgcattgagagatcctgcaggtgagggggcatgtaagcaatggcaggcaattcaagaacgaatcattgctgcaaatgctgggatggtatgcagctgaggtatctattgccttgtattttgtctcgcattgcatcggtggtgcgttctgtggcctgaggcacagttcttgctgtttgataagggttcgactgagttgtcgtgtgtgctgtgctgcaggcaattgcgtgcactttgttgcagaagaacaggactga

SEQ ID NO: 67 - DNA, 32 bp, Artificial Sequence
  AE596 Primer
tgcgacatgcagcttactaacctgctcgacat

SEQ ID NO: 68 - DNA, 28 bp, Artificial Sequence
  AE597 Primer
atgggctccttgatgttgtccgccgtta

SEQ ID NO: 69 - DNA, 21 bp, Artificial Sequence
  AE405 Primer
acccaaacccatgccagtgta

SEQ ID NO: 70 - DNA, 25 bp, Artificial Sequence
  AE406 Primer
actgtatgcagagtggtctgaagtg

SEQ ID NO: 71 - DNA, 4402 bp, Artificial Sequence
  Dual Promoter HygR cassette
cgtgcaggtgtacagattgaaggaaacaatggagatatctttggcagttgaaaaccgtgttcgaatcatgcttttctactctccaactgagacgaaatttatagcgccatgtcgcttctgactaccaggcttaggaaggcctcatcacaagctggatcggttcgaattaagcaggcactgaagccaagcttgcaagacagccaccttttaattccctcaaaacactttctcaattcagcccggtaaatatgccgattcacagcggccaagatagaggggaggttagcaagaatgttgcgatccctccccagtcgttgcctcgcacacaacctaggccttcacctttccatggaaaattgagaagtgaatattggttttcttacggcatatcagatgaaatcatgacccctaaacatgaagagctgcaggcaaaacacctgctctggacgagcacgatgaaatctcgagaacccgccgtacttcagttgatcccgcatgatgacggccgccattgaaataagccacctcactttattctagcaccgatttccaccgttgtgagggccgaacgaggacaatttcgtgcgaaacaagcacgaacacgcacacgattagtagtacagacgagcagatcgatggcatgcggcacggtctcgcgttctcggcgaccaggacaacggagcagagggaggcctgccgagttccgaggggcattttagtccaaaattgtgttgacacgtgaacaagtggcttgaaaagaggaaggaaatgcctgggtttcccttcgagagcgggaactcgcttgtgcgtcatcctagctacccatggtccctttgtgggggaggctgtttcgtcctaccgaatgtgtggcgctccatgcatcttctgcctcccaaaccaccaacatgagcacgcgaaggaaggagaaaaaagtggccgcaacgttctcttctcatatttattgtctcatcacaaacataggtacataatacaacaatcatgtccacagcccgaacccatgagagagaatcataatcaaagatgagccagccacgaagctaccggagaattctgtaagaaaaatgtttaaagttgaaaatgctaacagtgaagtgatatccttttttaatggagtgttgaggtgaagtctagcatcgtaggggaaaacaggattctgtgtcttccattctactccttgataaagcgaagaaatccgacaaaaccaaagagattgttcaagtttaagatttgtaagcgtacaactatgaacttcttctctttgtaggcctgagtggtcgtatgcatacgattcatgaagtgaatcagtatcgctggattttgcttaggagtaaagcacaactaagaaaatatgctgcctggcaggcatcctgagacatgaggcaagcgacgtagcaattgaatcctaatttaagccagggcatctgtatgactctgttagttaattgatgaaccaatgagctttaaaaaaaaatcgttgcgcgtaatgtagttttaattctccgccttgaggtgcggggccatttcggacaaggttctttggacggagatggcagcatgtgtcccttctccaaattggtccgtgtggtagttgagatgctgccttaaaattctgctcggtcatcctgccttcgcattcactcctttcgagctgtcgggttcctcacgaggcctccgggagcggattgcgcagaaaggcgacccggagacacagagaccatacaccgactaaattgcactggacgatacggcatggcgacgacgatggccaagcattgctacgtgattattcgccttgtcattcagggagaaatgatgacatgtgtgggacggtctttacatgggaagagggcatgaaaataacatggcctggcgggatggagcgtcacacctgtgtatgcgttcgatccacaagcaactcaccatttgcgtcggggcctgtctccaatctgctttaggctacttttctctaatttagcctattctatacagacagagacacacagggatcatggggaagaaaccggaactgaccgctacgtccgtggagaaattccttattgagaagttcgactctgtctccgacttgatgcaactgagcgagggagaggagagtagggcgttctcgtttgacgtagggggtcggggatacgtgttgagggttaatagttgtgcggacgggttctacaaggatcggtatgtctaccgtcatttcgcctccgccgctctccccataccagaggtactggacattggggagtttagcgaatctctcacgtactgcatctcgcgccgagcccagggagtgacgttgcaagatctgcccgaaactgaattgcctgccgttttgcaacccgtggccgaggccatggacgcgatcgctgccgcagatctgtctcagacgtccggctttggaccttttgggccccagggcatcgggcagtacacgacctggcgagacttcatctgcgccattgccgatcctcacgtctatcattggcagacagtcatggatgacaccgtgtctgcatccgtggcccaagcactggacgaactcatgttgtgggccgaggattgccctgaggtcaggcacctggtgcacgcggatttcggcagcaataacgtacttacagacaatggtcggattactgctgtcatcgactggtccgaagcgatgtttggtgatagccaatacgaagtggcgaacatattcttctggcgtccctggttggcgtgcatggagcagcagacacgctactttgaacggaggcacccggagctggccggctccccacgactccgcgcctatatgttgcgtatcggactcgatcagctttaccagtctctcgtcgacggcaacttcgacgacgccgcgtgggcgcagggccgctgcgacgcgatagtccgcagcggggctgggacggtgggtcggacccaaatcgcacgccggtcggctgcggtgtggacagacggctgtgttgaggtgcttgcggactcgggcaaccgtaggccgagcacccgaccgcgtgcaaaggagtgattgaatcattgaatgaaccattgtgtgcagaatcgatttcgggagtgttgccaacacaagaaatatgcccagggttgtgtagaagtttgcgtgaatgtgatgaagggaagccatacgctgaattatcgtgacgtgtgtgagacgaagtgtcacatcatacacccaatttgagaagctgtacctattagaagaatttgtgagatacattaaaccccttttggtacgtggtataattgttatttgggaagctgtaaacacgcagatcgttcctgagattgtcaattacttttgtggtgtttcctaaaggccgcatcactgcccgaatcgagttgatggcccgcaaaaataagcatacatcatatgaatacaattcagcttaaatttatcatacaaagatgtaagtgcagcgtgggtctgtaacgatcgggcgtaatttaagataatgcgagggaccgggggaggttttggaacggaatgaggaatgggtcatggcccataataataatatgggtttggtcgcctcgcacagcaaccgtacgtgcgaaaaaggaacagatccatttaataagttgaacgttattctttcctatgcaatgcgtgtatcggaggcgagagcaagtcataggtggctgcgcacaataattgagtctcagctgagcgccgtccgcgggtggtgtgagtggtcatcctcctcccggcctatcgctcacatcgcctctcaatggtggtggtggggcctgatatgacctcaatgccgacccatattaaaacccagtaaagcattcaccaacgaacgaggggctcttttgtgtgtgttttgagtatgattttacacctctttgtgcatctctctggtcttccttggttcccgtagtttgggcatcatcactcacgcttccctcgaccttcgttcttcctttacaaccccgacacaggtcagagttggagtaatcaaaaaaggggtgcacgaatgagatacattagattttgacagatatccttttactggagagggttcaagggatcaaatgaacagcgggcgttggcaatctagggagggatcggaggttggcagcgagcgaaagcgtgtccatccttttggctgtcacacctcacgaaccaactgttagcaggccagcacagatgacatacgagaatctttattatatcgtagaccttatgtggatgacctttggtgctgtgtgtctggcaatgaacctgaaggcttgatagggaggtggctcccgtaaaccctttgtcctttccacgctgagtctcccccgcactgtcctttatacaaattgttacagtcatctgcaggcggtttttctttggcaggcaaac

SEQ ID NO: 72 - DNA, 20 bp, Artificial Sequence
  ACCase target sequence 1
gggaaactgtgtgagaggag

SEQ ID NO: 73 - DNA, 20 bp, Artificial Sequence
  ACCase target sequence 2
ggggaggggcttccaccaca

SEQ ID NO: 74 - DNA, 20 bp, Artificial Sequence
  ACCase target sequence 3
ggtgcgtcgccaagactgcc

SEQ ID NO: 75 - DNA, 20 bp, Artificial Sequence
  ACCase target sequence 4
ggcgagctctcttttccgtg

SEQ ID NO: 76 - DNA, 18 bp, Artificial Sequence
  WX120-Accase Forward primer
ccttgatggtgctatatg

SEQ ID NO: 77 - DNA, 18 bp, Artificial Sequence
  WX107-Accase Reverse primer
ttggagacgaagagtgcc

SEQ ID NO: 78 - DNA, 18 bp, Nannochloropsis gaditana
  misc_feature: ZnCys-2845 gene target sequence
agtaggccattcccggag

SEQ ID NO: 79 - DNA, 120 bp, Artificial Sequence
  Oligonucleotide for producing chimeric guide targeting ZnCys-2845, first strand
aaaaaaagcaccgactcggtgccactttttcaagttgataacggactagccttattttaacttgctatttctagctctaaaacctccgggaatggcctactcctatagtgagtcgtatta

SEQ ID NO: 80 - DNA, 120 bp, Artificial Sequence
  Oligonucleotide for producing chimeric guide targeting ZnCys-2845, opposite strand
taatacgactcactataggagtaggccattcccggaggttttagagctagaaatagcaagttaaaataaggctagtccgttatcaacttgaaaaagtggcaccgagtcggtgcttttttt

SEQ ID NO: 81 - DNA, 20 bp, Artificial Sequence
  MA-ZnCys-Forward Primer
acctccttgtcactgagcag

SEQ ID NO: 82 - DNA, 21 bp, Artificial Sequence
  MA-ZnCys-Reverse Primer
gatcccaaaggtcatatccgt

SEQ ID NO: 83 - DNA, 20 bp, Artificial Sequence
  Bash-1 CRISPR target sequence
ggctgtcaaatcaacaaaac

SEQ ID NO: 84 - DNA, 20 bp, Artificial Sequence
  Bash-2 CRISPR target sequence
ggagctcagatatcttccag

SEQ ID NO: 85 - DNA, 20 bp, Artificial Sequence
  Bash-3 CRISPR target sequence
ggatcttccagtggtgggcg

SEQ ID NO: 86 - DNA, 20 bp, Artificial Sequence
  Bash-4 CRISPR target sequence
gggggactgtcccattgtgc

SEQ ID NO: 87 - DNA, 20 bp, Artificial Sequence
  Bash-5 CRISPR target sequence
ggtctgtctaaatcagcaca

SEQ ID NO: 88 - DNA, 20 bp, Artificial Sequence
  Bash-6 CRISPR target sequence
gggccaagtgcatcatgctc

SEQ ID NO: 89 - DNA, 20 bp, Artificial Sequence
  Bash-7 CRISPR target sequence
gggctcaggtacgcatctca

SEQ ID NO: 90 - DNA, 20 bp, Artificial Sequence
  Bash-8 CRISPR target sequence
ggattggaatcaattttgaa

SEQ ID NO: 91 - DNA, 20 bp, Artificial Sequence
  Bash-9 CRISPR target sequence
gggctgttcatcacaaagag

SEQ ID NO: 92 - DNA, 20 bp, Artificial Sequence
  Bash-10 CRISPR target sequence
ggctctttgtgatgaacagc

SEQ ID NO: 93 - DNA, 20 bp, Artificial Sequence
  Bash-11 CRISPR target sequence
ggcgtcggttcacgccaatc

SEQ ID NO: 94 - DNA, 20 bp, Artificial Sequence
  Bash-12 CRISPR target sequence
ggaactcgctcgtcgatcac

SEQ ID NO: 95 - DNA, 20 bp, Artificial Sequence
  MA-5'Bash-ZnCys Forward Primer
tagcagagcaggctcatcac

SEQ ID NO: 96 - DNA, 20 bp, Artificial Sequence
  MA-5'Bash-ZnCys Reverse primer
gaatatgtggtctagctcgt

SEQ ID NO: 97 - DNA, 20 bp, Artificial Sequence
  MA-3'Bash-ZnCys Forward Primer
atggctccaccctctgtaag

SEQ ID NO: 98 - DNA, 20 bp, Artificial Sequence
  MA-3'Bash-ZnCys Reverse primer
ctgactacagctagcacgat

SEQ ID NO: 99 - DNA, 21 bp, Artificial Sequence
  ZnCys-2845: Forward primer
atacaggaagcgtggttacag

SEQ ID NO: 100 - DNA, 21 bp, Artificial Sequence
  ZnCys-2845 Reverse primer
gaagtattaagggactggccg

SEQ ID NO: 101 - DNA, 849 bp, Nannochloropsis gaditana
  misc_feature: 1T5001704 Housekeeping gene
atgtcacggtcgcggtcctgttccgaagcttctgcggcctcttcgtcatcggcagcagcagcgtcttcgactcacgccccttcttcgcgcggagcttcggtggccgacggtgctgcaagggagcgagaagataatggcaaacgcctgaggtcaccgagccctgccggtggtgaagcttctggttccgaggaagcggaagaggatgatgagcccgccaaattgcatgtttctggtctaacaagaaacgtgacagaggagcatctcaacgagatattcgccacatttgggaagctgtcgcgtgtggaactggtacttgaccgacgagtgggcttatcgcggggcttcgcctatgttgagtacgatcatcggaaggacgctgaggaagcccagctgtacatggacggtggtcagcttgacggcgcacctttgaaagtgaactttgtgcttttgggcggagccgcagccgatctcctgtatcccgtggcggtggtcgagaaagggacctttacgatcgcaatggcggtccgccggagaggaggggcgggggagctcaatgggaggggcggcggggccggtctcgttctccgcctcgggggggtcgacacgaccgaggtcggttgccgccagggcggtttactcgaggagagcgcggacgcagccccccctaccgtcgccagccagaccctcgcggctggtcgccgccacggcgcgggccgggtgggcgggcatctccgcctcgggccgcggtcgcagccggagcagccgctcctcacgcagccgttcctagatggagggggcggcgccaacagggaaggcaagcaggagtctcacccgccgcttgaggcttga

SEQ ID NO: 102 - DNA, 408 bp, Artificial Sequence
  Region of ZnCys-2845 gene targeted by RNAi
gtttaaacgatcagccacgacggctctcgcatgcacaacgatggcatggattggcgcgcgaaggatgaggactgctcgtaccacaccgccgtggacgccagctgccacatcgacagtagctaccaccatgttgatgcctcaggccactccatggtcgacgcctcgggtcacagcacgatagacgcgtcgggccacgactccctcatcgactcaagcggccattacgacgactatctggcgcacaagggggacgcccgctacatggagcacagttgtgaagcctgcaagcgctcgaagaaacgatgcaaccgccgcaacccctgccagatctgcacctccaggggcatcaagtgtgtgccgcaaatccggggtcctgggcgccccccgggcagtaaaagcagtcggggc

SEQ ID NO: 103 - DNA, 163 bp, Artificial Sequence
  Terminator 9
gagtcaagggggaaggtgcatagtgtgcaacaacagcattaacgtcaaagaaaactgcacgttcaagcccgcgtgaacctgccggtcttctgatcgcctacatatagcagatactagttgtacttttttttccaaagggaacattcatgtatcaatttgaaat

SEQ ID NO: 104 - DNA, 22313 bp, Artificial Sequence
  pSGE06337-Asc/Not Fragment
  misc_feature: genes with promoters and terminators
gcggccgccgtatggtcgacggttgctcggatggggggggcggggagcgatggagggaggaagatcaggtaaggtctcgacagactagagaagcacgagtgcaggtataagaaacagcaaaaaaaagtaatgggcccaggcctggagagggtatttgtcttgtttttctttggccaggaacttgttctcctttcttcgtttctaggaccccgatccccgctcgcatttctctcttcctcagccgaagcgcagcggtaaagcatccattttatcccaccgaaagggcgctcccagccttcgtcgagcggaaccggggttacagtgcctcactcctttgcacgcggtcgggtgctcggcctacggttgcccgagtccgcaagcacctcaacacagccgtctgtccacaccgcagccgaccggcgtgcgatttgggtccgacccaccgtcccagccccgctgcggactatcgcgtcgcagcggccctgcgcccacgcggcgtcgtcgaagttgccgtcgacgagagactggtaaagctgatcgagtccgatacgcaacatataggcgcggagtcgtggggagccggccagctccgggtgcctccgttcaaagtagcgtgtctgctgctccatgcacgccaaccagggacgccagaagaatatgttcgccacttcgtattggctatcaccaaacatcgcttcggaccagtcgatgacagcagtaatccgaccattgtctgtaagtacgttattgctgccgaaatccgcgtgcaccaggtgcctgacctcagggcaatcctcggcccacaacatgagttcgtccagtgcttgggccacggatgcagacacggtgtcatccatgactgtctgccaatgatagacgtgaggatcggcaatggcgcagatgaagtctcgccaggtcgtgtactgcccgatgccctggggcccaaaaggtccaaagccggacgtctgagacagatctgcggcagcgatcgcgtccatggcctcggccacgggttgcaaaacggcaggcaattcagtttcgggcagatcttgcaacgtcactccctgggctcggcgcgagatgcagtacgtgagagattcgctaaactccccaatgtccagtacctctggtatggggagagcggcggaggcgaaatgacggtagacataccgatccttgtagaacccgtccgcacaactattaaccctcaacacgtatccccgaccccctacgtcaaacgagaacgccctactctcctctccctcgctcagttgcatcaagtcggagacagagtcgaacttctcaataaggaatttctccacggacgtagcggtcagttccggtttcttccccatcgagctcggtacccggggatccatgattgttgtattatgtacctatgtttgtgatgagacaataaatatgagaagagaacgttgcggccacttttttctccttccttcgcgtgctcatgttggtggtttgggaggcagaagatgcatggagcgccacacattcggtaggacgaaacagcctcccccacaaagggaccatgggtagctaggatgacgcacaagcgagttcccgctctcgaagggaaacccaggcatttccttcctcttttcaagccacttgttcacgtgtcaacacaattttggactaaaatgcccctcggaactcggcaggcctccctctgctccgttgtcctggtcgccgagaacgcgagaccgtgccgcatgccatcgatctgctcgtctgtactactaatcgtgtgcgtgttcgtgcttgtttcgcacgaaattgtcctcgttcggccctcacaacggtggaaatcggtgctagaataaagtgaggtggcttatttcaatggcggccgtcatcatgcgggatcaactgaagtacggcgggttctcgagatttcatcgtgctcgtccagagcaggtgttttgcctgcagctcttcatgtttaggggtcatgatttcatctgatatgccgtaagaaaaccaatattcacttctcaattttccatggaaaggtgaaggcctaggttgtgtgcgaggcaacgactggggagggatcgcaacattcttgctaacctcccctctatcttggccgctgtgaatcggcatatttaccgggctgaattgagaaagtgttttgagggaattaaaaggtggctgtcttgcaagcttggcttcagtgcctgcttaattcgaaccgatccagcttgtgatgaggccttcctaagcctggtagtcagaagcgacatggcgctataaatttcgtctcagttggagagtagaaaagcatgattcgaacacggttttcaactgccaaagatatctccattgtttccttcaatctgtacacctgcacggtgcaccagttggtacggcatattatggtttgaatgctggcgacctcatgaactttgttgatttttttagaattgtgtcatcgaaaaatatacaatgtcgaagtaaagtttatacactctgggtactcttcttctttgccatccagtaggtgtgggataggagtgcgtggtaattctctgagacagttttcctaccatgtttcgggtccacatagtacaagttgttactcgtgacacctcatttcgcttttgtttctccactaatggactacatttttcaaagcagcagcgtccgcgtttctcgattaagaatctcccgtccgctttgagtttgtttattttaaggattagaaggataaaagcggagctgcaaaggtgaaacatgcctgagaggactagaagacatacggagctgaagtgcggggaggttaaacccgatgatcccattccttgcatttgtcaaggctcaccgcattcatagttctaaaaagaaaatatttccgaataatgttaacacaaaaataattaaatactgttctatgtactccgttcatttgttgatggaatcaaaaggccagaaaaaaagagggggggactccaagctgccgcagacgctcgcctcgtctctcgttcgcggaatgccggtcgtggaaccgctgtgaagataccgtgccttggggatcaattcacacattgacgagggcgcctcacgccgtggcgtacttattcgggccaaaatgttatttccaaggggtgacggatggcatgctcgactcgtgtgatggctgatgcatcaaccctttcaatgctccttcctacttcctcttatccactggtagtctgtcatgagatgtggtgaaccgcgtccgtgataatagtgttctcatttaacctaacaaccaacacaatacaaaacttgattagatacccagtgcatcgaattttgggtgccttcaccgacaagcttgcactttctcgagggacgacaacaacaaaccacctacagcattaccgggcaatagcagcacaacatggaggacatcgtgattgccggaatttccggaagattgcctgagagcaacaacttggaggagttttggcagaacctcttcaatggcgtggacatggtgacagaggatgaccgaaggtggaaacctggattgtacggattgcctagacggaatgggaagttgaaggagattgaccggtttgacgccgcattttttggcgtgcatcctaaacaagcccatacgatggaccctcaattgcggttgatgttggagatcagttacgaggcgattgtggatggaggaattaatcccgtgagcatgagagggagcaaaactggcgtgtacatcggagtgagcggatctgaagcaggagaggccttttctaaagaccctgaagagttgttgggatactccatgacaggatgtcaacgagccatgttcgccaataggctcagctacttcttcgactttaacggacctagcacggcaatcgacacagcttgttcttctagcttgttggccttggaaaacgccttcaatgccatccggcacggacaatgtgatgccgccttgattggaggagtgaatttgttgttgaagcccaatacctccgtgcaattcatgaagctcgggatgttgtcccctgagggaacctgtaagtcctttgatgcctccggaaatggatactgtcggtctgaagcagctgtggctgtgttgttgacgaaaaagtctatggcaaagcggatctacgccaccgtgttgaatgcggggaacaatacagatggatacaaagagcaaggagtgacctttcctagcggagagatgcaacaacgattggtgcggtccctttaccaagaagccaacatctcccctgagcaagtggagtacattgaggcccatggaaccggaaccaaagtcggagatcctcaagaagtgaatggaatcgtgagcgtgttttgccaatcccctagagatcctttgttgattggatccaccaagtccaatatggggcaccctgaacctgcatctggattagccgcattggccaaagtcgtgttgtcattggagcatggagtgtgggcacctaacgtgcactttaacgagcctaaccctgacatccctgccttgacagatggaagattgtgtgtggtctccaaacctacacctgtgagaggaggaattgtcggaattaattcctttggatttgggggatcgaacgtccacgtcatcttgtctccccatgtgagcgactcttctgacaaaacacctgccccttctgtgccccgattgttgcaagcttctggacgaactgaagaggccgttacagccttgttttctaatgcccaacaacaccaagagaactcctcctacttgtccctgttgaatgatgtgtctggtgtgcctactgctggaatgccttaccgaggatacactttgattggcgcccaaggagaattgaccgaagtccaacagacccaacctacgcctcgacctttgtggtacatctgctccggaatgggaacgcaatgggctggaatgggacaatctttgatgcaattgtctgagtttcgagagtccattaaaagatccgatatcgccctgaaggacaccggattgtgcgtgtctcgattgttgatggaggccgatgagagcacctttgaagacaccgtccatgcatttgtgggattggccgccattcaagtggcccaaatcgacatgttgcggaagatggggttggagcctaatggaattgtgggacattctgtgggagaattggcatgtggatatgctgatggatctttgagccattccgaagccattttggcagcatactggcgaggaagatgcattaaagaggcgaacttgccccctggaggtatggcagcagtgggattgacatgggaagagtgtaaagcgcaatgccctcaaggagtggtgccagcttgccataatgcagaagatacagtgacaatttctggaccccaagactccgtgtccaaatttgtggcccaattgaaagaatctggcgtgtttgcgaaagaggtgcgatctgctggagtggcctttcattcgtactacatggcctccattgcccctgccttgttgtctgccttgcaaaaagtgatcaagtccccccgccctagaacagcacgatggatttctacatctattccccaatccgactgggaatctcctcttgccttgtactcttctgctgagtatcatgtgaacaatcttgtgtcccctgtcctcttccaagaggggttgaatcatgtccccgataatgccgtggtcgtcgaaatcgcccctcatgctttgttgcaagccatcctcaaacggtccttgaagcctacctgttccattttgcccttgatgaaacgtggccatgccaacaacctcgagttctttttgtcccatgtcggaaaagtgtacatgaacgggatcaacgtggattccaacaagctttaccctgccgtgaaataccctgtgcctcgtggaacccctctgatttccccttacatccagtgggatcactcccaatcctgggatgtgcctaaagtggaagactttcctgccggatctggcggatctacatctgcaactgtgtacaatatcgacatgaatcctgaatcccctgactactacatgattggacattgtatcgacggccgagtgttgtatcctgcaacgggctacctggtgttggcttggagaaccttgatgcgctctttgggaacggtgatggaccatacccctgtgacgtttgaagatgtgaccatccatcgagccacgatcttgcctaaaactggatctgtgcaattggaagtgcggttgatgcctgcaacaaatagatttgaagtgtccgagaatggcaatttggctgtgtccgggaaggtgtccgtgttggaagactctgggttggatgcgtttcatgccgagctgaacaagcccattaccgctgacaatgaagaccctaagctccgcctgaaatctggagatatctacaaggagttgcgattgaggggatacgactacggaaagacctttcaaggaattttggagagcaataatgccggagactccgggaaactccactggacgggaaattgggtgacgttcttggacacgatgctgcagatgatcgtcgtgggattgcctggaagaagcttgagactccctacccgaattcgatctgtgtgtgtggatcctaaattgcatgaggaacgcgtgaatgactacgaaggagaccaaaaagccgtgaatgtttttgtgaatcggtgcctcgacaacatcacagccggaggagtgcaaatctgtgggttgcatgctacagccgcccctcgaagacaacaacaacaaacaccccctaccttggaggaattcgtctttgtcccctacgaagatgccgattgcttgagaaccaatgagaaattggccgaccaattgcgacactgtaaaggattggtgcaacgattgcaacgcaaattggccaaacaaggcgtgaagatctccatccctggcttggaaggagcgtccgaagggcaattgattgaagcagaggccgagaaagggttgttgaggttgttgtccgtgttgtgcggcttggagttgaatgggaatttgagatccgaattggaacaaacggtgcaaaaagagagagactgcttgctgcaagatcccctgttgaatggcttgttggattctcaagcgttgcggcattgcctggataccgcgctggaaaattccacacctggcaagttcaaggtcttggaggcccttgctgctgatggacgcgtgttttctcaagctgtgtctttgctgaatattcaacctatgttgcgtttggactacactgcctctgatatttccgccgaccaattgtccgcccaacaatcttctttggaagagcagggaatctctaccgcccagtgggatcctcttcaaggacccgtgacaggaggattggatggagccgatcttgtggtgtgcaattgtgctgttggatctgccacgaatcctgcattgttgattgagaatttgacatctgccgctagagaaggaggattcatcttgttgcacacgttgttgagaggagatacgttgggagaaacagtggcgttcctcacgagccagaataaccggaagggcctgttgacgcaaaccgagtgggaagagctgttccaaaaagcctccctgaatgtggtgatgttgcggaagtcctattacggaagtgccttgtttttgtgtcgaagaagccaacaatccagccaaaagcaacctattcacatcttcgtggaccctaccgactacaaatgggtggagaccttgaaatccacactcgccgagtcctccgatatccccgtctggttgattgccaccaaaggccataatggagtcgtgggaatggtgaactgcttgcgtcaagagcctggaggaaatagaattcgatgcacatttgtctccaatttgtccaaaggagctgcagtgccttccttgttgcctaatgagaaggtgatgaaagccctgttgaagaaggacctggtgatgaacgtccaccgcgacggactgtggggagtgtttcgacatcaattgctgacccaagacctgtccgaagaattgaccgagcaggcctacgtgaatgtgttgacaagaggagatttgtctagtttgagatggattgcgtcccccttgaggcattttgtggcatcttctcctaatgtgcaattgtgcagagtgtactactcctccctgaacttccgcgacatcatgctcgccaccggaaaattgccccctgacgccatccctggagatgtggcattgcagcaatgtatgttgggaatggagttctccggaagagatccttctggaagaagagtgatgggattgttgcctgctaaaggattggccacatgtgtggatgccgataaaagatttttgtgggatgtgccttcttcttggacgttggagcaagccgcctctgtgcctgtcgtctacgctaccgcctactactccttggtggtcagaggaagattgagacctggagaaagtgtgttgattcattccggatctggtggagttggacaagccgctattgcaattgccttgagcatgcgctgtagagtgtttacaacagtgggatctaaagagaagaagcaatacttgcaagagcgcttcccccagttgacagccgagtccttcgccaattcccgcgattcctccttcgagcaacatgtgatgctgaacacacaaggaaaaggagtggacctcgtcttgaattccctcgccgaagagaaattgcaagcctccttgagatgtcttgccagacatggacgatttttggaaatcggaaaatacgatttgtccaacaacacccccctgggcatggccctgttcctgaagaacgtcgcctttcacgggatcttgctcgatgcactgtttgaagagggcaatcgtgaatgggaagaggtgtccgacctgttgaagaaaggaatttcctccggagtggtgcaacctttgagaacgaccgtgtttgagagaaaccaagtggaagaagcatttagatatatggcgcagggaaagcacatcggcaaggtgttgctgcaagtgcgctccgaagaatcctcctcctctggacctgcagtgtctgctttgagtattcctgccatttgccgaacgttttgtcctgcaagtttgtcctacatcatcaccggaggcttgggcggatttggattggaattggcccaatggttgacagaaagaggagcaagaaaattggtgttgacgtctagatccggaatccgcaacggctaccaagctaagagagtccgagagtggcaagccatgggaattcaagtgttggtctccacatccgacgtgtctaccttggatggaacagaacgattgatcacagaggcctgtaggttgggacctgtgggaggaattttccatttggcaatggtgttgaaagatggaatgctcgagaatttgacccctcaggagttcatcgaggtgaatcggcccaagtacgacgggacgatcaatttggacagcgtgacccgacaaaaatgcccccaattgcagcaattcgtcgtgttttcttccgtgtcttgtggacgagggaatgccggacagtccaattacggatttgcaaactccacaatggaaagaatctgcgaacaaagacgacaggagaatttgcctggattggccgtgcaatggggagccatcggagatgtgggagtggtcttggagacaatgggaggcaatgatgccgtgatcggaggaacattacctcaaagaatgtcttcctgcttggaggtgttggaccgctttttgtgtcaacaacgacctgtgatgtcctcttttgtgttggcagaaaaagtggtggtgacaaaaggagagggatccggacaaaaggacctggtggaagctgtggcgcacatcttgggagtgagggacgtgaatagcttgaatgccgacgcatcattggccgatttgggattggatagcttgatgggagtggaagtgagacaaaccttggagagagactacgacattgtgatggctatgagagagatcagacaattgacgatcaacaagttgcgggagttgagcaagcaatccggcgggaaggaggaatcccctgtgaagaggtctggagcccaagcattgttggaaagcgacttgtcccgaatgttggtgaatcctgacggacctacaatggcacccttgaatgaagtccaatccgcagaaagacccttgtttttggtacatcctatcgaaggatctattgccgcatttcgaaccttgacagcgaagctcagcgtgccctgctacggattgcaatgtaccaaagccgcccctttggactctatccaatctttggccgcctactatgtcgaatgtgtgaggcaagtgcagttggaaggaccctacagaattgccggatactcctttggagcttgtgtcgcttttgaaatgtgttcccaattgcaattggcgaaatgccctgtggagtacctgttcctgttcgacggatcccactcttacgtcgccgcgtacactcaatcttatcgagccaagttgacccccggaaaagaagctgaagcagaaacagaagccttgtgtgcctttatccagcagttcaccggaatcgagtacaacaaactcttggagaccttgttgcctttgtctgatttggaagccagagtggacaaagcagtggacctgatcacctcctcccacaagaacgtgtcccgcgatatgttgcattttgccgcctccacgttttaccacaagttgaaagccgccgacagatacgtgcctacatccaaataccacgggaatgtgaccttgttgagagccaaagcatcttctgagtatggagacggattgggatctgactacaaattgcacgaagtctgtgacgggaaggtgtccgtgcatgtgatcgagggcgaccatagaacctttttggagggagaaggagtggagtctatttccagcatcatccacagcagcttgtctgagcctagagtgtccacgagagaaggataaagtgatgcggcctttaggaaacaccacaaaagtaattgacaatctcaggaacgatctgcgtgtttacagcttcccaaataacaattataccacgtaccaaaaggggtttaatgtatctcacaaattcttctaataggtacagcttctcaaattgggtgtatgatgtgacacttcgtctcacacacgtcacgataattcagcgtatggcttcccttcatcacattcacgcaaacttctacacaaccctgggcatatttcttgtgttggcaacactcccgaaatcgattctgcacacaatggttcattcaatgattcaagtacgttttagacggactaggcagttcataatcaaagatgagccagccacgaagctaccggagaattctgtaagaaaaatgtttaaagttgaaaatgctaacagtgaagtgatatccttttttaatggagtgttgaggtgaagtctagcatcgtaggggaaaacaggattctgtgtcttccattctactccttgataaagcgaagaaatccgacaaaaccaaagagattgttcaagtttaagatttgtaagcgtacaactatgaacttcttctctttgtaggcctgagtggtcgtatgcatacgattcatgaagtgaatcagtatcgctggattttgcttaggagtaaagcacaactaagaaaatatgctgcctggcaggcatcctgagacatgaggcaagcgacgtagcaattgaatcctaatttaagccagggcatctgtatgactctgttagttaattgatgaaccaatgagctttaaaaaaaaatcgttgcgcgtaatgtagttttaattctccgccttgaggtgcggggccatttcggacaaggttctttggacggagatggcagcatgtgtcccttctccaaattggtccgtgtggtagttgagatgctgccttaaaattctgctcggtcatcctgccttcgcattcactcctttcgagctgtcgggttcctcacgaggcctccgggagcggattgcgcagaaaggcgacccggagacacagagaccatacaccgactaaattgcactggacgatacggcatggcgacgacgatggccaagcattgctacgtgattattcgccttgtcattcagggagaaatgatgacatgtgtgggacggtctttacatgggaagagggcatgaaaataacatggcctggcgggatggagcgtcacacctgtgtatgcgttcgatccacaagcaactcaccatttgcgtcggggcctgtctccaatctgctttaggctacttttctctaatttagcctattctatacagacagagacacacagggatcatggatggagtgagatgggcctttagatgtggatcttgggtgccttccagatctgagtggacattggcagcaagatgtgtgcaacaagaggagaagttgaggatcggacagttcgtgtttgccaaagacgccaaatctgcaatggccggacgattgttgatcaggaagttggtgtgcgagaaaatggggtttgcctgggacggatttaggttgcaaagaacagagcggggaaaaccttacttgccccaaacaagttccgccccttcttggagctttaatgtgagccatcaaggcgattacgcagtgttagcagccgaagctggaagacaagtgggaattgacgtcatgaaaacgtccagacctggaagctcttctgtgcaagagttcttccgcatcatgaatcgccaatttaccgacctcgagtggaccaatatccgaaccgcaggatctgactgggaccaactgcatatgttttaccgccattgggccttgaaagagtccttcaacaaggcaatcggaaccggattgggcttcgacttgcaacgtgccgaatttcatatctcccccaaccaaatgcgagaaggccaagtgtaccgacaaacaagaatgtacctcgactccgaagaagaagaagactggaccttcgaggagtccttgctcgacaaagatcaccatgtggctgtggccttgggaaaacctgacatctctatgtccaagaaagacggaggatcctcctgtgaggcaccacctgcagcttttacagtgttgtccttttccgacttggtgtcccaagcaacacctcttttggacgaagaccctacatattgggaggagtttcagaagaagaaggaggccccttcccgacaatccgatcaagagtaaccgtcaaaggcaaaggaggaaaagaagaaggcttacaccagtggcaccgaaatgttaatagcttgatgtttgcataaattgtcaaagtaaatgaaggtctagagcttgaaggttgcatctgaaaaaaatcaacaacagatggcgaaatcgatcgcatgctgaccgtcaggccttcagaattaccatcgcactgcatagtccgagcaggatgtcaatatagggccgtcgttaaggatacgtaggccgttgctgtttgctgccgcctgtggcccgttcatcgaatgaaaaaaaatgtgtatgttcaagttaatggttactaaatggttcgcaaggccgagtttcacagagcggcagaagacatccattgaaaactcgcaagtatgcaggaggaatgaatatactcagggtacgtgtatatttaaaactattgtgaagcattaggatagaaaggaaggatctgctacaaagtaaattcaggaacaatgtcggacacaccaaagattccgaccctgactgcccgcaaaaatggacgctattccaaaaacataaaggtaatgatacaaccccacgtaccttggcatttacgcatcccatacttatttgtttggcacccgttggtgtgttagtgggtagcgcttgttcttactttcgttcctgaacgcctgaaagccaggaagagaggcacgatttgagtctttataggggtcctccccggccaggcaacgcttctctcccccagctgctctcgcaaaatttctctgagggctgtcatagctctgcgcatccccttatgtgacgtcgccaccggtagatttcacgcggacacgggcatatctcccatgtgcgggaggaacaaatgacgatggggtcgcattccatcatagacttgggggcctctcccgtcatccagctctgcgtccagccttccggcactttgtcttgtgctcgtcgagcatcttccttcactccgacgcccatggttcgcttgcgcgcttgcgttcgttgtcccttgggtacgaaggcgatgctgttgtaatgaacgtcgataccccggtggagggatgggcgaagtttgtgaaagcgaggagaggtcatatgcagcaggaagagagagccaacccgccctctccgattcgagatgaacccttctaaagctgtgtgtcactcatgctcatgcatttccctacaatgcccatctataatgcgcgaatagagaagagatggccgctactctccgaatggatgaggcgggagccaacgaggcagggggtcgtgttggtggcgccggcgtggaggaggtccgggaacaagacagatatttgcccattgccaacatcagtcggataatgaagaagtctttggtaagtgtcgtgacgcatcctaatagtgcgctccttctagatgtcccaacatctgtcgccgatagaccttgttttgtcccacaagtctcctgttcccatcctcttctaccatgttctctttcctcactcatgtgctccctctctcgccactaatccgggcagccggcgaatgccaaaatagccaaggacgccaaagaaaccgtccaagaatgtgtttcagagttcatttctttcatcacctccgaagccagcgacaaatgccaacaggagaagcgaaagacgatcaacggggacgatctcctctgggccatgagcaccctgggcttcgacaaatacgtcgagcctctgaaacattatttggtcaagtaccgtgagtcagtgaaggggggtgagaaggcggacggagggaagaaagggaagtctgagggcacccaagtgacaggaagtagcgcggcgggtcctgtcacggcgaccgcgctagctgagcctcagggtgacagtcgggtggaatcgaccgaaagcagtagtctccccgagcagcaacatcacagttatgcagcccgtgctgtgtcaaggcagccgccttcctgaagacctgaaggcgagacagtaaattattttcagagtcgtacaggaaatggagagatgttgcggaaaagttatgccagtaacgtacgcgacacacatacaaactaaagataaaagcaaaattgcccacgcacagtctaaattgaatattttgctgcgagaggctacatgatcaagtggagagcatccattttttgagccccatgaggttcattcaagtctacttaagttgtcttttttaacttttcattgacatttttcgcctgttgtctcctctctgtgtcgatggccattcaataaaagcactgtcccggcattcaagagctgtagcggtatcatgtcaacaatcagtaggaataagcatacatcatatgaatacaattcagcttaaatttatcatacaaagatgtaagtgcagcgtgggtctgtaacgatcgggcgtaatttaagataatgcgagggaccgggggaggttttggaacggaatgaggaatgggtcatggcccataataataatatgggtttggtcgcctcgcacagcaaccgtacgtgcgaaaaaggaacagatccatttaataagttgaacgttattctttcctatgcaatgcgtgtatcggaggcgagagcaagtcataggtggctgcgcacaataattgagtctcagctgagcgccgtccgcgggtggtgtgagtggtcatcctcctcccggcctatcgctcacatcgcctctcaatggtggtggtggggcctgatatgacctcaatgccgacccatattaaaacccagtaaagcattcaccaacgaacgaggggctcttttgtgtgtgttttgagtatgattttacacctctttgtgcatctctctggtcttccttggttcccgtagtttgggcatcatcactcacgcttccctcgaccttcgttcttcctttacaaccccgacacaggtcagagttggagtaatcaaaaaaggggtgcacgaatgagatacattagattttgacagatatccttttactggagagggttcaagggatcaaatgaacagcgggcgttggcaatctagggagggatcggaggttggcagcgagcgaaagcgtgtccatccttttggctgtcacacctcacgaaccaactgttagcaggccagcacagatgacatacgagaatctttattatatcgtagaccttatgtggatgacctttggtgctgtgtgtctggcaatgaacctgaaggcttgatagggaggtggctcccgtaaaccctttgtcctttccacgctgagtctcccccgcactgtcctttatacaaattgttacagtcatctgcaggcggtttttctttggcaggcaaacatggagacttcgacgagaaaaggctttcatgaacgcagtgacgcacgatttccagctggagcgcttcatgattccatgaacttgacatcaaatgattcattcagaagctctcagtttggcaaggaaggcgccttcaacgaagtcaagaaagaccctggacgctggacggctgaggaacatatgttgtttcttaggggtctgcaattacacggtaaatcatggaagaaaatatccgagattgttacaacgcggacagtggtccaaattcgtacacatgcccagaaataccttataaagttggaaaaggctagaaaggctggtcatcagggtgtcttaatgatggatgggaaaggcgtcgataacactgaacgtcgaggcacttccaagaaatcatctttgtccacggaaacggtgagtttcacatctacttctcctgaatcttctgttctcgagcagaagagacagaaaaatgagccagcggctcacctgccaggtcctgtgcagcatactactgtacgcccttttgcacctgtcacaagagccgcaccttcaggctgccccccaactgcgcccgcaggattcgtgccatggatggtaggcccatacgcttgtgtccctccaacatactacaacatgcaaatgatggcccatggatatgactttggtgctccgctggtatcgccatcatcacaatatcgtgcgagtttttcaaatcccctgtctgcacccggaggaaattgccaagagcaggacttgggactaaacgcacctcaatctgtgagaatgcccttggaggctgaaatggctgcacaaattcattacctgggcattgacaacgaggaaactatcgcgcaaaatcagccaaattcctataagcgtctacgtgtccccgcaggtctggctatggcgacgcctgccgcggtttctacggcacaatcctctcattgtaaagtctacgttgccccgcagcagtcatgcacctcgccttctgatatgactccgactctaaccgcatcagccttacatcagccaccgcagggatctctttgcccgttcatgacatcaaatcctttagacgagctcatgcaaagcctgtcgcaggagaatctttcttcctcctgctcctcgacctctccatctatcgcacccgaagttgatgtacccagcatgcatgacatactcatttgggacctaaatgggaaacatagccgcccttcttcccttagctcctgggacgaggagggcttcgatggagtctcaacctcatcttcccctgcaagcattgacaatcacgttgtttgccaacctccggatttgagcgagcttcagtatgcgaaagctgcgtgagagtcaagggggaaggtgcatagtgtgcaacaacagcattaacgtcaaagaaaactgcacgttcaagcccgcgtgaacctgccggtcttctgatcgcctacatatagcagatactagttgtacttttttttccaaagggaacattcatgtatcaatttgaaatcaccagatataggtgacccgataacggagccaatagagtccaggcttttgcgtgtgacttgtacgtttgggggcagcagcatagctgggacggggtcgctcgtccctgtttcgagtatggcgcgcactctgacgccttcaagtgtggttgccatcttcgccgcaatcagctgagctgtcccgtcctcataacccaccacgacagctacttttcccatgccctccgctgacatcatcactaagcttttccctgcccttattgcacatgaatccttcagcgttgtccgtggtggagctagaaagccccatgctccttgttgcagcaaagtcagaaccgtgaagatcataaagccccacaatactgagaaatgcctgtgccatacactttgtcttgcgcctatcgacatttttttactcactatcactgatttggatcccagcttgtcctccccgtcctgtatcgtgcattgttgacttgagtttgataccagaaatgcttcgaaagtagtcagtcagcatccatgcgagtgttacaaaggacatgtccgtgcgccgacgcgcttccatgcaactttcactgattggggcttaaaaggagacaccccgcggtacgcgataccttgagacggacgccgggagacggtctaaagcgggttcccaggggccagcaaggggggaggtcgcttcctgcgggggcgacggaggtgagcgctctctccgtccatgtccagccccgccccgccaggcaggtgtgatgcgggcgttgcatgcgtggtcaggcagcgaagagagcctgagacacctgcgccaaccactgctgcctcacccgtgcgcggtggtggccgggcaagtgcgtgtaaggagggagccggacatggaggcgaggaggatgagagtgcacctcaaggctctcctcttctgctgtccacatcgcccaaataaaaaccaccatcctttatatcattggagcacatatcctgttgaatcacagatcaacgttttaaagagtcgtcaatccgcgacgacaggagagggggccgaagacagcgacgccaccatgtctatcagagggaagatatacctcatttctggctccgctgaaatcactgacctcccccgtggcgtcttcggtgttcgaggcggatgcgaagcagcagcaactcttgaaagattccctcaccgcagaccttaaactgctcttgcacgagtttgaacgcttccagcaagcgacagcattagtgtcgagagagggctcgaaagaggtggaggcaatggagcgggcggcgaaagtggaattcttcctaggctacatcggaaaggtgcttcaggaacttgccggcgccgacgcaccgaagctccaggaattagaggttcggatcaagaccagcctccttccattgaaggggcaagtggtgaacaagcttgcatcttccctgctctcgtcctccgccctcggtggtctgcagcatgagccttcctcctccgcatccatcccgtcgccttcctcttctccttcctcctcatgcagcacccacaccactccccccatctcccccgtatcaggggagaagatgacagtccaggatgatggccggagggagaggacgcatccgacggccgccgcgctcatgccctccgtgcgagtccaacgcctcgacagctcctccagtggcgccaccacctgctcggagaactccgaggaggggcgcggacagcttgacgatatggagtgcctgagcctgctcatggaggaagacggccagggactggggaggccacgatccggcactgtctttgcctttctctctgcgtcctctccctccggccatcatcctggactgtcatcttctcccctgatacgggggagatggggggagtggtgtgggtgctgcatgaggaggaaggagaagaggaaggcgacgggatggatgcggaggaggaaggctcatgctgcagaccaccgagggcggaggacgagagcagggaagatgcaagcttgttcaccacttgccccttcaatggaaggaggctggtcttgatccgaacctctaattcctggagcttcggtgcgtcggcgccggcaagttcctgaagcacctttccgatgtagcctaggaagaattccactttcgccgcccgctccattgcctccacctctttcgagccctctctcgacactaatgctgtcgcttgctggaagcgttcaaactcgtgcaagagcagtttaaggtctgcggtgagggaatctttcaagagttgctgctgcttcgcgtccgcctcgaacaccgaagacgccacgggggaggtcagtgatttcagcggagccaccggtgatccggcactgtctttgcctttctctccacaggtgtccactcccaggttcaatacagctagagagaaaatgatgtgaagaggaagagataggtttggaaaaagcatgtacaaagtaattacgatggagattttggtgctcttgccaggaagaatatatgctttttgtacactgctgcctctcaggactattttctcgggccttaataacacacagtctacttaattaaaaacatctatcctccagatcaccagggccagtgaggccggcataaaggacggcaaggaaagaaaagaaagaaagaaaaggacacttatagcatagtttgaagttataagtagtcgcaatctgtgtgcagccgacagatgctttttttttccgtttggcaggaggtgtagggatgtcgaagaccagtccagctagtatctatcctacaagtcaatcatgctgcgacaaaaatttctcgcacgaggcctctcgataaacaaaactttaaaagcacacttcattgtcatgcagagtaataactcttccgcgtcgatcaatttatcaatctctatcatttccgcccctttccttgcatagagcaagaaaagcgacccggatgaggataacatgtcctgcgccagtagtgtggcattgcctgtctctcatttacacgtactgaaagcataatgcacgcgcataccaatatttttcgtgtacggagatgaagagacgcgacacgtaagatcacgagaaggcgagcacggttgccaatggcagacgcgctagtctccattatcgcgttgttcggtagcttgctgcatgtcttcagtggcactatatccactctgcctcgtcttctacacgagggccacatcggtgcaagttcgaaaaatcatatctcaatcttcagatcctttccagaaacggtgctcaggcgggaaagtgaaggttttctactctagtggctaccccaattctctccgactgtcgcagacggtccttcgttgcgcacgcaccgcgcactacctctgaaattcgacaaccgaagttcaattttacatctaacttctttcccattctctcaccaaaagcctagcttacatgttggagagcgacgagagcggcctgcccgccatggagatcgagtgccgcatcaccggcaccctgaacggcgtggagttcgagctggtgggcggcggagagggcacccccgagcagggccgcatgaccaacaagatgaagagcaccaaaggcgccctgaccttcagcccctacctgctgagccacgtgatgggctacggcttctaccacttcggcacctaccccagcggctacgagaaccccttcctgcacgccatcaacaacggcggctacaccaacacccgcatcgagaagtacgaggacggcggcgtgctgcacgtgagcttcagctaccgctacgaggccggccgcgtgatcggcgacttcaaggtgatgggcaccggcttccccgaggacagcgtgatcttcaccgacaagatcatccgcagcaacgccaccgtggagcacctgcaccccatgggcgataacgatctggatggcagcttcacccgcaccttcagcctgcgcgacggcggctactacagctccgtggtggacagccacatgcacttcaagagcgccatccaccccagcatcctgcagaacgggggccccatgttcgccttccgccgcgtggaggaggatcacagcaacaccgagctgggcatcgtggagtaccagcacgccttcaagaccccggatgcagatgccggtgaagaataagggtgggaaggagtcggggagggtcctggcagagcggcgtcctcatgatgtgttggagacctggagagtcgagagcttcctcgtcacctgattgtcatgtgtgtataggttaagggggcccactcaaagccataaagacgaacacaaacactaatctcaacaaagtctactagcatgccgtctgtccatctttatttcctggcgcgcc

SEQ ID NO: 105 - DNA, 20 bp, Artificial Sequence
  HygR-forward primer
atggggaagaaaccggaact

SEQ ID NO: 106 - RNA, 80 nt, Artificial Sequence
  Cas9 Tracr RNA
ggaaccauucaaaacagcauagcaaguuaaaauaaggcuaguccguuaucaacuugaaaaaguggcaccgagucggugcu

SEQ ID NO: 107 - RNA, 42 nt, Artificial Sequence
  crRNA targeting Nannochloropsis acyl-CoA oxidase gene
gacgggggcuguggcgcgcgguuuuagagcuaugcuguuuug

SEQ ID NO: 108 - RNA, 42 nt, Artificial Sequence
  crRNA targeting Parachlorella cpSRP54 gene
ggcgugggacauggugcgcaguuuuagagcuaugcuguuuug

SEQ ID NO: 109 - RNA, 103 nt, Artificial Sequence
  Entire chimeric guide RNA for targeting Nannochloropsis LAR1 gene
ggugugggugcugcaugaggguuuuagagcuagaaauagcaaguuaaaauaaggcuaguccguuaucaacuugaaaaaguggcaccgagucggugcuuuuuuu

SEQ ID NO: 110 - protein, 342 aa, P1 bacteriophage
  misc_feature: Cre recombinase
SNLLTVHQNLPALPVDATSDEVRKNLMDMFRDRQAFSEHTWKMLLSVCRSWAAWCKLNNRKWFPAEPEDVRDYLLYLQARGLAVKTIQQHLGQLNMLHRRSGLPRPSDSNAVSLVMRRIRKENVDAGERAKQALAFERTDFDQVRSLMENSDRCQDIRNLAFLGIAYNTLLRIAEIARIRVKDISRTDGGRMLIHIGRTKTLVSTAGVEKALSLGVTKLVERWISVSGVADDPNNYLFCRVRKNGVAAPSATSQLSTRALEGIFEATHRLIYGAKDDSGQRYLAWSGHSARVGAARDMARAGVSIPEIMQAGGWTNVNIVMNYIRNLDSETGAMVRLLEDGD

SEQ ID NO: 111 - DNA, 1511 bp, Artificial Sequence
  Synthetic cre gene codon optimized for Nannochloropsis with nuclear localization sequence and intron
atgccgaaaaagaaacgcaaggtggggtccaacctgttgacggtgcatcagaacttgcctgccttgcctgtggatgccacatccgatgaagtgcggaagaacctgatggacatgttccgagacagacaagccttcagcgagcacacctggaagatgctgctgtccgtgtgtagatcttgggcagcatggtgcaagctcaataaccggaagtggttcccagccgaacctgaggacgtgagagactacctgctgtacctgcaagccagaggattggcagtgaaaaccatccagcagcacttgggccagctgaacatgttgcatcgacgatccgggttgcctagacctagcgactctaatgccgtgtctctggtgatgcgccgaatcagaaaggagaacgtggatgccggagaacgggccaaacaagcattggcctttgagcgaaccgacttcgaccaagtgagatccttgatggagaactccgaccggtgccaagacatccggaatctggcgttcttgggaatcgcctacaacacgttgttgagaatagccgagatcgcccggatccgcgtgaaagacatctccagaacagacggaggacggatgttgatccatatcggacggacgaagaccctggtgtctacagctggagtggaaaaggccctgtccttgggagtgacgaaattggtggagcgatggatctccgtgtctggagtggccgatgatcccaacaactacctgttctgcagagtgcggaagaatggagtggcagcccctagtgccacgtcccaattgtccacaagagccttagagggaatcttcgaagccacacatcgcctgatctacggcgccaaggacgattccggacaacggtatttggcctggtctggacattctgcaagagtgggagcagcccgagatatggtaagtgtttgcaagaggtcgtgcggaggatgaagaggtgcctgagaacgatagatggaaagggtcgggtggccttggtgatggcattcttttcagagctttccgaacacagtcttgtatctgcagtattaattgatgtatgcagtgtgtatgatcccacccagtgcctttatgcagcatgggattgttaaatagatatgaaagcataaccggtagaaaagaaagagagatgagacgcttggtagaacgccataatctatgcgttatatgaggagatacaagcataggctgtcactcaatatgtaaatgggagaagaagcgtatgttacttgtagatcagggagacgtgtggataaagcgcgcagcgatttgtcttcccctctccgtctcgatacctttctgctcggtaacaaactgacatggactctatcttatataaatcacaacgtttgtaggcgcgcgctggagtgtccattcccgagatcatgcaagctggaggatggaccaacgtgaacatcgtgatgaactacatccggaacctggactccgagacgggagcaatggtgcggctgttggaagatggagattaa

SEQ ID NO: 112 - DNA, 683 bp, Nannochloropsis gaditana
  misc_feature: Nitrite/Sulfite Reductase Promoter
ctggtgtcgtcaacagccagctgccacaagaaagtgaacatgcgtctatttatgacgtcattcatcaaccaccccgtttccaaacaccgtcccacgcgctgttgagagatgattttttgaatgccatatggtgctcaaacatgtgcatcgacgctgtcgcacaagcaggagcgggcttgcccactcgttcttgttaacggcttgattcaaaatccccgcccggaacaaaatatgccggagcgatccaacgaagcaaaagtcaaccagagcctctctttccgtccaacacccgtgttggtgccatgttaacaatagattcatgcatggataggcgaagacgtgagaagttacggagtttgggtcatgcttgcgtacatcactcaacccttttccccaaaaaaaaatcccgccatgcgattgccttcgttgcaccgcaaaacggaaattagttatggcgtcattgctcaagattactgtttttcgacaaggtgctgcacaaccttggaagaaaactctgcaaatccgtcaatcacatgagttgtagtttttttcggcaaggcgggtgagcgtagtgaattatattccttgtaaggcaaagcggatactaattttcacgtagttgccctgacctcctatgctcggaaacgccgccgtactgccccacccgaactcagatcaccagt

SEQ ID NO: 113 - DNA, 990 bp, Nannochloropsis gaditana
  misc_feature: Nitrite/Sulfite Reductase Terminator
aggcagggtccccgccaaaaagggtggcgaggacaagaagaagaaacaggaagggggggggcacgacggaggacttgtcgagtccatcagggaggtaggggcgggaagcctcgaatctgctagttggtagggataaatagagttcaaggaccgaaggaggaggcgccaggatcagcgaaagcctggattaagagcgagactccttgcgctgcagtcaaggcgattacaggacccccggtgtctgggtttggagatgacctcttggaggacggcttgatgcgggtttttgaggaaggttgtacatttttgtttgaaatttgcaaggaaagcgtcgcgctccggcatagagggatagggggaggaaagggcacttgtgcccgctccgtctctgtacgggtctttgaagaaaagattcgagaaaccacccaaagggcatcaaatgcgaaacctccctgaaaaaagtttcgattttctttatttgttgaggaggagagggaagagtggtatccaatgtggggtgtattcacgccaacaaagcggggggagctgacccagaggccacctgccacaggctccatccaaacaagctttcagggctgattccagaattagggttagagtaagaatgagggctacgccagcagtcatcctttgcgggcgtcttgagtcgcaagaagctctccaaggaaagcgaaggcgaattttccccaaaaacaaaggcagtggcgagctccttgtccctctttgagcacccctcctcgctaattttcttactctgattttttggggaagtgtttctccttctttcggagacgtggccttatgctccatcgccttcgcgcaccgactcgaccatgcccacacactctccgtgccccccttccctctgccacccttccctctccccccctcccttcctccctccctccctccctccctccctccctcctcccaggcacacccctattgtccacttcgcgccccaggctc

SEQ ID NO: 114 - DNA, 34 bp, P1 bacteriophage
  misc_feature: loxP sequence
ataacttcgtataatgtatgctatacgaagttat

SEQ ID NO: 115 - DNA, 4341 bp, Artificial Sequence
  Floxed HygR-GFP fragment
tccacagcccgaaccccttaagctagacgaacacagttagcgcggccgcataacttcgtatagcatacattatacgaagttatgatgctagcgtgtttaagaagtcacttaattaacgtatggtcgacggttgctcggatggggggggcggggagcgatggagggaggaagatcaggtaaggtctcgacagactagagaagcacgagtgcaggtataagaaacagcaaaaaaaagtaatgggcccaggcctggagagggtatttgtcttgtttttctttggccaggaacttgttctcctttcttcgtttctaggaccccgatccccgctcgcatttctctcttcctcagccgaagcgcagcggtaaagcatccattttatcccaccgaaagggcgctcccagccttcgtcgagcggaaccggggttacagtgcctcactcctttgcacgcggtcgggtgctcggcctacggttgcccgagtccgcaagcacctcaacacagccgtctgtccacaccgcagccgaccggcgtgcgatttgggtccgacccaccgtcccagccccgctgcggactatcgcgtcgcagcggccctgcgcccacgcggcgtcgtcgaagttgccgtcgacgagagactggtaaagctgatcgagtccgatacgcaacatataggcgcggagtcgtggggagccggccagctccgggtgcctccgttcaaagtagcgtgtctgctgctccatgcacgccaaccagggacgccagaagaatatgttcgccacttcgtattggctatcaccaaacatcgcttcggaccagtcgatgacagcagtaatccgaccattgtctgtaagtacgttattgctgccgaaatccgcgtgcaccaggtgcctgacctcagggcaatcctcggcccacaacatgagttcgtccagtgcttgggccacggatgcagacacggtgtcatccatgactgtctgccaatgatagacgtgaggatcggcaatggcgcagatgaagtctcgccaggtcgtgtactgcccgatgccctggggcccaaaaggtccaaagccggacgtctgagacagatctgcggcagcgatcgcgtccatggcctcggccacgggttgcaaaacggcaggcaattcagtttcgggcagatcttgcaacgtcactccctgggctcggcgcgagatgcagtacgtgagagattcgctaaactccccaatgtccagtacctctggtatggggagagcggcggaggcgaaatgacggtagacataccgatccttgtagaacccgtccgcacaactattaaccctcaacacgtatccccgaccccctacgtcaaacgagaacgccctactctcctctccctcgctcagttgcatcaagtcggagacagagtcgaacttctcaataaggaatttctccacggacgtagcggtcagttccggtttcttccccatcgagctcggtacccggggatccatgattgttgtattatgtacctatgtttgtgatgagacaataaatatgagaagagaacgttgcggccacttttttctccttccttcgcgtgctcatgttggtggtttgggaggcagaagatgcatggagcgccacacattcggtaggacgaaacagcctcccccacaaagggaccatgggtagctaggatgacgcacaagcgagttcccgctctcgaagggaaacccaggcatttccttcctcttttcaagccacttgttcacgtgtcaacacaattttggactaaaatgcccctcggaactcggcaggcctccctctgctccgttgtcctggtcgccgagaacgcgagaccgtgccgcatgccatcgatctgctcgtctgtactactaatcgtgtgcgtgttcgtgcttgtttcgcacgaaattgtcctcgttcggccctcacaacggtggaaatcggtgctagaataaagtgaggtggcttatttcaatggcggccgtcatcatgcgggatcaactgaagtacggcgggttctcgagatttcatcgtgctcgtccagagcaggtgttttgcctgcagctcttcatgtttaggggtcatgatttcatctgatatgccgtaagaaaaccaatattcacttctcaattttccatggaaaggtgaaggcctaggttgtgtgcgaggcaacgactggggagggatcgcaacattcttgctaacctcccctctatcttggccgctgtgaatcggcatatttaccgggctgaattgagaaagtgttttgagggaattaaaaggtggctgtcttgcaagcttggcttcagtgcctgcttaattcgaaccgatccagcttgtgatgaggccttcctaagcctggtagtcagaagcgacatggcgctataaatttcgtctcagttggagagtagaaaagcatgattcgaacacggttttcaactgccaaagatatctccattgtttccttcaatctgtacacctgcacgggccagtgaggccaggaaataaagatggacagacggcatgctagtagactttgttgagattagtgtttgtgttcgtctttatggctttgagtgggcccccttaacctatacacacatgacaatcaggtgacgaggaagctctcgactctccaggtctccaacacatcatgaggacgccgctctgccaggaccctccccgactccttcccacccttattcttcaccggcatctgcatccggggtcttgaaggcgtgctggtactccacgatgcccagctcggtgttgctgtgatcctcctccacgcggcggaaggcgaacatggggcccccgttctgcaggatgctggggtggatggcgctcttgaagtgcatgtggctgtccaccacggagctgtagtagccgccgtcgcgcaggctgaaggtgcgggtgaagctgccatccagatcgttatcgcccatggggtgcaggtgctccacggtggcgttgctgcggatgatcttgtcggtgaagatcacgctgtcctcggggaagccggtgcccatcaccttgaagtcgccgatcacgcggccggcctcgtagcggtagctgaagctcacgtgcagcacgccgccgtcctcgtacttctcgatgcgggtgttggtgtagccgccgttgttgatggcgtgcaggaaggggttctcgtagccgctggggtaggtgccgaagtggtagaagccgtagcccatcacgtggctcagcaggtaggggctgaaggtcagggcgcctttggtgctcttcatcttgttggtcatgcggccctgctcgggggtgccctctccgccgcccaccagctcgaactccacgccgttcagggtgccggtgatgcggcactcgatctccatggcgggcaggccgctctcgtcgctctccaacatgtaagctaggcttttggtgagagaatgggaaagaagttagatgtaaaattgaacttcggttgtcgaatttcagaggtagtgcgcggtgcgtgcgcaacgaaggaccgtctgcgacagtcggagagaattggggtagccactagagtagaaaaccttcactttcccgcctgagcaccgtttctggaaaggatctgaagattgagatatgatttttcgaacttgcaccgatgtggccctcgtgtagaagacgaggcagagtggatatagtgccactgaagacatgcagcaagctaccgaacaacgcgataatggagactagcgcgtctgccattggcaaccgtgctcgccttctcgtgatcttacgtgtcgcgtctcttcatctccgtacacgaaaaatattggtatgcgcgtgcattatgctttcagtacgtgtaaatgagagacaggcaatgccacactactggcgcaggacatgttatcctcatccgggtcgcttttcttgctctatgcaaggaaaggggcggaaatgatagagattgataaattgatcgacgcggaagagttattactctgcatgacaatgaagtgtgcttttaaagttttgtttatcgagaggcctcgtgcgagaaatttttgtcgcagcatgattgacttgtaggatagatactagctggactggtcttcgacatccctacacctcctgccaaacggaaaaaaaaagcatctgtcggctgcacacagattgcgactacttataacttcaaactatgctataagtgtccttttctttctttcttttctttccttgccgtcctttatgcccctgcagggtacgttttagacggactaggcagtataacttcgtatagcatacattatacgaagttatggcgcgccaggctacgttagttcagcagctgagaacgaccacgaacgggaa

SEQ ID NO: 116 - DNA, 7536 bp, Artificial Sequence
  Encodes fatty acid synthase of Danio rerio, codon optimized for Nannochloropsis
atggaggacatcgtgattgccggaatttccggaagattgcctgagagcaacaacttggaggagttttggcagaacctcttcaatggcgtggacatggtgacagaggatgaccgaaggtggaaacctggattgtacggattgcctagacggaatgggaagttgaaggagattgaccggtttgacgccgcattttttggcgtgcatcctaaacaagcccatacgatggaccctcaattgcggttgatgttggagatcagttacgaggcgattgtggatggaggaattaatcccgtgagcatgagagggagcaaaactggcgtgtacatcggagtgagcggatctgaagcaggagaggccttttctaaagaccctgaagagttgttgggatactccatgacaggatgtcaacgagccatgttcgccaataggctcagctacttcttcgactttaacggacctagcacggcaatcgacacagcttgttcttctagcttgttggccttggaaaacgccttcaatgccatccggcacggacaatgtgatgccgccttgattggaggagtgaatttgttgttgaagcccaatacctccgtgcaattcatgaagctcgggatgttgtcccctgagggaacctgtaagtcctttgatgcctccggaaatggatactgtcggtctgaagcagctgtggctgtgttgttgacgaaaaagtctatggcaaagcggatctacgccaccgtgttgaatgcggggaacaatacagatggatacaaagagcaaggagtgacctttcctagcggagagatgcaacaacgattggtgcggtccctttaccaagaagccaacatctcccctgagcaagtggagtacattgaggcccatggaaccggaaccaaagtcggagatcctcaagaagtgaatggaatcgtgagcgtgttttgccaatcccctagagatcctttgttgattggatccaccaagtccaatatggggcaccctgaacctgcatctggattagccgcattggccaaagtcgtgttgtcattggagcatggagtgtgggcacctaacgtgcactttaacgagcctaaccctgacatccctgccttgacagatggaagattgtgtgtggtctccaaacctacacctgtgagaggaggaattgtcggaattaattcctttggatttgggggatcgaacgtccacgtcatcttgtctccccatgtgagcgactcttctgacaaaacacctgccccttctgtgccccgattgttgcaagcttctggacgaactgaagaggccgttacagccttgttttctaatgcccaacaacaccaagagaactcctcctacttgtccctgttgaatgatgtgtctggtgtgcctactgctggaatgccttaccgaggatacactttgattggcgcccaaggagaattgaccgaagtccaacagacccaacctacgcctcgacctttgtggtacatctgctccggaatgggaacgcaatgggctggaatgggacaatctttgatgcaattgtctgagtttcgagagtccattaaaagatccgatatcgccctgaaggacaccggattgtgcgtgtctcgattgttgatggaggccgatgagagcacctttgaagacaccgtccatgcatttgtgggattggccgccattcaagtggcccaaatcgacatgttgcggaagatggggttggagcctaatggaattgtgggacattctgtgggagaattggcatgtggatatgctgatggatctttgagccattccgaagccattttggcagcatactggcgaggaagatgcattaaagaggcgaacttgccccctggaggtatggcagcagtgggattgacatgggaagagtgtaaagcgcaatgccctcaaggagtggtgccagcttgccataatgcagaagatacagtgacaatttctggaccccaagactccgtgtccaaatttgtggcccaattgaaagaatctggcgtgtttgcgaaagaggtgcgatctgctggagtggcctttcattcgtactacatggcctccattgcccctgccttgttgtctgccttgcaaaaagtgatcaagtccccccgccctagaacagcacgatggatttctacatctattccccaatccgactgggaatctcctcttgccttgtactcttctgctgagtatcatgtgaacaatcttgtgtcccctgtcctcttccaagaggggttgaatcatgtccccgataatgccgtggtcgtcgaaatcgcccctcatgctttgttgcaagccatcctcaaacggtccttgaagcctacctgttccattttgcccttgatgaaacgtggccatgccaacaacctcgagttctttttgtcccatgtcggaaaagtgtacatgaacgggatcaacgtggattccaacaagctttaccctgccgtgaaataccctgtgcctcgtggaacccctctgatttccccttacatccagtgggatcactcccaatcctgggatgtgcctaaagtggaagactttcctgccggatctggcggatctacatctgcaactgtgtacaatatcgacatgaatcctgaatcccctgactactacatgattggacattgtatcgacggccgagtgttgtatcctgcaacgggctacctggtgttggcttggagaaccttgatgcgctctttgggaacggtgatggaccatacccctgtgacgtttgaagatgtgaccatccatcgagccacgatcttgcctaaaactggatctgtgcaattggaagtgcggttgatgcctgcaacaaatagatttgaagtgtccgagaatggcaatttggctgtgtccgggaaggtgtccgtgttggaagactctgggttggatgcgtttcatgccgagctgaacaagcccattaccgctgacaatgaagaccctaagctccgcctgaaatctggagatatctacaaggagttgcgattgaggggatacgactacggaaagacctttcaaggaattttggagagcaataatgccggagactccgggaaactccactggacgggaaattgggtgacgttcttggacacgatgctgcagatgatcgtcgtgggattgcctggaagaagcttgagactccctacccgaattcgatctgtgtgtgtggatcctaaattgcatgaggaacgcgtgaatgactacgaaggagaccaaaaagccgtgaatgtttttgtgaatcggtgcctcgacaacatcacagccggaggagtgcaaatctgtgggttgcatgctacagccgcccctcgaagacaacaacaacaaacaccccctaccttggaggaattcgtctttgtcccctacgaagatgccgattgcttgagaaccaatgagaaattggccgaccaattgcgacactgtaaaggattggtgcaacgattgcaacgcaaattggccaaacaaggcgtgaagatctccatccctggcttggaaggagcgtccgaagggcaattgattgaagcagaggccgagaaagggttgttgaggttgttgtccgtgttgtgcggcttggagttgaatgggaatttgagatccgaattggaacaaacggtgcaaaaagagagagactgcttgctgcaagatcccctgttgaatggcttgttggattctcaagcgttgcggcattgcctggataccgcgctggaaaattccacacctggcaagttcaaggtcttggaggcccttgctgctgatggacgcgtgttttctcaagctgtgtctttgctgaatattcaacctatgttgcgtttggactacactgcctctgatatttccgccgaccaattgtccgcccaacaatcttctttggaagagcagggaatctctaccgcccagtgggatcctcttcaaggacccgtgacaggaggattggatggagccgatcttgtggtgtgcaattgtgctgttggatctgccacgaatcctgcattgttgattgagaatttgacatctgccgctagagaaggaggattcatcttgttgcacacgttgttgagaggagatacgttgggagaaacagtggcgttcctcacgagccagaataaccggaagggcctgttgacgcaaaccgagtgggaagagctgttccaaaaagcctccctgaatgtggtgatgttgcggaagtcctattacggaagtgccttgtttttgtgtcgaagaagccaacaatccagccaaaagcaacctattcacatcttcgtggaccctaccgactacaaatgggtggagaccttgaaatccacactcgccgagtcctccgatatccccgtctggttgattgccaccaaaggccataatggagtcgtgggaatggtgaactgcttgcgtcaagagcctggaggaaatagaattcgatgcacatttgtctccaatttgtccaaaggagctgcagtgccttccttgttgcctaatgagaaggtgatgaaagccctgttgaagaaggacctggtgatgaacgtccaccgcgacggactgtggggagtgtttcgacatcaattgctgacccaagacctgtccgaagaattgaccgagcaggcctacgtgaatgtgttgacaagaggagatttgtctagtttgagatggattgcgtcccccttgaggcattttgtggcatcttctcctaatgtgcaattgtgcagagtgtactactcctccctgaacttccgcgacatcatgctcgccaccggaaaattgccccctgacgccatccctggagatgtggcattgcagcaatgtatgttgggaatggagttctccggaagagatccttctggaagaagagtgatgggattgttgcctgctaaaggattggccacatgtgtggatgccgataaaagatttttgtgggatgtgccttcttcttggacgttggagcaagccgcctctgtgcctgtcgtctacgctaccgcctactactccttggtggtcagaggaagattgagacctggagaaagtgtgttgattcattccggatctggtggagttggacaagccgctattgcaattgccttgagcatgcgctgtagagtgtttacaacagtgggatctaaagagaagaagcaatacttgcaagagcgcttcccccagttgacagccgagtccttcgccaattcccgcgattcctccttcgagcaacatgtgatgctgaacacacaaggaaaaggagtggacctcgtcttgaattccctcgccgaagagaaattgcaagcctccttgagatgtcttgccagacatggacgatttttggaaatcggaaaatacgatttgtccaacaacacccccctgggcatggccctgttcctgaagaacgtcgcctttcacgggatcttgctcgatgcactgtttgaagagggcaatcgtgaatgggaagaggtgtccgacctgttgaagaaaggaatttcctccggagtggtgcaacctttgagaacgaccgtgtttgagagaaaccaagtggaagaagcatttagatatatggcgcagggaaagcacatcggcaaggtgttgctgcaagtgcgctccgaagaatcctcctcctctggacctgcagtgtctgctttgagtattcctgccatttgccgaacgttttgtcctgcaagtttgtcctacatcatcaccggaggcttgggcggatttggattggaattggcccaatggttgacagaaagaggagcaagaaaattggtgttgacgtctagatccggaatccgcaacggctaccaagctaagagagtccgagagtggcaagccatgggaattcaagtgttggtctccacatccgacgtgtctaccttggatggaacagaacgattgatcacagaggcctgtaggttgggacctgtgggaggaattttccatttggcaatggtgttgaaagatggaatgctcgagaatttgacccctcaggagttcatcgaggtgaatcggcccaagtacgacgggacgatcaatttggacagcgtgacccgacaaaaatgcccccaattgcagcaattcgtcgtgttttcttccgtgtcttgtggacgagggaatgccggacagtccaattacggatttgcaaactccacaatggaaagaatctgcgaacaaagacgacaggagaatttgcctggattggccgtgcaatggggagccatcggagatgtgggagtggtcttggagacaatgggaggcaatgatgccgtgatcggaggaacattacctcaaagaatgtcttcctgcttggaggtgttggaccgctttttgtgtcaacaacgacctgtgatgtcctcttttgtgttggcagaaaaagtggtggtgacaaaaggagagggatccggacaaaaggacctggtggaagctgtggcgcacatcttgggagtgagggacgtgaatagcttgaatgccgacgcatcattggccgatttgggattggatagcttgatgggagtggaagtgagacaaaccttggagagagactacgacattgtgatggctatgagagagatcagacaattgacgatcaacaagttgcgggagttgagcaagcaatccggcgggaaggaggaatcccctgtgaagaggtctggagcccaagcattgttggaaagcgacttgtcccgaatgttggtgaatcctgacggacctacaatggcacccttgaatgaagtccaatccgcagaaagacccttgtttttggtacatcctatcgaaggatctattgccgcatttcgaaccttgacagcgaagctcagcgtgccctgctacggattgcaatgtaccaaagccgcccctttggactctatccaatctttggccgcctactatgtcgaatgtgtgaggcaagtgcagttggaaggaccctacagaattgccggatactcctttggagcttgtgtcgcttttgaaatgtgttcccaattgcaattggcgaaatgccctgtggagtacctgttcctgttcgacggatcccactcttacgtcgccgcgtacactcaatcttatcgagccaagttgacccccggaaaagaagctgaagcagaaacagaagccttgtgtgcctttatccagcagttcaccggaatcgagtacaacaaactcttggagaccttgttgcctttgtctgatttggaagccagagtggacaaagcagtggacctgatcacctcctcccacaagaacgtgtcccgcgatatgttgcattttgccgcctccacgttttaccacaagttgaaagccgccgacagatacgtgcctacatccaaataccacgggaatgtgaccttgttgagagccaaagcatcttctgagtatggagacggattgggatctgactacaaattgcacgaagtctgtgacgggaaggtgtccgtgcatgtgatcgagggcgaccatagaacctttttggagggagaaggagtggagtctatttccagcatcatccacagcagcttgtctgagcctagagtgtccacgagagaaggataa

SEQ ID NO: 117 - DNA, 882 bp, Artificial Sequence
  Encodes pantetheine phosphotransferase of Danio rerio, codon optimized for Nannochloropsis
atggatggagtgagatgggcctttagatgtggatcttgggtgccttccagatctgagtggacattggcagcaagatgtgtgcaacaagaggagaagttgaggatcggacagttcgtgtttgccaaagacgccaaatctgcaatggccggacgattgttgatcaggaagttggtgtgcgagaaaatggggtttgcctgggacggatttaggttgcaaagaacagagcggggaaaaccttacttgccccaaacaagttccgccccttcttggagctttaatgtgagccatcaaggcgattacgcagtgttagcagccgaagctggaagacaagtgggaattgacgtcatgaaaacgtccagacctggaagctcttctgtgcaagagttcttccgcatcatgaatcgccaatttaccgacctcgagtggaccaatatccgaaccgcaggatctgactgggaccaactgcatatgttttaccgccattgggccttgaaagagtccttcaacaaggcaatcggaaccggattgggcttcgacttgcaacgtgccgaatttcatatctcccccaaccaaatgcgagaaggccaagtgtaccgacaaacaagaatgtacctcgactccgaagaagaagaagactggaccttcgaggagtccttgctcgacaaagatcaccatgtggctgtggccttgggaaaacctgacatctctatgtccaagaaagacggaggatcctcctgtgaggcaccacctgcagcttttacagtgttgtccttttccgacttggtgtcccaagcaacacctcttttggacgaagaccctacatattgggaggagtttcagaagaagaaggaggccccttcccgacaatccgatcaagagtaa

SEQ ID NO: 118 - DNA, 12447 bp, Artificial Sequence
  Encodes Type I fatty acid synthase of Thraustochytrid sp., codon optimized for Nannochloropsis
atgtccgaccagcagcaacaacagcagatcaaggtggaggagacagcccctgtggcccaagagcctaaaacccacttgtttgtggaccctgaagtgtcctcctgtattgccgcctttggaggccaaggatccgattggttgggagagttgcgatccttgcacaagaacgggaaatcctccgtgcgggagtttttggaactgggcctgtccaaattggaggatattgccgcgtccgatgagtggtacgccaaccacgggggcttgaatgtgagagcctggattgcctccgacaaatctgtgccgagcttcgacctgttgcgctacgcccctgtgagctttccgctgatcttcatgacgcaaatggccaactacatgcgggtgctggagttgttgggaacgagccacgagaaagtcgcacaacaaggctggtttaagggagccttgggacacagccagggagtcgtcgccgccgctgtgactgctgctgcatctactgatcgagaattgagaaacttgtccgtcgccggtttggagttcatgtcccaaattggattgggagcccaaaagagcatgaacttcgagttgtcccgcagatccgccggacctgaatcccctatgttgtctgtgcaaggcatgtccgaagccacgctcctgaaggccttcaaggaggccacgaagctcgccgtgcagaaagagaccatgatggccaaattttccacgtcctccaaggacgacaaagccgcccctaatgcctcccaaagattgggaattgccttgtgtaatggaaccgacgactacgtggtgtgtggagaacctaaggacctgcgcatgttgcggaaggtgatcgtgtccatgtccgccgaagtcgggaaagaggcccaagcccgagtgccattcagcaaaagaaaacctgtgacccaaacgacgtttctgcgcatgacagcgccattccattctgccttgaatgccgaagcctttgaacaagtggccgcttgggcagcatcttctgcttttggacaggaattggcccaacgcaccttgagaatccctgtgtgggacaccgagaaaggagccgacctccgcaagatggagccttcccaagtggtgaacatgttggcccgaaataccttggtctcctccgccaatttgctcagcacattgagagccgccgaagctgactgtaaagcctcccacttgatctcctttggacctggatctgtggccggacaccttatggccaatgcccttgtgggaactggaatccaggtgatccaggcgaatgaccctgactccaagagcaaggaaaatgccgccaccgcgagcagctcgtcgagccggagcagcgccaaatctcttgccgccatcttgacagccgaaaaacctgagcgaatccctgttgcaacaccttggggagagaaattcgcccctaagattgccgtgcgtgcgtgtgatggagaacgagtgttgatgaccaagtacacctccaccatcggacgagcccctgtgatgatgtccgggatgacgcctacgacgtcgttccacggaattgacttggtggccgcctgtgcaaatgccggatacaatgccgaattggctgctggaggattgcctacacctgacctgtttaagatgaaggtgcaggaactggcctccaagttgaaccctggagtgggaatggccattaacatgctgtacctgaacgcctaccagtggggcttccagttcccactggtgtgcgaattggcaaaagccgggctccccatcgagagcatcacaatcggagccggagtgcctaccgaagaaaaagccaaggacatctttgacggattgcaaggagccggcatcaacttgatcgggttcaaacctgggtccaaacaagccattagagacgtgctccaacttgcctccttgagaccctccatgaacatcatgctccagtggacctccggacgcggcggcggacatcacagctttgaggacttccacgagcccttgttggccacatacgaagagatcagacaacacgacaacatcatcctggtgatcggaagcggctttggagacgcccaaggagtgatgacataccttgatggatcctggtcccaatcccccaaatttggacgcttggccaaaatgcctgtggacggcgtgctcttcgggtcccggtgtatggtggcgaaagaggcagccacagcccctgaagtgaaacaattgatcgtcgatgctgctggattggaagacgagttgagctgggagaagtcctacgacgaagtggcaggaggagtcgttactgtgcaatctgagttgggagaacccattcacaaattggccacacggggcatactgttgtggcgggagttcgacaagcggttcttcagcttgcctcggggggagaaacggagagatgccatcttggcagcaaaagacgagattatcgcgaagctcaatgcggacttccagaaaccctacttcggccgcaaacgagacggatctgtgtgtgaagtggaggacatgacatatgctgaagtgctggagcggatggtgcagctgatgcacatcaagaacgggggggacaaggccgggcggttggcgcctacacgatggattgatcctacatatgcctctagagtgatgctgatgatgcaacgttccgccgcgagattggccaaggacaaaatggacaaggtggtgccttccaacaagctgttgatggaagaccctgacaaagccatcgccgacttcttggcagccattcctgccttggaggactccctgatggccgacgacgacgtgacctacttcctcgacttgtgcaaagtgcctacacgtggaaaacctgtgaacttcgtgcccgtggtggatgaggacttggtgttttgggtgaagaaggactccctgtggttttccgagcagttggatgcagtgcctgacagagatcctggacgagtgtgcgtgttgcatggacctgtggctgcccgatactccaccatcgtggatgagcctattgccgacattatggggaacatccacaaggacttggtgcgggacctgaagtgtgacgaggtgaaagtgaacgtgttggcccctgtggagttgcaacaagcaagcgtgctgaagatcatctccgagacaccccaattggtgagaggacgctcctttgtgcccaaccccatcgccaaggtgttgaaacgcgaggccttcgagaaagtgaagtacacatccgagggaggattggagtccatcaacgtgcaagaccctgagcgaggattgaccgtggccaccttgtcccaagtcggatccgacaacaaattggcagagttgcaagtgttcgacaaagaagccggagccgtgttgaagcagaagttcaccatcgacctgaccagcctccgccccatctttcagacagaggaggacaacttgagcgcaacgaagcagttgtacagaaccgcctgggactgtcaaggcgagttccatgccggagacacgttcaccgacgaagtggtggtcacatccgaaaacattgaggcctttaatcgagggacgcataccgagtacaatggatccgcagaagcccctatcgacatcagcatcatggccggatggcggcctttggcccgagcgttgttcgtggaagaattgcaatccaacctcctgaagctcgtccatctgaccaacggcatccggttgcccaaccccaaaacccgaacacctgtgaaagccggagaagtgattagatctgaggtgcgcattacaggaatcacgatccagcccaaagtgggcaagaaagtggcggtgaagggcatcatcacccgcgcctccgacaaaaatgccacgcccgaaatgtgggtcgaaatgaattccgccttcctcatccgcggagtcgccgagacacctgaagaatacgccacgacgttcgaagagtttcctgccgaaacccatgtgattgatgtgaaagatgccacggtggccgaattggtggcctctagagcctggatcaaactggacaacggccgcaaggtgcaagagggagaccgagtgacgatttccttgtcccatgtgtccaatcgctttgccggacccaaccgcttgaaggacatcaaggtgaccggagacgtgtttatcgagtccacctccgtgaaatcctccaattccggatccacccctttgggatcccctacgaattcctccgtctctggaacacaatccgacgacttcgtggacgtggacacctcctccaaggtgaaagcaggaacagtcgagtttgcctcctccgagggcgaagagttccagttgaatcccgtgatgtcgttcctggaaaagtactccgagcctatgcacaatggccatatcgccgagaatggcgggtacgagttgatcgccgagcctatggtggtgcctgcacctgctgattgtacgatgtacgcacgcggatccagagatgccaatcctatccatcgcgaatccgcattcgccgtgttggccgatttgcctggaggagagcctatcgtccatggaatgtggacagcatgtatggctagagctagattggaagaaggacctgccggaggaaatcctgcccgaatcgtctcctacgaggcctcctttgtggatatggtgcattgcggcgacgaactggtggtgacggctaaacaaacaggggtgaaggacggactgatgctgatcaacctgagcgtgaatcgggcctccgaccgagcattggtgatgactgctagagctgaattggaacaacctacaacggcctacttgttcacggggcaaggatccgcctctcccggaatgggaatggacagatatgcagcttccgcaacggtgcgcaaagtgtgggatgtggcagatgagtacttgagaaaccgatacgggttcagcatcctccagatcgtgcgggagaaccccaagtccttgacggtccactttggaggacctagaggaaaggtgattcgcgaaaatttgcgctccctgcagaccgaggaccctacaaccgggaaaaaaatgcccctgatccccgagatctcctccacgaccaagtccttcaccttcaattcccctaccggcttgttgtttgccacccaattctcccaacccgccctcgtcttggtgcagaaagccgcctttgaagaattgagagaagccggccttgtccctgaaaaagccttctttgccggccactctttgggcgagtatgccgcattggccggatttgccgatgtcctgtctgtggaggaccttgtggaaaccgtgtttttgaggggaatggtgatgcagaatgccgtgcctagggatgccgacggaaccagcaattacgccatggtggcagcaaatcctttgagagtcggacgtggatttacccctgagaccttgggagaagtcgtggacttgctgtgtgagcgggaggacttgggaaagcccttgctgcagatcgtgaactacaacgtgagatacacccagtacgtggtggcaggagagttgctcgcattggacgccttgggagaagccctgaatttggcctttgcaaccggaaataggaatgccgcggaattggccgagaaaggagcacaagcagccttggcctctttggcaaagaggggaggacggaaagagcccttgaaacggggaaaagccacaattcctttgcctggaatcgatgtgcccttccattcccggaagttgttgcccggagtgggagcgttcagacaactgttgagccctagacttgccttgagtacgatggagcggatctaccaccggttggtgggcaactacatccctaacgtgacagccgaggtcttgacgttggacagatcctacgccgagaaagtgcagaaagtgaccggaagtgcccctatgttggagttgttggccgactacgattccgccacccctgccgaaaaatgccgaacgttggtgatcgagttgttggcacatcagttcgccatgcctgtgcgctggattgagacccaagatctgatgtttggagcccgagtgcaacgcgtgatcgagatgggacctgcagccacattgacaacaatggccaagcacacgttgaaatccggagcctttggagacgccgacgagtacaaccctgagatcatgtggtggaagaacgaccgagagcgagtgtactacgagttggacgacgagggaccgagcttcgccgcctttgtggaacaattgaaggccgagatggagtccgaggccggagactctgaggagggagaagtgtccgaagcacctgcagcacctgcacctacacctgctcctgcacctgcacctgtggcacctaaacctgcacctgcacctgttgctgctcctgcacctgcaccttctggaggagcatctacacctgatgcacctgttgatacaaaacatgttttgagagtgttgttagcctccaagctcaagaagcccattggcgaagtccctgcctctacgtccgtccaaaccttgtccgccggccgatctgctgtccagaacgagatcatgggcgagttgtccgccgagttcaaaggcggcatccccgacaatgccggagaaatgcctttgtccgaattggccggaaatttgtcctcctacaaagaacctggagccgtgtctacaaaacttgtcacccgaacattgtctgcagccttgcctggaggctttggagccaatgccgccaaggactacctcacgcaacactgggggttgggaacgggacggaacttctccgtgctgttgcactcctgcacaatggcccctgagaaacgcttgaaatctgaggaggaaggaaaacaatggctcgactccgtctgcaaagcctacggtgatgatgttggagtgtctttgtcccctgccggagctggaggagctggaggagcaccttctggaatgatgatgatgccccagatgatgtccatgggaggacctgccgccgtgccgccaccggatgcacctgtctctgcattgcatgctatgagagtgatgttggccacaaaattcgagaaagggttcaacgagattagcgattctgccacagtggcctctctgtccaacgggaaatccgccctccagaacgaggtggccggagatttggcagccgaatttggagctgaaggagacgattccgcccagaagcccctcaccgaactcgccgccgcttttcaagccggatactctggacctggtaaagttttgtcaagagacatcaataaagtgttgggacaatgtctccccggaggatttggactgtccgccgcacgagcctaccttgcatctgaccgccttttgcctgccggacgagttgaatccgtgatgatccactccctgaccatggcccctaaggagcgcatcaagtccgccgaagacgcaaaggcctggctggatacagtgtgtggagcatatggatcttttgcaggaattgatatccctagagctggagcaggaggaggaggaggagccatgatgggatttgcgggacctggagtgtcttctgccgaagtgaatgggttgaaagcgaacctgcagtcgatggtggagacccagttggaggcccttcagcggttcatggagcaggaccccttgcatgccgacagattgttggatgtggagagaaaattgagaggagaaacagaggccaagttggacgccatccacgccgagttgacagtggacttctgcgagagagtgcaaccccaattcgacgagaaacgtgtgcgagtgtacgactccttctggaactgggtggtgcaagacgcgatgcagatgcacctgcacgtgctgtcccggttgaatgaggcccggaaaggacaatctacaggattacctgcaggagatgccaatccccatttcgaggacatgtccaagtggttgttgggaacgtcgagcagcgaagtgccccctacagcctggtttcgcaatttcttgtgcaatagagccacgccccagttgttgcaagccgtcaagttcttcgccaactccatgcacgaggccggacacgtggactacgcccaagccattgctttgcttgccgaacaggtgcaatgctggttgaataatgtgcctgtacatgtcgccacctttgaccccgtctcccccaatgtgcgagtgttggacaatggaacagtcgactacttcgagacccctagagaaggcgtgcctgacgccgtgagatacgtggcagaaatgagccgcggcctgttctacgtgagaagatctcctgccagagtggccaatccttcccaagcagtgaatgtggctggagatggacaattggcattgcctcctgctgctgattctaccggattgcaacctgccgatggagaacttgcttctggatggagacgacctagatccgaggccgaattggcccgagagttgaacaaccggtccggatccggccttgaagcattggacttggaagccgatgaagcctctgaggagtctaaagaagccttgcccgaaggacctaccttggaccgattgagattgacggtgtctagagatgcagcctcttctggagaagatgccggaagccctgggaaaatttccacgagctcgctgaagaacggctacgagtccatccacgtgtccaagcaggtgcccttcgtccacctcaagtccttgtccggagtcgacaaatctgtgcgcatcctcaatgagcagcttacctccgagtacttttcgtgccttgacgaaatcgccacatccggagtgtcctttgccggccaagtcgccttggttacaggagcaggagcaggatccattggaacagagttggtgaagtccctgttggagggaggagcaaccgtgttgtgtgccatgcgaaccgccagatccgagaatgcattgaccaaggaatacgcccgctttcagaacatctacaaggagtttggggccaaagacagcaagctctacctcgtgccgtgcaactgtgcgtccagccaggacatgaagagcatcgtggcctacacgtacgagcaattgggattggacgtggacttcgtcgtgccctttgccgcagccgcccaacaaggaaaagatatctcctctattgacgccgcctctgaagcctctcataggatgatgatgaccaatgtggtgcgcctcttgggagccttgcgtgatgccaaagccagccggggaattgtgacaagacctgccatggtgttgatcccttgctctcctaatcatggcgagttcgggaatgacggcctgtacgccgagtccaaattgggatgtgaagccttgctcaacaagtggtcctccgagggatggggagattatttgtccttggccgcctgcgtgatcggatggacaagaagtgccctcatggagcacaacaacattgtcgcccccggaatcgaagccttgggatgcagaacatttgcccctgaagaaacgaacttcaacctggtcggcctcttgcatccccgaatggtgaccttggccgccgaagaacctttgtgggccgatttgacaggaaattgggtggtgatccccaacatgaaggacgcagccgacggattgagaagcgagttgatgaccaagtcccgcattgccagagctgtcgccacatccaaccaattggaagagtccaaaaaacctgagggaggacgggagttgccgccaccggaatccgccggacctttggccggaacgatgttgggaatgacgccgtttccgaccttgcctagcgaagaagcccgaaagtccctgtctgccttggaaggaatggtggacttgcggaaagtcgtcgtgatcaccggatacggagaagtgggaccttggggaaatgcaagaacacgatgggaaatggagagctacggagagttctccctggagggggccatcgagttggcctggatggtcggattgatcaaaagacatgacggacctttgcctagcggacctcctcgacaacggtatgtgggatgggtggatgcaacgagtggagaagcagtggcagatcatgaggtgaaacggagatacgagaagaccctgttgcaatcttgcggaatccggattgtggaacccgccatcttcgagggctacaaccccgacgccaagcgctttttgcatagtgtggtgcttgaccgagatatgcccgccatcgagttggcctctctggaagaagggctgcagtacatgaaggagttgggagaggagtgctgtgacgtgtttgccagacctagcgatggacaatacatgatgcgcgtgaaaaaaggagccgaggtgagcatcgccaaagccctcaagttcaaccggaacgtggccggacaagtgcctacaggatgggatgccaggagattgggattgcctgccgatatcgcgaacagtgtggaccctgtgacgttgtacacgttggtgagcaccgtggaagccttgatggcagctggattgtcagacccttacgaattgtaccaatacgtccatgtgagcgaggtggggaatacaagcggaggaggaatggggggaatgaggtcgttgaagcggatgttccatcagcggaagctcgacgaggacatccctagtgacaccttggccgagtccttcatcaacacgatgcctgcctgggtgaacatgctgctcgtgtctagctccggacctatcaaaacacctgtgggagcatgcgcaacagcagccgaatctttggatattggaatggagaccatcctcagcggaaaagccagagtggtgatcgccggaggatacgacgactttggggaggagggatcctacgagttcgcccaaatgggagccacgaacaacaccgtcttggatgccgcacgtggaagaacagtgagagaatctagccgacctatgtcgtcgagcagggcaggatttgtggaatctcatggagccggaattcaagtgttgatggatgccgaattggccctggagatgggagcccctatcttcgccatcctggccctgacaaataccgccaccgacaaacagggacgctccattcctgcacctggacgtggaatcttgacatctgccagagaaagcaccaaagccggagtgagccctatgctttccttggaacgacgaagacaaggcttggaaatggaattggacgccttgaagacgctgaatgcccagaaggagcagtccgagggggaggatgccgcctttcttgagagactcgtgcagaaacgacgagcagcagccttggagacctggggacaagggtttttcaagaatgacccctccatcgcccctttgagaggagccttggccgtgtggggattgggagtggatgatttgggagttgcatcatttcatggaacgtctacgaagttgaacgacacgaacgagtccggcgtgctgaacaagcagatggagcatttgggacggagcaagggcaacgtgctcttcgtggtggcccagaagtacttgacgggacaccctaaaggagccgcctgtgcgtggatggtgaacgggttggtgcagtgtatgttggacgcacgagtgcctggaaatagaaatttggacaatgtggatgtgaagttgcagacgaactcctacctcgtgtaccccaatgagcccgtgcaactccccaagatcgaagccgccctgctgaagtccttcggattcggacaagccggagcagaggtcgtgatcgtgcatcctgaccgcttgttggccaccttgtctcctgaagccttcgccaactacatcgaagccagaaatattagagaaagacgaacgttccgaaatgcccagaacgtgatgtccggatcccgcaacatggtgatcgtgaaggagcaccccccctaccctgccgagttggaagaagccgtgtacctcgaccctcttgcccgtgcctcctatgatgccaaggagaatacctggacgttccgatccgccgctggacttacatcttctggaatgcctaaaattgcgtcgagccaagcgccgtcgtcgccgaaacctgcagcagcacctgtgtctgaatctgcctcccaatccgcccagatgtccgccaaagaccgattgcagatgacgatggccgagcaagccgccggaatcgcagcaagagctggaggttctggtgtgggagtcggagttgatgtcgaaaatgtgtccacttttgctgattacgctggatccaagcaagacttcatccaacggaacttcaccgaagccgagatcgcctactgcaagtccgccgccgatcctgccgcctcctttgctggaagatgggcagccaaagaagccgtcgtcaaagccttgtcctccattgcccctgattcccgatccttgtgggccggaggtcatgcatctttagttgatatcgaagtggtcgcaaatccttctggagcacctcaaattagattgcacggtcaccctgagcaagtctcccagatgctcgccgtgaacgacctgagcgtctccatctcccataccgccgaagtggcaatcgccaacgccatcgcccgaaagtga